European Patent Specification EP 3 592 384 B1, published July 2, 2025. Title: Antibodies specifically binding to human IL-1R7. Applicant: MAB Discovery GmbH. The sequence listing filed with the application follows.

SEQUENCE LISTING (1206 sequences)

SEQ ID NO: 1 - protein, 119 aa, Oryctolagus cuniculus
QSLEESGGRLVTPGTPLTLTCTISGIDLSAYAINWVRQAPGKGLEWIGGIANNGPTYYANWAKGRFTISKISTTVDLKITSPTTEDTATYFCARFPPGTNGGTDYFNIWGPGTLVTVSL

SEQ ID NO: 2 - protein, 114 aa, Oryctolagus cuniculus
QSVEESGGRLVTPGTPLTVTCTVSGFSLSGYDMNWVRQAPGKGLEWIGMIYPNSGTNYATWAKGRFTISKTPTTVALKITSPTTEDTATYFCARDSGWGAFDPWGPGTLVTISS

SEQ ID NO: 3 - protein, 119 aa, Oryctolagus cuniculus
QSLEESGGRLVTPGTPLTLTCTVSGFSLSTYAISWVRQAPGKGLEWIGGISNSGTTYYASWAKGRFTISKISTTVDLKITSPTTEDTATYFCARFPPGSNSGTDYFNIWGPGTLVTVSL

SEQ ID NO: 4 - protein, 113 aa, Oryctolagus cuniculus
QSLEESGGRLVTPGTPLTLTCTASGFSLSGLVVSWVRQAPGKGLEWIGVIGKSGNTYYASWAKGRFSISKTSSTTVDLKIASPTTEDTATYFCGRNISGSAVWGPGTLVTVSL

SEQ ID NO: 5 - protein, 126 aa, Oryctolagus cuniculus
QSLEESGGDLVKPGASLTLTCTASGFSFSSSYYMCWVRQAPGKWLEWIACIYAGSSGSTYYASWAKGRFTVSKTSSTTVTLEMTSLTAADTATYFCARDLGAGYAGYGYASDFNLWGPGTLVTVSS

SEQ ID NO: 6 - protein, 119 aa, Oryctolagus cuniculus
QSLEESGGRLVTPGTPLTLTCTVSGFSLSIYAISWVRQAPGKGLEWIGGIGNNGIIHYANWAKGRFTSSKISTTVDLKITSPTTEDTATYFCARFPPGSNSGTDYFNIWGPGTLVTVSL

SEQ ID NO: 7 - protein, 118 aa, Oryctolagus cuniculus
QSLEESGGDLVKPGASLTLTCTASGFSFSSSYYMCWVRQAPGKGLEWIGCIYGGSSGKTWYASWAKGRFTISKTSSTTVTLQMTSLTAADTATYFCARDNYDWYFNLWGPGTLVTVSS

SEQ ID NO: 8 - protein, 119 aa, Oryctolagus cuniculus
QSLEESGGRLVTPGTPLTLTCTVSGFSLSMYAINWVRQAPGKGLEWIGGIANNGPTYYASWAKGRFTISKISTTVDLRITSPTTEDTATYFCARFPPGSNSGTDYFNIWGPGTLVTVSL

SEQ ID NO: 9 - protein, 124 aa, Oryctolagus cuniculus
QSLEESGGDLVKPGASLTLTCKASGFDLSSYYYMCWFRQAPGKGPEWIACIYADDATTYYATWAKGRFTVSITSSTTVTLQMPSLTAADTATYFCARRDADYVGFIWAYYFNLWGPGTLVTVSS

SEQ ID NO: 10 - protein, 113 aa, Oryctolagus cuniculus
QSVEESGGRLVTPGTPLTLTCTVSGIDLSRNAMSWVRQAPGKGLEWIGIIRNTGTTWYASWAKGRFTISKTSTTVDLKITSPTTEDTATYFCARGNPGWASTWGPGTLVTVSS

SEQ ID NO: 11 - protein, 124 aa, Oryctolagus cuniculus
QEQLVESGGGLVQPGASLTLTCKTSGFSFSDNYAMCWVRQAPGKGLEWIACIYVGSGSTYYASWAQGRFTISKTSSTTVTLQMTSLTAADTATHFCARGVVIGNAYSMAHFSLWGSGTLVTVSS

SEQ ID NO: 12 - protein, 125 aa, Oryctolagus cuniculus
QSLEESGGGLVKPGASLTLTCTASGFSFSSGYYMCWVRQAPGKGLEWIGCIYTSSGSTYYASWAKGRFTISKTSSTTVTLQMTSLTAADTATYFCARRLNYVTYPAYGYGYFNLWGPGTLVTVSS

SEQ ID NO: 13 - protein, 121 aa, Oryctolagus cuniculus
QEQLEESGGDLVKPGASLTLTCTASGFSFNGNYYICWVRQAPGKGLEWIACIYAGSSGSTYYASWAKGRFTISKTSSTTVTLQMTSLTAADTATYFCVRDKPAGGSSYTLWGPGTLVTVSS

SEQ ID NO: 14 - protein, 120 aa, Oryctolagus cuniculus
QEQLEESGGDLVKPGASLTLTCTASGFSFSRSYYMCWVRQAPGKGLEWIACIYAGSSDSTYYASWAKGRFTISKTSSTTVTLQMTSLTAADTATYFCARGGGIIYTQNLWGPGTLVTVSS

SEQ ID NO: 15 - protein, 124 aa, Oryctolagus cuniculus
QSLEESGGDLVKPGASLTLTCTASGFSFVSMYWMCWVRQAPGKGLEWIACIYTGSSGKTHYASWAKGRSTISKTSSTTVTLQMTSLTAADTALYSCARAGSVGYGYDTAYFNLWGPGTLVTVSS

SEQ ID NO: 16 - protein, 114 aa, Oryctolagus cuniculus
QSVEESGGRLVTPGTPLTLTCTVSGFSLNSYDMSWVRQAPGKGLEYIGIIYDSGSTYYANWAKGRFTIAKTSTTVDLKITSPTTEDTATYFCARTLNTLPFNIWGPGTLVTVSL

SEQ ID NO: 17 - protein, 120 aa, Oryctolagus cuniculus
QEQLEESGGGLVQPEGSLTLTCTASGFSFSSSYWICWVRQAPGKGLEWIACIAAGSGSTYYASWAKGRFTISKTSSTTVTLQMTSLTAADTATYFCARDLGDDGYAYGLWGPGTLVTVSS

SEQ ID NO: 18 - protein, 120 aa, Oryctolagus cuniculus
QSLEESGGVLVKPGASLTLTCTASGIDFSSSYYICWVRQAPGKGLEWIACIYAGSSGSTYYASWAKGRFTISKTSSTTVTLQMTSLTAADTATYFCARGTGSSHYTSNLWGPGTLVTVSS

SEQ ID NO: 19 - protein, 120 aa, Oryctolagus cuniculus
QEQLVESGGGLVQPEGSLTLTCTASGFSFSDGYWMCWVRQAPGKGLEWIGCIYTGPGGTFYASWAKGRFTISKTSSTTVTLQLNSLTAADTATYFCARDLNGADSGSALWGPGTLVTVSS

SEQ ID NO: 20 - protein, 116 aa, Oryctolagus cuniculus
QSVEESGGRLVTPGTPLTLTCTASGFSLSSYAMSWVRQAPGKGLEWIGIIHYSGYTAYASWAKGRFTISKTSTTVDLKITSPTTEDTATYFCARGGDADNFYYNIWGPGTLVTVSL

SEQ ID NO: 21 - protein, 120 aa, Oryctolagus cuniculus
QEQLKESGGGLVTPGGTLTLTCTASGFTISNYQMTWVRQAPGKGLEYIGFIKADGSAYYANWAKGRFTISRTSTAVTLSLTTPTTGDTATYFCARDFYAGSSGNVNGDIWGPGTLVTVSL

SEQ ID NO: 22 - protein, 119 aa, Oryctolagus cuniculus
QSLEESGGRLVTPGTPLTLTCTVSGFSLNMYAINWVRQAPGKGLEWIGGIATNGIIHYASWVKGQFTISKISTTVDLKITSPTTEDTATYFCTRFPPGSNGGTAYFNIWGPGTLVTVSL

SEQ ID NO: 23 - protein, 114 aa, Oryctolagus cuniculus
QSVEESGGRLVTPGTPLTLTCTVSGFSLSNYDMNWVRQAPGKGLEWIGMIYPNSGTNYASWAKGRFTISKTPTTVALKITSPTTEDTATYFCARDSGWGAFDPWGPGTLVTVSS

SEQ ID NO: 24 - protein, 114 aa, Oryctolagus cuniculus
QSVEESGGRLVTPGTPLTLTCTVSGFSLSNYDMNWVRQAPGKGLEWIGMIYPNGGTNYATWAKGRFTISKTPTTVALKITSPTTEDTATYFCARDSGWGAFDPWGPGTLVTVSS

SEQ ID NO: 25 - protein, 112 aa, Oryctolagus cuniculus
QSVEESGGRLVTPGTPLTLTCTVSGIDLSSNAMIWVRQAPGKGLEWIGIIYASDSTYYATWAKGRFTISKTSTTVDLRMTSLTTEDTATYFCARGYSDIDIWGPGTLVTVSL

SEQ ID NO: 26 - protein, 119 aa, Oryctolagus cuniculus
QSLEESGGRLVTPGTPLTLTCTVSGFSLSMYTINWVRQAPGKGLEWIGGIATHGIIHYASWVKGRFTISKISTTVDLKITSPTTEDTATYFCARFPPGSNGGTAYFNIWGPGTLVTVSL

SEQ ID NO: 27 - protein, 121 aa, Oryctolagus cuniculus
QSVEESGGRLVTPGTPLTLTCTASGFSLSSNSISWVRQAPGKGLEWLGIISSSGSTYYASWAKGRFTISKASSTTVDLKITSPTTEDTATYFCAKGLGRGEYTSNDAFDPWGPGTLVTVSS

SEQ ID NO: 28 - protein, 118 aa, Oryctolagus cuniculus
QSLEESGGDLVKPGASLTLTCTASGFSFTSTYWMSWVRQAPGKGPEWIGCIVTGRGNTYYANWAKGRFTISKTSSTTVTLQMTSLTAADTATYFCARGSSDEIALDLWGQGTLVTVSS

SEQ ID NO: 29 - protein, 118 aa, Oryctolagus cuniculus
QSVEESGGRLVAPGTPLTLTCTVSGFSLNNYALSWVRQAPGKGLEYIGFINIIHGAYYASWAKGRFTISKTSTTVDLKITSPTTEDTATYFCARGPYYVGSEYVFDPWGPGTLVTVSS

SEQ ID NO: 30 - protein, 118 aa, Oryctolagus cuniculus
QSLEESGGRLVTPGGSLTLTCTVSGIDLSSHATSWVRQAPGKGLEWIGFIKTGGSAYYASWAKGRFTISKTSATVDLKITSPTTEDTATYFCASMFYAGDSGHYLHLWGPGTLVTVSS

SEQ ID NO: 31 - protein, 108 aa, Oryctolagus cuniculus
QSVEESGGGLVTPGGPLTLTCTVSGFSLSTYGVSWVRQAPGKGLEWIGYINTGGSASYATWAKGRFTISKTSTTVDLKITSPTTEDTATYFCAANNLWGPGTLVTVSS

SEQ ID NO: 32 - protein, 120 aa, Oryctolagus cuniculus
QSLEESGGDLVKPGASLTLTCTASGFSFSSNYYICWVRQAPGKGLEWIACIYTGSTGSTYYASWAKGRFTISKTSSTTVTLQMTSLTAADRATYFCARGGYSYGGAVSLWGPGTLVTVSS

SEQ ID NO: 33 - protein, 116 aa, Oryctolagus cuniculus
QSVEESGGRLVTPGTPLTLTCTVSGFSLTTYAMTWVRQAPGKGLEWIGIISNSGATAYASWAKGRFTISKTSTTVDLKITTPTTEDTATYFCARGRSGGWDALDPWGPGTLVTVSS

SEQ ID NO: 34 - protein, 122 aa, Oryctolagus cuniculus
QEQLEESGGDLVKPEGSLTLTCTASGFSFSSSYWICWVRQAPGKGLEWIACIGTSSTISYYASWAKGRFTISKTSSTTVTLRMTSLTAADTATYFCAREDYAGGTDYYFRLWGPGTLVTVSS

SEQ ID NO: 35 - protein, 116 aa, Oryctolagus cuniculus
QSVEESGGRLVTPGTPLTLTCTVSGFSLNNYAMSWVRQAPGKGLEWIGIIHYSGYIAYANWAKGRFTISKTSTTVDLKITSPTTEDTATYFCARGGDADNFYYNIWGPGTLVTVSL

SEQ ID NO: 36 - protein, 120 aa, Oryctolagus cuniculus
QEQLKESGGGLVTPGGTLTLTCTASGFTISNYQMTWVRQAPGKGLEYIGFIKPGGSAYYASWAKGRFTISRTSTTVTLKLTSPTTGDTATYFCARDFYAGSSGNVNGDIWGPGTLVTVSL

SEQ ID NO: 37 - protein, 116 aa, Oryctolagus cuniculus
QSLEESGGDLVKPGASLTLTCTASGFSFSSTYWACWVRQAPGKGLEWIACIDGGSSGITGYANWAKGRFTLSRTSSTAVTLQMTSLTAADTATYFCARELDYFNLWGPGTLVTVSS

SEQ ID NO: 38 - protein, 120 aa, Oryctolagus cuniculus
QEQLKESGGGLVTPGGTLTLTCTASGFTISSYQMTWVRQAPGKGLEYIGFINTGGSAYYASWAKGRFTISRTSTTVDLIITSPTTGDTATYFCARDFYAGSSGNVNGDIWGPGTLVTVSL

SEQ ID NO: 39 - protein, 119 aa, Oryctolagus cuniculus
QSLEESGGDLVKPGASLTLTCTASGFSFSSSYYMCWVRQAPGKGLEWIACIYAGSSGSTYYASWAKGRFTISKTSSTTVTLQMTSLTAADTATYFCARGAGSNGDFNLWGPGTLVTVSS

SEQ ID NO: 40 - protein, 120 aa, Oryctolagus cuniculus
QSLEESGGDLVKPGASLTLTCKASGFDFSSNYYMCWVRQAPGKGLEWIACIYTGSSGSTYYASWAKGRFTISKTSSTTVTLQMTSLTAADRATYFCARGAGSYGGAVRLWGPGTLVTVSS

SEQ ID NO: 41 - protein, 121 aa, Oryctolagus cuniculus
QSLEESGGDLVKPEGSLTLTCTASGFSFSSSYYMCWVRQAPGKGLEWIACIHAGSSGAAYYATWAKGRFTISKASSTTVTLHMTSLTAADTATYFCVRDGYDDYGDPFNLWGPGTLVTVSS

SEQ ID NO: 42 - protein, 118 aa, Oryctolagus cuniculus
QSVEESGGHLVTPGTPLTLTCTVSGFSLSNWIMSWVRQAPGEGLEWIGIITTSGNTYYASWAKGRFTISKTSTTVDLKITSPTTEDTATYFCARISAGSDSYIIDNIWGPGTLVTVSL

SEQ ID NO: 43 - protein, 120 aa, Oryctolagus cuniculus
QSLEESGGDLVKPGASLTLTCTASGFSLSSTYSMCWVRQAPGKGLEWVACIYTGSSGGTYYASWAKGRFTISKTSSTTVGLKMTSLTAADTATYFCARDAGNSGYYINLWGPGTLVTVSS

SEQ ID NO: 44 - protein, 112 aa, Oryctolagus cuniculus
QSLEESGGDLVKPGASLTLTCTASGFDFSSGYDMCWVRQAPGKGLELIACIYTVNDNTWYASWAKGRFTISKTSSTTVTLQMTSLTAADTATYFCARLYKLWGPGTLVTVSS

SEQ ID NO: 45 - protein, 120 aa, Oryctolagus cuniculus
QSLEESGGDLVKPGASLTLTCTASGIYFSSTYYTCWVRQAPGKGLEWIACIVDGSSGNTYYASWAKGRFTISKSSSTTVTLQMTSLTVADTATYFCGRPYVGYGYATDLWGPGTLVTVSS

SEQ ID NO: 46 - protein, 116 aa, Oryctolagus cuniculus
QSVEESGGRLVTPGTPLTLTCTVSGFSLSSAAMGWVRQAPGKGLEYIGYISTSGTPYYASWVNGRFTISKTSTTVDLKITSPTTEDTATYFCARDSYAGDYAFNLWGPGTLVTVSS

SEQ ID NO: 47 - protein, 114 aa, Oryctolagus cuniculus
QSVEESGGRLVTPGTPLTLTCTVSGFSLNSYDMSWVRQAPGKGLEYIGIIYNSGTTYYANWAKGRFTIAKTSTTVNLKITSPTTEDTATYFCARTHNTLPFYIWGPGTLVTVSL

SEQ ID NO: 48 - protein, 119 aa, Oryctolagus cuniculus
QSLEESGGDLVKPEGSLTLTCTASGFSFSSTYWICWVRQAPGKGLEWIACIYTDSSTSTYYASWAKGRFTISKTSSTTVTLQMTSLTAADTATYFCARGSGGSDYFNLWGPGTLVTVSS

SEQ ID NO: 49 - protein, 121 aa, Oryctolagus cuniculus
QEELVESGGGLVQPEGSLTLTCTASGFSFSSSYWICWVRQAPGKGLEWIACIVGGGGVNTYYANWAKGRFTISKTSSTTVTLEMTSLTVADTATYFCARDLGADGYAYHLWGPGTLVTVSS

SEQ ID NO: 50 - protein, 121 aa, Oryctolagus cuniculus
QELVESGGGLVQAGESLKLSCKASGIDFSSDGISWVRQAPGKGLKWIAFIYPGVGITHYAHSVKGRLTISSDNAQNTVFLQMTSLTASDTATYFCVRDPIYDDYGGRLDLWGQGTLVTVSS

SEQ ID NO: 51 - protein, 119 aa, Oryctolagus cuniculus
QSLEESGGRLVTPGTPLTLTCTVSGFSLSSYAISWVRQAPGKGLEWIGGVANNGITNYASWARGRFTISKISTTVDLKIISPTTEDTATYFCARFPPGSNGGTDYFNIWGPGTLVTVSL

SEQ ID NO: 52 - protein, 116 aa, Oryctolagus cuniculus
QSVEESGGRLVTPGTPLTLTCTVSGIDLSSNALGWVRQAPGKGLEYIGYISTGGSAYYATWVNGRFTISKTSTTVDLKMTSLTAADTATYFCARDSYAGDYAFNLWGPGTLVTVSS

SEQ ID NO: 53 - protein, 114 aa, Oryctolagus cuniculus
QSLEESGGRLVTPGTPLTLTCTVSGFSLNSYDMSWVRQAPGKGLEYIGIIYDSGSTYYASWAKGRFTIAKTSTTVDLKITSPTTEDTATYFCARARNTLPFNIWGPGTLVTVSL

SEQ ID NO: 54 - protein, 119 aa, Oryctolagus cuniculus
QSVEESGGRLVTPGTPLTLTCTVSGIDLSNYAMGWVRQAPGKGLEWIGVISSNGGTVYANWAKGRFTISKVSTSVPLKITSPTTEDTATYFCARGLYSASGWSYCFDIWGPGTLVTVSL

SEQ ID NO: 55 - protein, 118 aa, Oryctolagus cuniculus
QSVEESGGRLVTPGGSLTLTCTVSGIDLSVYAMSWVRQAPGKGLEWIGIITFSGNTYYASWAKGRFTISKTSTTVDLKITSPATGDTATYFCARFDFLVGLTYAGVLWGPGTLVTVSS

SEQ ID NO: 56 - protein, 118 aa, Oryctolagus cuniculus
QSVEESGGRLVTPGTPLTLTCAVSGFSLSTYGVSWVRQAPGKGLEWIGYINIYGRTYYANWAKSRFTISKTSTTVDLKMTSPTTEDTATYFCARNGASGTYYSSLYIWGPGTLVTVSL

SEQ ID NO: 57 - protein, 119 aa, Oryctolagus cuniculus
QSLEESGGRLVTPGTPLTLTCTVSGFSLSMYAINWVRQAPGKGLEWIGGIANNGPTYYASWAKGRFTISKISTTVDLKITSPTTEDTATYFCARFPPGSNSGTDYFNIWGPGTLVTVSL

SEQ ID NO: 58 - protein, 111 aa, Oryctolagus cuniculus
QSVEESGGRLVTPGTPLTLTCTVSGIDLSRYAMSWVRQAPGKGLEYIGIISSSGNSYYASWAKGRFTISKASTTVDLKITVPTTEDTATYFCVGGSGWDLWGQGTLVTVSS

SEQ ID NO: 59 - protein, 115 aa, Oryctolagus cuniculus
QSLEESGGRLVTPGGSLTLTCTVSGIDLSSYAMGWVRQAPGKGLEYIGIISSGLTYYASWAKGRFTISKTSTTVDLKMTSLTTEDTATYFCARGLGAASATWDIWGPGTLVTVSL

SEQ ID NO: 60 - protein, 120 aa, Oryctolagus cuniculus
QSLEESGGDLVKPGASLALTCTASGFSFSSSYWICWVRQAPGKGLEWIACINFGRSGNIYYARWAKGRFTISKTSSTTVTLQMTSLTAADTATYFCARDKAGDSYYFNLWGPGTLVTVSS

SEQ ID NO: 61 - protein, 112 aa, Oryctolagus cuniculus
QSLEESGGRLVTPGTPLTLTCTASGFSLNNYYMTWVRQAPGEGLEYIGFIDPYSSPYYASWAKGRFTISRTSTTVDLKISSPTAEDTATYFCARGVAVGDIWGPGTLVTVSL

SEQ ID NO: 62 - protein, 112 aa, Oryctolagus cuniculus
QSLEESGGRLVTPGTPLTLTCTVSGIDLSSYHMSWVRQAPGKGLEWIGVIYGSGSAWYASWAKGRFTISKTSTTVDLKITSPTTEDTATYFCVRGILVSDLWGPGTLVTVSS

SEQ ID NO: 63 - protein, 121 aa, Oryctolagus cuniculus
QQQLEESGGGLVKPEGSLTLTCKASGFDFSTIPMCWVRQAPGKGLEWIACIYPDYGDTFYATWAKGRFTISKTSSTTVTLQMTSLTVADTATYFCARGPIMVVSPSYFNFWGPGTLVTVSS

SEQ ID NO: 64 - protein, 123 aa, Oryctolagus cuniculus
QSLEESGGDLVQPGASLTLTCTASGFIFSDNYAMCWVRQAPGKGLEWIACIFGSSGSIAYATWAKGRFTISKTSSTTVTLQMTSLAAADTATYFCARSYYSGGYKYVYVFDLWGPGTLVTVSS

SEQ ID NO: 65 - protein, 113 aa, Oryctolagus cuniculus
QEQLVESGGGLFQPGGSLTLTCTASGFTISSYHMGWVRQAPGEGLEYIGFITTTGGSYYASWARGRFTISKTSTTVDLKMTSLTAADTATYFCAKGIAVASLWGPGTLVTVSS

SEQ ID NO: 66 - protein, 118 aa, Oryctolagus cuniculus
QSLEESGGDLVKPGASLRLTCTASGLSFSSRYWIYWVRQAPGKGLEWIACIDTGSRGFTYYPSWAKGRFTISKTSSTTVTLQMTSLTAADTATYFCARLDTYDDYDLWGPGTLVTVSS

SEQ ID NO: 67 - protein, 118 aa, Oryctolagus cuniculus
QSVEESGGRLVTPGTPLTLTCTASGFSLYSYFLTWVRQSPGKGLEWIGFMNSGGSTYYASWVNGRFTISKTSATVDLKITGATTEDTATYFCARMFYAGDSGHYFDLWGPGTLVTVSS

SEQ ID NO: 68 - protein, 121 aa, Oryctolagus cuniculus
QSVEESGGRLVTPGTPLTLTCTVSGIDLSSYAMSWVRQAPGKGLEWIGMIRSSGITWYASWAKGRFTISKTSTTVDLKITSPTTEDTATYFCARDSDYDDYGNSYYGMDPWGPGTLVTVSS

SEQ ID NO: 69 - protein, 120 aa, Oryctolagus cuniculus
QEQLEESGGDLVKPEGSLTLTCTASGFDFSSNAMCWVRQAPGKGLEWIACIYAGSRGSAYYASWVNGRFSISKTSSTTVTLQMTSLTAADTATYFCAREYVGSQGYFNLWGPGTLVTVSS

SEQ ID NO: 70 - protein, 118 aa, Oryctolagus cuniculus
QSVEESGGRLVTPGTPLTLTCTVSGFSLSVYAMSWVRQAPGKGLEWIGIITWSADTYYTSWAKGRFSISKTSTTVDLKVASPTTEDTATYFCARFDYLVGGTWAGVLWGPGTLVTVSS

SEQ ID NO: 71 - protein, 117 aa, Oryctolagus cuniculus
QSVEESGGRLVTPGTPLTLTCTASGFSLNSYAMGWVRQAPGKGLEWIGINGVSGTTYYATWANGRFTISKTSTTVDLKIIRPTTEDTATYFCARGVGDTTDTQLDLWGQGTLVTVSS

SEQ ID NO: 72 - protein, 120 aa, Oryctolagus cuniculus
QEQLVESGGGLVQPEGSLTLTCTASGFDFSGSYWNCWVRQAPGKGLEWIACIDGEGSGNTYYASWVNGRFTISKTSSTTVTLQMTRLTAADTATYFCARDPSAWGGLDLWGPGTLVTVSS

SEQ ID NO: 73 - protein, 118 aa, Oryctolagus cuniculus
QSLEESGGDLVKPGASLTLTCKASGFSFSSGYDMCWVRQAPGKGLEWIACIDTGDGSTYYASWVNGRFTISKTSSTTVTLQMTSLTAADTATYFCARYNNGWDYFNLWGPGTLVTVSS

SEQ ID NO: 74 - protein, 108 aa, Oryctolagus cuniculus
QSVEESGGRLVTPGTPLTLTCTVSGFSLIAYGVNWVRQAPGKGLQWIGSISNSGGTYYASWAKGRFTVSKTSTTVDLRITSPTTEDTATYFCGRGSLWGPGTLVTVSS

SEQ ID NO: 75 - protein, 124 aa, Oryctolagus cuniculus
QEQLVESGGGLVQPEGSLTLTCTASGFTISNSYYMCWVRQAPGKGLEWIGCIDAGSVGDTSYATWAKGRFTISKTSSTTVTLQMTSLTAADTATYFCARRYGAGSGYFISPNLWGPGTLVTVSS

SEQ ID NO: 76 - protein, 120 aa, Oryctolagus cuniculus
QEQLVESGGGLVQPEGSLTLTCKASGFDFSSNAMCWVRQAPGKGPEWIACIYNGDGSTYYASWVNGRFTISRSTSLNTVTLQMTSLTAADTATYFCAREYVDSQGYFNLWGPGTLVTVSS

SEQ ID NO: 77 - protein, 117 aa, Oryctolagus cuniculus
QSLEESGGRLVTPGTPLTLTCTVSGFSLSSYAMGWVRQAPGKGLEWIGIISNSGATAYASWAKGRFTISKTSSTTVDLKMTTPTTEDTATYFCARGRSGGWDAFDPWGPGTLVTVSS

SEQ ID NO: 78 - protein, 108 aa, Oryctolagus cuniculus
QSLEESGGRLVTPGTPLTLTCTVSGIDLNTNGVSWVRQAPGKGLEWIGYIFTGGNTYYASWAKGRFTISKTSTTVDLKMTSLTTADTATYFCARFDIWGPGTLVTVSL

SEQ ID NO: 79 - protein, 121 aa, Oryctolagus cuniculus
QEQLEESGGGLVKPGASLTFTCRASGFSFSSGYYMCWVRQAPGKGLEWIACIYVGITGSTYYASWAKGRFTISKTSSTSVTLQMTSLTAADTATYFCARDTGNSNYQFNLWGPGTLVTVSS

SEQ ID NO: 80 - protein, 126 aa, Oryctolagus cuniculus
QSLEESGGDLVKPGASLTLTCTASGFSFSSGYCLCWVRQAPGKGLEWIACKHGGASGTTYYATWAKGRFTISKTSSTTVTLQVTSLTVADTATYFCARDDVSVGDANYPYTAFDLWGPGTLVTVSS

SEQ ID NO: 81 - protein, 120 aa, Oryctolagus cuniculus
QSLEESGGDLVKPGASLTLTCTASGSDISSYWMCWVRQAPGKGLEWIACSYAGGSGGTYYASWAKGRFTISKTSSTTVTLQMTSLTAADTATYFCAREAYSSANSYYDLWGPGTLVTVSS

SEQ ID NO: 82 - protein, 120 aa, Oryctolagus cuniculus
QSLEESGGDLVKPGASLTLTCTASGFSFSSYYYMSWVRQAPGKGLEWIACTDGTGGITYYASWAKGRFTTSKTSPTTVTLQMTSLTAADTATYFCARDPTAAGGVYFDLWGPGTLVTVSS

SEQ ID NO: 83 - protein, 118 aa, Oryctolagus cuniculus
QEQLEESGGDLVKPEGSLTLTCTASGFDFSYNTICWVRQAPGKGLEWIAYINTGSSGTTYYASWAKGRFTISKTSSTTVTLQLNSLTAADTATYFCAGGSGYSKFRLWGPGTLVTVSS

SEQ ID NO: 84 - protein, 118 aa, Oryctolagus cuniculus
QSLEESGGDLVKPGASLTLTCTASGFSFSSSYYMCWVRQAPGKGLEWIACIYAGSSGSTYYASWAKGRFTISKTSSTTVALQMTSLTAADTATYFCARDRGDTDISLWGPGTLVTVSS

SEQ ID NO: 85 - protein, 118 aa, Oryctolagus cuniculus
QSVEESGGRLVAPGTPLTLTCTVSGFSLSNYAMSWVRQAPGKGLEYIGFINIIDSTYYTNWAKGRFTISKTSTTVDLKMTSPTTEDTATYFCARGPYYVNNENVFDPWGPGTLVTVSS

SEQ ID NO: 86 - protein, 116 aa, Oryctolagus cuniculus
QSLEESGGRLVTPGGSLTLTCTVSGIDLSNYAVGWVRQAPGKGLEYIGVINAGGSAYYATWAKGRFTISRTSTTVDLKITSPTTEDTATYFCARSYAGNRYDFAIWGPGTLVTVSL

SEQ ID NO: 87 - protein, 116 aa, Oryctolagus cuniculus
QSLEESGGDLVKPGASLTLTCTASGFSVSSSYYMCWVRQAPGKGLEWIACIYADSSGSTYYASWAKGRFTISSTSSTTVTLQMTSLTAADTATYFCARGPYSFDFWGPGTLVTVSS

SEQ ID NO: 88 - protein, 120 aa, Oryctolagus cuniculus
QSLEESGGDLVKPGASLTLTCTASGFSFSSRYYVCWVRQAPGKGLEWIACIDAGDGSTDYARWAKGRFTISKTSSTTVTLQMTGLTAADTATYFCARGDAYRDDYASDLWGPGTLVTVSS

SEQ ID NO: 89 - protein, 117 aa, Oryctolagus cuniculus
QSLEESGGRLVTPGESLTLTCTVSGIDLSANAMSWVRQAPGKGLEWIGTIFDTYLTYNANWAKGRFTISRTSTTVELKMTSPTIEDTATYFCARYIGSVGYRRMDIWGPGTLVTVAL

SEQ ID NO: 90 - protein, 118 aa, Oryctolagus cuniculus
QSVEESGGRLVTPGGSLTLTCTASGFSLNNYHMSWVRQAPGKGLEWIGFIRTDGSAFYATWAKGRFTISKTSATVDLKVTSATTEDTATYFCARMFYAGDSGHYFDLWGPGTLVTVSS

SEQ ID NO: 91 - protein, 118 aa, Oryctolagus cuniculus
QSVEESGGRLVTPGTPLTLTCTVSGFSLSNYGLTWVRQAPGKGLEWIGYINNNGRTYYASRAKGRFTISKTSTTVDLQMTSPTTEDTATYFCARNGAGGYYYSSLYIWGPGTLVTVSL

SEQ ID NO: 92 - protein, 118 aa, Oryctolagus cuniculus
QSLEESGGDLVKPGASLTLTCTASGFSFSSSYYMCWVRQAPGKGLEWIACVYAGSSGSTYYASWAKGRFTISKTSSTTVTLQMTSLTAADTATYFCARDRGGTDISLWGPGTLVTVSS

SEQ ID NO: 93 - protein, 116 aa, Oryctolagus cuniculus
QSVEESGGRLVTPGTPLTLTCKASGFSLSTYAMSWVRQAPGKGLEYIGIIDASVTTYYASWAKGRFTISKTSTTVDLTITSPTTEDTATYFCARSSSTYAYGFDPWGPGTLVTVSS

SEQ ID NO: 94 - protein, 118 aa, Oryctolagus cuniculus
QEQLKESGGGLVQPGGSLKLSCKASGFDFSNYGVSWVRQAPGKGLEWVGYIDPVFRSAYYASWVNGRFTISSHNAQNTLYLQLNSLTAADTATYFCARKGYFHYFNLWGPGTLVTVSS

SEQ ID NO: 95 - protein, 119 aa, Oryctolagus cuniculus
QSLEESGGDLVKPGASLTLTCTASGFSFSVSYWICWVRQAPGKGLEWIACIGGNSGNIYYARWAKGRFTISKTSSTTVTLQMTSLTAADTATYFCARDRAGNSYYFNLWGPGTLVTVSS

SEQ ID NO: 96 - protein, 112 aa, Oryctolagus cuniculus
QSLEESGGDLVKPGASLTLTCTASGFSFSSGYDMCWVRQAPGKGLEWIGCIYSSNGLTWYATWAKGRFTVSKTSSTTVTLQMTSLTAADTASYFCWRVWSLWGPGTLVTVSS

SEQ ID NO: 97 - protein, 119 aa, Oryctolagus cuniculus
QEQLVEYGGDLVQPEGSLTLTCKASGFDFSSNAMCWVRQAPGKGLEWIGCIVTGSGSTYYASWAKGRITISETSSTTVTLQMTSLTAADTATYFCARGYDGYGYVLVLWGPGTLVTVSS

SEQ ID NO: 98 - protein, 120 aa, Oryctolagus cuniculus
QSLEESGGDLVKPGASLTLTCTASGFSFSSSYYMCWVRQAPGKGLEWVAGVDGSGGIKWYANWAKGRFTISKTSPTTVTLQMTSLTAADTATYFCARDPTAAGGVYFDLWGPGTLVTVSS

SEQ ID NO: 99 - protein, 122 aa, Oryctolagus cuniculus
QSLEESGGDLVKPGASLTLTCTASGFSFSSSYWIYWVRQAPGKGLEWIACFHAGSGSTYYASWVNGRFTISKTSSTTVTLQMTSLTAADTATYFCARGSGSIYYTPSYFDLWGPGTLVTVSS

SEQ ID NO: 100 - protein, 108 aa, Oryctolagus cuniculus
QSVEESGGRLVTPGTPLTLTCTVSGFSLSRYGVSWVRQAPGKGLEWIAWISSSGSAYYATWAKGRFTISKTSTTVDLKITSPTTEDTATYFCGESDIWGPGTLVTVSL

SEQ ID NO: 101 - protein, 119 aa, Oryctolagus cuniculus
QSLEESGGGLVQPEGSLTLACTASGFSFNNNYYMCWVRQAPGKGLEWVACIYTGSTGSTYYANWAKGRFTISKLSSTTVTLQMTSLTAADTATYFCARDDKVEHGYGLWGPGTLVTVSS

SEQ ID NO: 102 - protein, 128 aa, Oryctolagus cuniculus
QSLEESGGDLVKPGASLTLTCTASGFSFSSNYYMCWVRQAPGKGLEWIACIYAGSSGSSYYASWAKGRFTISKTSSTTVTLQMTSLTAADTATYFCARSMEAYGYAGYAMPGYYFNLWGPGTLVTVSS

SEQ ID NO: 103 - protein, 121 aa, Oryctolagus cuniculus
QSVEESGGRLVTPGTPLTLTCTVSGFSLSSYAMSWVRQAPGKGLEWIGIIRRSGATWYANWARGRFTISKTSTTVDLKITSPTTEDTATYFCARDSDYDDYGDSYYGMDPWGPGTLVTVSS

SEQ ID NO: 104 - protein, 127 aa, Oryctolagus cuniculus
QSLEESGGDLVKPGASLTLTCTASGFSFSSSYCMCWVRQAPGKGLEWIGCIYDGSSDSAYYATWAKGRFTISKTSSTTVTLQMTSLTAADTATYFCARDYDTYDYDGYTYAAGFDLWGPGTLVTVST

SEQ ID NO: 105 - protein, 116 aa, Oryctolagus cuniculus
QSLEESGGRLVTPGTPLTLTCTVSGIDLSSYAMGWVRQAPGKGLQYIGIITYGGSTYYASWAKGRFTISKTSTTVNLKMTSLTTEDTATYFCARGLGGASTTWDIWGPGTLVTVSL

SEQ ID NO: 106 - protein, 123 aa, Oryctolagus cuniculus
QSLEESGGDLVKPGASLTLTCTASGFSFSSGYDMCWVRQAPGKGLEWIACIAVYSSGSTYYASWAKGRFTISKTSSTTVTLQMPSLTAADTATYFCARDIITDSVWITRLDLWGQGTLVTVSS

SEQ ID NO: 107 - protein, 118 aa, Oryctolagus cuniculus
QSVEESGGRLVTPGTPLTLTCTASGFSFSDYYMSWVRQAPGKGLEWIGVVSWNGNTYYASWAKGRFTVSKTSTTVDLKIISPTTEDTATYFCARFDYLVGDTYAGVLWGPGTLVTVSS

SEQ ID NO: 108 - protein, 119 aa, Oryctolagus cuniculus
QSLEESGGRLVTPGTPLTLTCTVSGIDLSSHATSWVRQAPGKGLEWIGFIKSGGSTYYASWAKGRFTISETSATVDLKITSPTTEDTATYFCASMFYAGDSSGNYLHLWGPGTLVTVSS

SEQ ID NO: 109 - protein, 121 aa, Oryctolagus cuniculus
QSLEESGGDLVKPGASLTLTCTASGFSFSSGYWICWVRQAPGKGLEWIACIDAGSNGSTYYASWARGRFTISKTSSTTVTLQMTSLTAADTATYFCAREGSSAYPSYFNFWGPGTLVTVSS

SEQ ID NO: 110 - protein, 116 aa, Oryctolagus cuniculus
QSLEESGGRLVTPGGSLTLTCTVSGIDLSSYTMAWVRQAPGKGLEYIGVINTGGSAYYASWAKGRFTISKTSTTVDLKITSPTTEDTATYFCARSYGGNRYDFNIWGPGTLVTVSL

SEQ ID NO: 111 - protein, 119 aa, Oryctolagus cuniculus
QSVEESGGRLVTPGTPLTLTCTASGFSLSSYHMCWVRQAPGKGLEWIGFIKADGNTYYATWAKGRFTISRSSATVDLKITSATAEDTATYFCARMFYAGHTSGHYFDLWGPGTLVTVSS

SEQ ID NO: 112 - protein, 130 aa, Oryctolagus cuniculus
QSLEESGGDLVKPEASLTLTCTASGFSFSGDYDMCWVRQAPGKGLEWIACIGAGSSNDTYYASWAKGRFTISKTSSTTVTLQMTSLTAADTATYFCARGFDYTYGDAGYTYSTSHYFNLWGPGTLVTVSS

SEQ ID NO: 113 - protein, 120 aa, Oryctolagus cuniculus
QSLEESGGGLVQPEGSLTLTCTASGFSFSSSYYMCWVRQAPGKGLEWIACISVGSSGSTYYANWAKGRFTISKTSSTTVTLQMTSLTAADTATYFCAREGADYQGHFNLWGPGTLVTVSS

SEQ ID NO: 114 - protein, 121 aa, Oryctolagus cuniculus
QSVEESGGRLVTPGTPLTLTCTVSGFSLSSYAMSWVRQAPGKGLEWIGIIRRSGFTYYASWARGRFTISKTSTTVDLKITSPTTEDTATYFCARDSDYDDYGNSYYGMDPWGPGTLVTVSS

SEQ ID NO: 115 - protein, 119 aa, Oryctolagus cuniculus
QSVEESGGRLVTPGTPLTLTCTVSGFSLSSYTMTWVRQAPGKGLEWIGLISRSGRTYYATWAKGRLTISKTSTTVDLKITSPTTEDTATYFCAREIGSGYDAPYYFNLWGPGTLVTVSS

SEQ ID NO: 116 - protein, 119 aa, Oryctolagus cuniculus
QSLEESGGGLVQPEGSLTLTCTASGFSFNSKYYMCWVRQAPGKGLEWIACIYTGTTGSTYYASWAKYRFTISKISSTTVTLQMTSLTAADTATYFCARDDRVEHGYGLWGPGTLVTVSS

SEQ ID NO: 117 - protein, 119 aa, Oryctolagus cuniculus
QEQLEESGGGLVKPEGSLTLTCKASGFTISSYYIYWVRQAPGKGLEWIGCIAIINSITYYANWAKGRFTISKTSSTTVTLQMTSLTAADTATYFCARDLSSSIYDMDLWGPGTLVTVSS

SEQ ID NO: 118 - protein, 121 aa, Oryctolagus cuniculus
QSLEESGGDLVKPGASLTLTCKASGLDFSSVYDMCWVRQAPGKGLEWIACIYSDGSGSTYYANWAKGRFTISETSSTTVTLQMTNLTAADTATYFCARVLNGWGEYYFNLWGPGTLVTVSS

SEQ ID NO: 119 - protein, 112 aa, Oryctolagus cuniculus
QSVEESGGRLVTPGTPLTLTCTASGFSLSSYHMSWVRQAPGKGLEYIGFIVGTGDTYYASWAKGRFTISKTSTTVDLKITSPTTEDTATYFCGRGVAAGDIWGPGTLVTVSL

SEQ ID NO: 120 - protein, 113 aa, Oryctolagus cuniculus
QSLEESGGRLVTPGTPLTLTCTASGFSLSGLVVSWVRQAPGKGLEWIGVIGKSGSTYYASWAKGRFSISKTSSTTVDLKIASPTTEDTATYFCGRNISGSAVWGPGTLVTVSL

SEQ ID NO: 121 - protein, 119 aa, Oryctolagus cuniculus
QEQLVESGGGLVQPEGSLTLTCKASGFDFNRDAMSWVRQAPGKGLEWIGSIVSGSGSTYYASWAKGRFTISETSSTTVTLQMTSLTAADTATYFCARGGDGYGYVLVLWGPGTLVTVSS

SEQ ID NO: 122 - protein, 115 aa, Oryctolagus cuniculus
QSLEESGGDLVKPGASLKLSCAASGFTLSSYWICWVRQAPGKGLEWIACIYAGSSGSTYYASWAKGRFTISKTSSTTVTLQMTSLTAADTATYFCARGISYALLWGPGTLVTVSS

SEQ ID NO: 123 - protein, 116 aa, Oryctolagus cuniculus
QSVEESGGRLVTPGTPLTLTCTVSGIDLSRYAMIWVRQAPGKGLESIGIIDIRGTTYYASWAKGRFTISKTSSTTVDLKMTSLTTEDTATYFCARGGVGHEVNNLWGPGTLVTVSS

SEQ ID NO: 124 - protein, 121 aa, Oryctolagus cuniculus
QSLEESGGDLVKPGASLTLTCTASGFSFSNNYWICWVRQAPGKGLEWIACIVAGSSGRTYYANWAKGRFTISKTSSTTVTLQMTSLTAADTATYFCARKLSDWDYGYFNLWGPGTLVTVSS

SEQ ID NO: 125 - protein, 127 aa, Oryctolagus cuniculus
QSLEESGGDLVKPGASLTLTCTASGIDFSTYYYMCCVRQAPGKGLEWIACIHAGSSGSTYYASWAKGRFTISKTSSTTVTLQMTSLTAADTATYFCARGYAGYYGYGYPTPSWLDLWGQGTLVTVSS

SEQ ID NO: 126 - protein, 119 aa, Oryctolagus cuniculus
QSVEESGGRLVTPGTPLTLTCKASGFSLSSYWMSWVRQAPGEGLEWIGTINAASGATWYASWAKGRFTISKTSTTVDLKMTSLTTEDTATYFCARGGTTGSNYYGMDPWGPGTLVTVSS

SEQ ID NO: 127 - protein, 109 aa, Oryctolagus cuniculus
QSVEESGGRLVTPGTPLTLTCTVSGIDLSRNAASWVRQAPGKGLEWIGIISTGGSTYYATWAKGPFTISKTSTTVDLKMTSLTTEDTATYFCVVGIRFWGPGTLVTVSS

SEQ ID NO: 128 - protein, 122 aa, Oryctolagus cuniculus
QSVEESGGRLVTPGTPLTLTCTVSGFSLSNYAMTWVRQAPGKGLEWIGIIINTGYTYYASWAKGRFTISKASTTVDLKITSPTTEDTATYFCARVLGAGSSYYTSYDRLDLWGQGTLVTVSS

SEQ ID NO: 129 - protein, 116 aa, Oryctolagus cuniculus
QSLEESGGRLVTPGTPLTLTCTVSGIDLISNAISWVRQAPGKGLEWIGHSDIRGSAYYASWAKGRFTISRTSSTTVDLKMTSLTTEDTATYFCARIADVNTQLDLWGQGTLVTVSS

SEQ ID NO: 130 - protein, 120 aa, Oryctolagus cuniculus
QSLEESGGDLVKPGASLTLTCAASGFSFSVGYYMCWVRQAPGKGLEWVACIYAGSNGSTYYASWAKGRFTFSKPSSTTVTLQMTSLTAADTATYFCARGAGYAGYGFNLWGPGTLVTVSS

SEQ ID NO: 131 - protein, 125 aa, Oryctolagus cuniculus
QEQLVESGGGLVKPEGSLTLTCTASGFSFSSSYWICWVRQAPGKGLEWIACIYADGSGSIYCATWAKGRFTISKTSSTTVTLQMTSLTAADTATYFCSRGNAGSYWDIYYGMDLWGPGTLVTVSS

SEQ ID NO: 132 - protein, 118 aa, Oryctolagus cuniculus
QSLEESGGDLVKPGASLTLTCTASGFSFSSSYYMCWVRQAPGKGLEWIACIYIGDGNTYYASWAKGRFTISKTSSTTVTLQMTSLTAADTATYFCARGSGGYFVDNLWGPGTLVTVSS

SEQ ID NO: 133 - protein, 118 aa, Oryctolagus cuniculus
QSVEESGGRLVTPGTPLTLTCTASGFDINNYHMTWVRQAPGKGLEWIGFIKAGGSAGYASWAKGRFTISKTSATVDLRITGATTEDTGTYFCVRMFYAGDSGHYFDLWGPGTLVTVSS

SEQ ID NO: 134 - protein, 118 aa, Oryctolagus cuniculus
QSVEESGGRLVTPGTPLTLTCTVSGFSLSSYDMTWVRQAPGKGLEWIGVISSSDSTYYASWAKGRFTISKPSSTTVDLKVTSPTTEDTATYFCARDHPAFSTVDLDIWGPGTLVTVSL

SEQ ID NO: 135 - protein, 121 aa, Oryctolagus cuniculus
QEQLVESGGGLVKSGASLTLTCTASGFSLSSSYCVCWVRQAPGKGLEWIACIYGGSSGGTYYASWAKGRITISKTSSTTVTLQMTSLTAADTATYFCARDAGSSGYYINLWGPGTLVTVSS

SEQ ID NO: 136 - protein, 118 aa, Oryctolagus cuniculus
QSLEESGGDLVKPGASLTLTCTASGFSFSSNAMCWVRQAPGKGPEWIGCIYTSSSGSTYYASWVNGRFTISKTSSTTVTLQMTSLTVADTATYFCARYNNGWDYFNLWGPGTLVTVSS

SEQ ID NO: 137 - protein, 121 aa, Oryctolagus cuniculus
QEQLVESGGGLVKPGASLTLTCTASGFSFNGNYYMCWVRQAPGKGLEWIACIYADNSGSTYYASWAKGRFTISKTSSTTVTLQMTSLTAADPATYFCVRHKPAGGSSYILWGPGTLVTVSS

SEQ ID NO: 138 - protein, 112 aa, Oryctolagus cuniculus
QSLEESGGRLVTPGTPLTLTCTVSGIDLSSYHMNWVRQAPGKGLEWIGVIYGSGSTDYASWAKGRFTISKTSTTVDLKITSPTTEDTATYFCARGILVSNLWGPGTLVTVSS

SEQ ID NO: 139 - protein, 116 aa, Oryctolagus cuniculus
QSLEESGGDLVKPGASLTLTCTASGFTISSSYYMCWVRQAPGKGLEWIACIYSDSSGSTYNANWVKGRFTISKTSSTTVTLRMTSLTAADTATYFCARGTYPFTLWGPGTLVTVSS

SEQ ID NO: 140 - protein, 118 aa, Oryctolagus cuniculus
QSVEESGGRLVTPGTPLTLTCTVSGFSLSSYPVNWVRQAPGKGLEWIGVIGNRGSTDYASWAKGRFTISKTSTTVDLKITSPTTEDTATYFCARGSGYGTGWDAFDPWGPGTLVTVSS

SEQ ID NO: 141 - protein, 114 aa, Oryctolagus cuniculus
QSLKESGGGLVTPGTPLTLTCKVSGFSLSSYDMSWVRQAPGKGLEWIGTIYDGGSTYYASWTKGRFTISKASTTVDLKITSPTTEDTATYFCARGSTNMEFWFWGPGTLVSVSS

SEQ ID NO: 142 - protein, 119 aa, Oryctolagus cuniculus
QSVEESGGRLVTPGTPLTLTCTVSGFSLNNYGMTWVRQAPGKGLEWIGIINIIDNTYYASWAKGRFTISKTSTTVDLKITSPTTEDTATYFCARADYYPDTTGWYLNIWGPGTLVTVSL

SEQ ID NO: 143 - protein, 113 aa, Oryctolagus cuniculus
QSVEESGGRLVTPGTPLTLTCTVSGFSLSTYWMSWVRQAPGKGLEWIGTISTGGSAYYASWAKSRFTISKTSTTVDLKITSPTTEDTATYFCARDGDSYFKLWGPGTLVTVSS

SEQ ID NO: 144 - protein, 115 aa, Oryctolagus cuniculus
QSLEESGGRLVTPGTPLTLTCTVSGIDLSSYAMGWVRQAPGKGLEYIGYINRGNTYYANWAKGRFTISKTSTTVDLKITSPTTEDTATYFCARDSYGGDYAFNLWGPGTLVTVSS

SEQ ID NO: 145 - protein, 121 aa, Oryctolagus cuniculus
QSLEESGGGLVKPGASLTLTCTASGFSFSSSYYMCWVRQAPGKGLEWIACIHAGSSGSAYYASWAKGRFTISKTSSTTVTLQMTSLTAADTATYFCARDGYDDYGDPFNLWGPGTLVTVSS

SEQ ID NO: 146 - protein, 126 aa, Oryctolagus cuniculus
QSLEESGGDLVKPGASLTLTCTASGFSFSSGQDMCWVRQAPGKGLEWIACIYGGDGNTYYASWAKGRFTIYKTSSTTVTLKMTSPTAADTATYLCARLHYSPYGDAGYPYVSFNLWGPGTLVTVSS

SEQ ID NO: 147 - protein, 114 aa, Oryctolagus cuniculus
QSVEESGGRLVTPGTPLTLTCTASGFSLSSYNMGWVRQAPGKGLEWIGYIWSGGSAYYASWAKGRFTISRTSTTVTLKMTSLTAADTATYFCARNGASGTFDIWGPGTLVTVSL

SEQ ID NO: 148 - protein, 121 aa, Oryctolagus cuniculus
QEQLVESGGGLVQPEGSLTLTCTASGFSFSSSYYMCWVRQAPGKGLEWIACIYAGSSGSTYYASWAKGRLTISKISSTTVTLQMTSLTAADTATYFCARGGGSGGVDNNLWGPGTLVTVSS

SEQ ID NO: 149 - protein, 113 aa, Oryctolagus cuniculus
AQVLTQTPSSVSAAVGGTVTINCQASQSLYNNKNLAWYQQKLGQPPKLLIYDVSTLASGVPSRFKGSGSGTQFTLTISGVQCDDAATYYCQGEFSCSSGDCYAFGGGTEVVVK

SEQ ID NO: 150 - protein, 110 aa, Oryctolagus cuniculus
AQVLTQTASSVSAVVGGTVTISCQSSQSVYDKKWLGWYQQKPGQPPKLLIYKASTLASGVPSRFKGSGSGTQFTLTISDLECDDAATYYCAGGYSGNIWSFGGGTEVVVK

SEQ ID NO: 151 - protein, 113 aa, Oryctolagus cuniculus
AQVLTQTPSSVSAAVGGTVTIICQASQSLYNNKNLAWYQQKLGQPPKLLIYDVSTLASGAPSRFKSSGSGKQFTLTISGVQCDDAATYYCQGEFSCSSGDCYAFGGGTEVVVK

SEQ ID NO: 152 - protein, 110 aa, Oryctolagus cuniculus
AQVLTQTASPVSAAVGDTVTISCQSSESVYNNNLLSWYQQKPGQPPKLLIYTTSSLASGVPSRFKGSGSGTQFTLTISGVQCDDAATVYCQGGYTDATYAFGGGTEVVVK

SEQ ID NO: 153 - protein, 104 aa, Oryctolagus cuniculus
DIVMTQTPSSVSAAVGGTVTINCQASQSVSNLLAWYQQKPGQPPKLLIYGASNLESGVPSRFRGSGSGTEFTLTISGMKAEDAATYYCQSGYYTFGAGTKVEIK

SEQ ID NO: 154 - protein, 113 aa, Oryctolagus cuniculus
AQVLTQTPSSVSAAVGGTVTINCQASQSLYNNKNLAWYQQKPGQPPKLLIYDASTLASGVPSRFKGSGSGTQFTLTISGVQCDDAATYYCQGEFSCGSGDCYAFGGGTEVVVK

SEQ ID NO: 155 - protein, 110 aa, Oryctolagus cuniculus
DPVLTQTPSSASEPVGGTVTIKCQASEDIESYLAWYQQKPGQPPKLLIYDASDLASGVPSRFKGSGSGTQFTLTISGVQCADAATYYCQSYYYGSSYVVAFGGGTEVVVK

SEQ ID NO: 156 - protein, 113 aa, Oryctolagus cuniculus
AQVLTQTPSSVSAAVGGTVTINCQASQSLYNNKNLGWYQQKLGQPPKLLIYDVSTLASGVPSRFKGSGSGTQFTLTISDLECDDAATYYCQGEFSCSSGDCYAFGGGTEVVVK

SEQ ID NO: 157 - protein, 111 aa, Oryctolagus cuniculus
DIVMTQTPASVEAAVGGSVTIKCQASQTISSYLAWYQQKPGQPPKLLIYGASTLASGVPSRFSGSGSGTEYTLTISGVQCDDAATYYCLYSYYTSNSADNTFGGGTEVVVK

SEQ ID NO: 158 - protein, 111 aa, Oryctolagus cuniculus
AAVLTQTPSPVSAAVGGTVSISCQSSQSVYDNNALAWYQQKPGQPPKLLIYETSTLASGVPSRFEGSGSGTQFTLTISDVQCDDAATYYCAGGYNSGSDAAFGGGTEVVVK

SEQ ID NO: 159 - protein, 110 aa, Oryctolagus cuniculus
AQVLTQTPSPVSAPVGGTVTISCQSSQNVDRNNRLAWYQQKLGQPPKLLIYYASILASGVPSRFKGSGSGTQFTLTINELQCDDAATYYCQGYYSGDINVFGVGTEVVVK

SEQ ID NO: 160 - protein, 111 aa, Oryctolagus cuniculus
DIVMTQTPASVEAAVGGTVTIKCQASQSIGSNLAWYQQKPGQPPKLLIYKASTLASGVPSRFKGSGSGTEFTLTISDLECADAATYYCQSYYGTSNSYGDAFGGGTEVVVK

SEQ ID NO: 161 - protein, 111 aa, Oryctolagus cuniculus
DVVMTQTPASVSEPVGGTVTIKCQASEDIESYLAWYQQKPGQPPKLLIYQASKLASGVSSRFSGSGYGTEFTLTLSDLECADAATYYCQCTLYGVNFVPNVFGGGTEVVVK

SEQ ID NO: 162 - protein, 111 aa, Oryctolagus cuniculus
DVVMTQTPASVSEPVGGTVTIKCQASEDIESYLAWYQQKPGQPPKLLIYSASTLASGVSSRFKGSGSGTEFTLTISDLECADAATYYCQCILYGVNFVPNTFGGGTEVVVK

SEQ ID NO: 163 - protein, 111 aa, Oryctolagus cuniculus
DVVMTQTPASVSAAVGGTVTIKCQASQNIYDNLAWYQQKPGQRPKLLIYGASNLESGVPSRFKGSGSGTEYTLTISDLECADAATYYCQCSYDGGSYVPNAFGGGTEVVVQ

SEQ ID NO: 164 - protein, 111 aa, Oryctolagus cuniculus
AAVLTQTPSPVSAAVGGTVSISCQSSPSVYNNNRLSWFQQKPGQPPKLLIYYASTLASGVPSRFKGSGSGTQFTLTISDVQCDDAATYYCAGGYSTISDNAFGGGTEVVVK

SEQ ID NO: 165 - protein, 110 aa, Oryctolagus cuniculus
DVVMTQTPASVSEPVGGTVTIKCQASQNIGNNLAWYQQKPGQPPKLLIDYASTLASGVPSRFKGSGSGTQFTLAISDLDCADAATYYCQCTFYGSGYVAAFGGGTEVVVK

SEQ ID NO: 166 - protein, 111 aa, Oryctolagus cuniculus
DVVMTQTPASVSEPVGGTVSINCQASEDIESYLAWYQQKPGQPPKLLIYGASNLASGVSSRFKGSGSGTEYTLTISDLECDDAATYYCQCGIYGVNFVPNVFGGGTEVVVK

SEQ ID NO: 167 - protein, 110 aa, Oryctolagus cuniculus
AYDMTQTPASVEVGVGGTVTIKCQASQNINSWLSWYQQKPGQPPKLLIYKASTLASGVSSRFKGSGSGTEFTLTISDLECADAATYYCQQGAGWNNLDNAFGGGTEVVVK

SEQ ID NO: 168 - protein, 111 aa, Oryctolagus cuniculus
AQVLTQTPSSVSAAVGGTVTINCQSSQSVYSNNHLAWYQQKPGQPPNLLIYRASKLASGVPSRFSGSRSGTQFTLTISGVQCDDAATYYCLGVYDDDADNAFGGGTEVVVK

SEQ ID NO: 169 - protein, 112 aa, Oryctolagus cuniculus
AVVMTQTASPVSAAVGGTVTINCQSSQIVHNNNNLAWYQLKPGQPPKLLIFQASTLASGVPSRFKGSGSGTQFTLTISDLECDDAAAYYCAGGYSTNTDTYIFGGGTEVVVR

SEQ ID NO: 170 - protein, 113 aa, Oryctolagus cuniculus
AQVLTQTPSSVSAAVGGTVTINCQASQSLYNKKNLAWYQQKLGQPPKLLIYDASTLTSGVSSRFKGSGSGTQFTLTISGVQCDDAATYYCQGEFSCSAGDCYAFGGGTELVVK

SEQ ID NO: 171 - protein, 110 aa, Oryctolagus cuniculus
AQVLTQTASSVSAVVGGTVTISCQSSQSVYDNKWLGWYQQKPGQPPKLLIYSASTLASGVPSRFKGSGSGTHFTLTISDLECDDATTYYCAGGYSGNIWSFGGGTEVVVK

SEQ ID NO: 172 - protein, 110 aa, Oryctolagus cuniculus
AQVLTQTPSPVSAAVGGTVTISCQSSQSVYDNKWLGWYQQKPGQPPKLLIYKASTLASGVPSRFKGSGSGTQFTLTISDLECDDATTYYCAGGYSGNIWSFGGGTEVVVK

SEQ ID NO: 173 - protein, 111 aa, Oryctolagus cuniculus
AAVLTQTPASVSAAVGGTVTISCQSSKSVFDNNWLSWFQQKPGQPPKLLIYKASTLASGVPSRFKGSGSGTQFTLTISDVQCDDAATYYCAGIYSSDSDNAFGGGTEVVVK

SEQ ID NO: 174 - protein, 113 aa, Oryctolagus cuniculus
AQVLTQTPSSVSAVVGGTVTINCQASQSLYNKKNLAWYQQKLGQPPKLLIYDASTLASGVPSRFKGSGSGTQFTLTISGVQCDDAASYYCQGEFSCSSGDCYAFGGGTELVVK

SEQ ID NO: 175 - protein, 110 aa, Oryctolagus cuniculus
AYDMTQTPFSVSAAVGGTVTINCQASETIYSYLNWYQQKPGQPPKLLIYSASTLASGVPSRFKGSGSGTQFTLTISGVECADAATYYCQQGYSGRNVENTFGGGTEVVVK

SEQ ID NO: 176 - protein, 111 aa, Oryctolagus cuniculus
AAVLTQTPSPVSAAVGGTVTISCQSSQNIYNKNQLSWFQQKPGQPPKLLIYEASKLASGVPSRFKGSGSGTQFTLTISDVQCDDAATYYCLGGYISSSDTTFGGGTEVVVK

SEQ ID NO: 177 - protein, 110 aa, Oryctolagus cuniculus
DVVMTQTPASVSTAVGGTVTIKCQASQSIGGSLAWYQQKPGQPPNLLIYSASNLASGVSSRFKGSRSGTEFTLTISDLECADAATYYCQCTYYDDSYDVPFGGGTEVVVK

SEQ ID NO: 178 - protein, 112 aa, Oryctolagus cuniculus
AAVLTQTPSPVSAAVGGTVTISCQSSQSVNNNKNLAWYQQKLGQPPKLLIYDTSTLASGVPSRFKGSGSGTQFTLTISDLECDDATTYYCAGGYSSSADTFAFGGGTEVVVR

SEQ ID NO: 179 - protein, 112 aa, Oryctolagus cuniculus
DIVMTQTPASVSAAVGGTVTIKCQASQNIGSTLAWYQQKPGQPPKRLIYGASTLSSGVPSRFKGSGSGTDFTLTISDLECADAATYYCQSNYGSNSGGYVFPFGGGTEVVVK

SEQ ID NO: 180 - protein, 111 aa, Oryctolagus cuniculus
DVVMTQTPASVSEPVGGTVTIKCQASEDIETYLAWYQQKPGQPPKLLIYRASTLASGVPSRFKGSGSGTQFTLTISDLECADAATYYCQCTLYGVNFVANAFGGGTEVVVK

SEQ ID NO: 181 - protein, 109 aa, Oryctolagus cuniculus
AFELTQTPSSVSAAVGGTVTINCQASEDIENYLAWYQQKPGQPPKLLIYSASTLASGVSSRFKGSGSGTEYTLTISDLGCADAATYYCQSYYDGAVTFTFGGGTEVVVK

SEQ ID NO: 182 - protein, 112 aa, Oryctolagus cuniculus
AQVLTQTASPVSAAVGGTVTIKCQSSQSVDNNWLSWYQQKPGQPPKLLIYTTSKLASGVPSRFKGSGSGTQFTLTISDVQCDDAATYYCLGGYDSMSADCFAFGGGTEVVVK

SEQ ID NO: 183 - protein, 111 aa, Oryctolagus cuniculus
AQVLTQTPSSVSAAVGGAVTINCQSSQSVYSNNHLAWYQQKPGQPPKLLIYRASKLASGVPSRFSGSGSGTQFTLTISGVQCDDAATYFCLGVYDDDADNAFGGGTAVVVK

SEQ ID NO: 184 - protein, 112 aa, Oryctolagus cuniculus
AVVMTQTASPVSAAVGGTVTINCQSSQSVHNNNNLAWYQQKPGQPPKLLIFQASTLASGVPSRFKGSGSGTQFTLTISDLECDDAAAYYCAGGYSTNTDTFTFGGGTEVVVR

SEQ ID NO: 185 - protein, 112 aa, Oryctolagus cuniculus
ALVMTQTPASVEAAVGGTVTISCQASEDISSSLAWYQQKPGQPPNLLIYRASNLASGVPSRFKGSGSGTQFTLTISGVQCADAATYYCQAYYYSISDDLYNAFGGGTEVVVK

SEQ ID NO: 186 - protein, 112 aa, Oryctolagus cuniculus
AVVMTQTASPVSAAVGGTVTISCQASQSVHNNNNLAWYQQKPGQPPKLLIFQASTLASGVPSRFKGSGSGTEFTLTISDLECDDAAAYYCAGGYSTNTDTFTFGGGTEVVVR

SEQ ID NO: 187 - protein, 111 aa, Oryctolagus cuniculus
DVVMTQTPASVSAAVGGTVTIKCQASEDIESYLAWYQQKPGQPPKLLIYRASTLASGVPSRFKGSGSGTQFTLTISDLECADAATYYCQCTIYGVNFVPNAFGGGTEVVVK

SEQ ID NO: 188 - protein, 111 aa, Oryctolagus cuniculus
DVVMTQTPASVSAAVGGTVTIKCQATEDIESFLAWYQQKPGQPPKLLIYRASTLESGVPSRFKGSGSGTEFTLTISDLECADAATYYCQCTVYGVNFVANAFGGGTEVVVR

SEQ ID NO: 189 - protein, 108 aa, Oryctolagus cuniculus
AIKMTQTPSSVSAAVGGTVTINCRASEDIKSYLAWYQQKPGQPPKLLIYDASDLASGVPSRFKGSGSGTEYTLTISGVQCDDAATYYCQSVWYAGGAAFGGGTEVVVQ

SEQ ID NO: 190 - protein, 113 aa, Oryctolagus cuniculus
AQVLTQTASPVSAAVGGTVTINCQASQSVYNHKNLAWYQQKPGQPPKLLIYDTSTLASGVSSRFKGSGSGTQFTLTISGVQCDDAATYYCAGEFSCASADCFAFGGGTEVVVK

SEQ ID NO: 191 - protein, 110 aa, Oryctolagus cuniculus
DVVMTQTPASVSEPVGGTVTIKCQASQSIGSSLAWYQQKAGQRPKLLIYYVSNLESGVSSRFSGSGSGTEFTLTISGVQCDDAATYYCQSYGYGSGYVFAFGGGTEVVVK

SEQ ID NO: 192 - protein, 113 aa, Oryctolagus cuniculus
AQVLTQTPSPVSAAVGGTVSISCQSSQSVYGVNELSWYQQKAGQPPKLLIYKAATLASGVPSRFKGSGSGTQFTLTISDVQCDDAATYYCLGNYDCESDDCYAFGGGTEVVVK

SEQ ID NO: 193 - protein, 113 aa, Oryctolagus cuniculus
DVVMTQTPASVEAPVGGTVTIKCQASQSISNLLAWYQQIPGQSPKLLIYDASDLASGVPSRFKGSGSGTEYTLTISDLECADAATYYCQCTYGSSSSSAYGWAFGGGTEVVVK

SEQ ID NO: 194 - protein, 111 aa, Oryctolagus cuniculus
AAVLTQTPSPVSAAVGGTVSISCQSSKSVYNNNWLSWFQQKPGQPPKLLIYGASTLASGVPSRFKGSGSGTQFTLTISDVQCDDAATYYCLGSYISSSDNAFGGGTEVVVK

SEQ ID NO: 195 - protein, 111 aa, Oryctolagus cuniculus
AAVLTQTPSPVSAAVGGTVSISCQSSPSVYNNNRLSWFQQKPGQPPKLLIYYASTLASGVPSRFKGSGSGTQFTLTISDVQCDDAATYYCAGGYSSISDNGFGRGTEVVVK

SEQ ID NO: 196 - protein, 112 aa, Oryctolagus cuniculus
DVVMTQTLPSVSEPVGGTVTIKCQASQSIGSYLSWYQQKPGQPPKLLIYDASTLASGVPSRFKGGGSGTQFTLTISDLECADAATYYCQGYYYYISNTYGYPFGGGTEVVVK

SEQ ID NO: 197 - protein, 110 aa, Oryctolagus cuniculus
DVVMTQTPASVSEPVGGTVTIKCQASQNIGNNLAWYQQKPGQPPKLLMYDASDLASRVPSRFSGSGSGTEFTLTISDLECADAATYYCQCTYGYSGYVSAFGGGTEVVVK

SEQ ID NO: 198 - protein, 110 aa, Oryctolagus cuniculus
ALVMTQTPSPVSAAVGGTVTINCQASEDIYSNLAWFQQKPGQPPKLLIYSASTLASGVSSRFKGSGSGTKFTLTISGLQCDDAATYYCLGVYTYISADNAFGGGTEVVVK

SEQ ID NO: 199 - protein, 113 aa, Oryctolagus cuniculus
AQVLTQTPSSVSAAVGGTVTINCQASQSLYNNKNLAWYQQKLGQPPKLLIYDVSTLASGVPSRFKGSGSGKQFTLTISGVQCDDAATYYCQGEFSCSSGDCYAFGGGTEVVVK

SEQ ID NO: 200 - protein, 111 aa, Oryctolagus cuniculus
AAVLTQTPSPVSAAVGGTVSISCQSSKTVYNNNWLAWFQQKPGQPPKLLIYGASTLASGVPSRFKGSGSGTQFTLTISDVQCDDAATYYCLGSYISSSDNGFGGGTEVVVK

SEQ ID NO: 201 - protein, 111 aa, Oryctolagus cuniculus
AAVLTQTPSPVSAAVGGTVTISCQSSPSVYNNVRLSWFQQKPGQPPKLLIYSASTLASGVPSRFKGSGSGTQFTLTISDVQCDDAATYYCAGGYSDISDNAFGGGTEVVVK

SEQ ID NO: 202 - protein, 112 aa, Oryctolagus cuniculus
AQVLTQTPSSVSAAVGGTVTISCQSSQSVYSTNLAWYQQKPGQPPKLLIDYASTLASGVPSRFKGSGSGTQFTLTISGVQCDDAAAYYCQGEFNCGSGDCSTFGGGTEVVVK

SEQ ID NO: 203 - protein, 110 aa, Oryctolagus cuniculus
DVVMTQTPASASAAVGGTVTINCQASENIANHLAWYQQKPGQPPKLLIYSASALASGVPSRFKGSGSGTEFALTISDLECDDAAIYYCQCTFWDINNFGGFGGGTEVVVK

SEQ ID NO: 204 - protein, 111 aa, Oryctolagus cuniculus
AAVLTQTPSPVSAAVGGTVTIKCQSSQSVYGNNELSWYQQKPGQPPKLLIYDASKLASGVPHRFSGSGSGTQFTLTISGVQCDDAATYYCLGGYDADADNAFGGGTEVVVK

SEQ ID NO: 205 - protein, 113 aa, Oryctolagus cuniculus
AQVLTQTPSSVSAAVGGTVTINCQASQSLYNKKNLAWYQQKLGQPPKLLIYDVSTLASGVPSRFKGSGSGTQFTLTISDLECGDAAAYFCQGEFSCSSGDCYAFGGGTEVVVK

SEQ ID NO: 206 - protein, 110 aa, Oryctolagus cuniculus
AQVLTQTASSVSAAVGGSVTISCQSSQSVYGSDALAWFQQRPGQSPKRLIYGASTLASGISSRFKGSGSGTQFTLTISDLECDDAATYFCAGAYSGNVGTFGGGTEVVVK

SEQ ID NO: 207 - protein, 110 aa, Oryctolagus cuniculus
AYDMTQTPASVEVAVGGTVTIKCQASQSISSNLAWYQQKSGQPPKLLIYLASTLASGVPSRFKGSGSGTEFTLTISDLECADAATYYCQQTYSGSNVENSFGGGTEVVVK

SEQ ID NO: 208 - protein, 111 aa, Oryctolagus cuniculus
AIDMTQTPSPVSAAVGDTVTINCQASENIYSFLAWYQQKPGHSPKLLIYSASTLESGVPSRFKGSGSGTQFTLTISDVQCDDAATYYCQQTYIYNNAEDNTFGGGTEVVVK

SEQ ID NO: 209 - protein, 112 aa, Oryctolagus cuniculus
DVVMTQTPASVEAAVGGTVTIKCQASQSISDYLSWYQQKPGQPPKLLIYRASNLASGVPSRFKASESGTEFTLTISDLECADAATYYCQCTFGATNDDYGNAFGGGTEVVVK

SEQ ID NO: 210 - protein, 113 aa, Oryctolagus cuniculus
DIVMTQTPASVEAAVGGTVTIKCQASQSISSYLSWYQQKPGQPPKLLIYDASDLASGVSSRFKGSGSGTEFTLTISDLECADAATYYCQCTVGSSGVTGYGNAFGGGTEVVVK

SEQ ID NO: 211 - protein, 112 aa, Oryctolagus cuniculus
DPVMTQTPASVSEPVGGTVTIKCQASQNINNLLAWYQQKPGQPPKLLIYKASTLASGVSSRFKGSGSGTEFTLTISDLECADAATYYCQNYYGYGLSTNYVVFGGGTEVVVK

SEQ ID NO: 212 - protein, 113 aa, Oryctolagus cuniculus
AQVLTQTPSSVSAAVGGTVTINCQASQSVYANNYLAWYQQKPGQPPKLLIYKASTLASGVPSRFSGSGSGTQFTLTINGVQCDDAATYYCQGEFSCSSGDCTAFGGGTEVVVK

SEQ ID NO: 213 - protein, 112 aa, Oryctolagus cuniculus
DVVMTQTPASVEAAVGGTVTIKCQASESISNYLSWYQQKPGQPPKLLICYDSTLESGVPSRFKGSGSGTDFTLTISDLECADAATYYCQCTAGSINVSYGNAFGGGTEVVVK

SEQ ID NO: 214 - protein, 113 aa, Oryctolagus cuniculus
AQVLTQTASPVSEPVGGTVTIKCQSSQSVYNNNWLSWFQQKPGQPPKRLIYGASTLASGVPSRFKGSGSGTHFTLTISDVQCDDAATYYCLGSYDCSSVDCNAFGGGTEVVVK

SEQ ID NO: 215 - protein, 112 aa, Oryctolagus cuniculus
AAVLTQTPSPVSAAVGGTVTISCQASQSVHKHKNLAWYQQKPGQPPKLLIYEASKLASGVPPRFSGSGSGTQFTLTMSDLECDDAATYYCAGGYDSTIDTFTFGGGTEVVVK

SEQ ID NO: 216 - protein, 113 aa, Oryctolagus cuniculus
DVVMTQTPASVEAAVGGTVTIKCQASQSISSYLSWYQQKPGQPPKLLIYRASSLKSGVPSRFKGTGSGTEFTLTISDLECADAATYYCQCTYGSSTSSRSGNAFGGGTEVVVT

SEQ ID NO: 217 - protein, 113 aa, Oryctolagus cuniculus
DIVMTQTPASVEAAVGGTVTIKCQASQNINNELSWYQQKPGQPPKLLIYKASTLASGVPSRFKGSGSGTQFTLTISDLECADAATYYCQSYYYGISSTYAFYTFGGGTEVVVK

SEQ ID NO: 218 - protein, 110 aa, Oryctolagus cuniculus
DVVMTQTPASASAAVGGAVTIKCRASEDIESYLAWYQQKPGQPPKLLIYSASSLASGVPSRFKGSGSGTEFTLTISDLECDDAATYYCQCTYWDSSTVGAFGGGTAVVVK

SEQ ID NO: 219 - protein, 111 aa, Oryctolagus cuniculus
AAVLTQTPSPVSAAVGGTVSISCQSSQSVYNDNDLAWFQQKPGQPPKLLIYGASTLASGVPSRFKGSGSGTQFTLTISGVQCDDAATYYCSGGYISSSDNAFGGGTEVVVK

SEQ ID NO: 220 - protein, 109 aa, Oryctolagus cuniculus
DVVMTQTPASVSAAVGGTVTIKCQASESIYSGLAWYQQKPGQPPKLLIYRASTLESGVSSRFKGSGSGTQFTLTISDLECADAATYYCQSTYYGSSGNAFGGGTEVVVK

SEQ ID NO: 221 - protein, 111 aa, Oryctolagus cuniculus
DIVMTQTPASVSAAVGGTVTINCQASQSISYYLNWYQQKPGQPPKLLIYRASTLASGVPSRFSGSGSGTQFTLTISGVQCDDAATYYCLYGYVTSSNADFAFGGGTEVVVE

SEQ ID NO: 222 - protein, 113 aa, Oryctolagus cuniculus
AQVLTQTPSSVSAAVGDTVTINCQASQSVYKNNYLAWFQQKPGQPPKRLIYSASTLDSGVSSRFKGSGSGTQFTLTISDVQCDDAATYYCLGTYDCVSADCGAFGGGTEVVVK

SEQ ID NO: 223 - protein, 112 aa, Oryctolagus cuniculus
AQVLTQTASSVSAAVGGTVTISCQSSQSVYNNNWLGWYQQKPGQPPKLLIYSASTLASGVPSRFKGSGSGTQFTLTISGVQCYDAATYYCQGTYSNNGWYFAFGGGTEVVVK

SEQ ID NO: 224 - protein, 113 aa, Oryctolagus cuniculus
DIVMTQTPASVSEPVGGTVTIKCQASEDIYNLLAWYHQKPGQPPKLLIYGASTLASGVPSRFKGSGSGTQFTLTISDLECADAATYYCQSYYYGISSTYAFYTFGGGTEVVVE

SEQ ID NO: 225 - protein, 109 aa, Oryctolagus cuniculus
AFELTQTPSSVSAAVGGTVTINCQASEDIESYLAWYQQKPGQPPKFLIYGASTLASGVPSRFKGSGSGTEYTLTISDLECADAATYYCQTYYGGINIFTFGGGTEVVVE

SEQ ID NO: 226 - protein, 113 aa, Oryctolagus cuniculus
AQVLTQTASPVSAAVGSTVTINCQASQSVYSNNYLSWFQQKPGQPPKLLIYDASDLASGVPSRFKGSGSGTQFTLTISDLECDDAATYYCLGTYDCSSTDCYAFGGGTEVVVK

SEQ ID NO: 227 - protein, 111 aa, Oryctolagus cuniculus
DVVMTQTPASVSEPVGGTVSLKCQASESIDSYLNWYQQKPGQPPKLLIYGASTLASGVSSRFKGSRSGTEYTLTISDLECADAATYYCQCTVYGVNFVPNAFGGGTEVVVK

SEQ ID NO: 228 - protein, 110 aa, Oryctolagus cuniculus
ALVMTQTPSSVSAAVGGTVTINCQASQNIYSSLAWYQQKPGQPPKLLIYGASNLESGVPSRFKGSGSGTEFTLTISALECDDAATYYCQGGYYISSTDNAFGGGTEVVVK

SEQ ID NO: 229 - protein, 110 aa, Oryctolagus cuniculus
AYDMTQTPASVEAVVGGSVTIKCQASQSISYYLAWYQQKPGQRPKLLIYRASTLASGVPSRFKGSGSGTEYTLTISDLECADAATYYCQQGYSSSNVDNAFGGGTEVVVK

SEQ ID NO: 230 - protein, 110 aa, Oryctolagus cuniculus
AFELTQTPSSVSAAVGGTVTIKCQASQNIYSRLAWYQQKPGQRPKLLIYAASTLASGVPSRFKGNGSGTEFTLTISDLECADAATYYCQGGYYGSSDTVTFGGGTEVVVK

SEQ ID NO: 231 - protein, 111 aa, Oryctolagus cuniculus
AAVLTQTPSPVSAAVGGTVTISCQSSQSVTDNFLSWFQQKPGQRPKLLIYGASTLASGVPSRFKGSGSGTQFTLTISDVQCDDAATYYCAGGYSGSSDVFAFGGGTEVVVK

SEQ ID NO: 232 - protein, 111 aa, Oryctolagus cuniculus
AYDMTQTPSSVSAAVGGTVTINCQASEDIESYLAWYQQKPGQPPKLLIYSASTLASGVPSRFKGSGSGTQFTLTISDLECADAATYYCQCTVYGVNYVPNAFGGGTEVVVK

SEQ ID NO: 233 - protein, 110 aa, Oryctolagus cuniculus
DVVMTQTPASVSAAVGGTVTIKCQASQSIGSSLAWYQQKPGQSPKLLIYSASNLASGVSSRFKGSGSGTEYTLTISDLECADAATYYCQCTYYGGSGDVPFGGGTEVVVK

SEQ ID NO: 234 - protein, 112 aa, Oryctolagus cuniculus
DIVMTQTPASVEAAVGGTVTIKCQASQSISSYLAWYQQKPGQPPKLLIYRTSILESGVPSRFKGSGSGTEFTLTISDLECADAATYYCQCTYGTTNTGHYVGFGGGTEVVVK

SEQ ID NO: 235 - protein, 109 aa, Oryctolagus cuniculus
DVVMTQTPASVSEPVGGTVTIKCQASQNIGSDLAWYQQKPGQRPKLLIYDASALASGVPSRFSGSGSGTEFTLTISGVQCDDSATYYCQCTYYSGSPHTFGGGTEVVVK

SEQ ID NO: 236 - protein, 114 aa, Oryctolagus cuniculus
DIVMTQTPASVEAAVGGTVTIKCQASQSISSYLAWYQQKPGQPPKLLIYRASTLASGVPSRFKGSGSGTEFTLTISDLECADAATYYCQSNYGSSSISNYGGGAFGGGTEVVVK

SEQ ID NO: 237 - protein, 110 aa, Oryctolagus cuniculus
AQVLTQTPASVSAAVRGTVTIKCQASESVVGKNELSWYHQKPGQPPKLLIFGTSTLASGVPSRFSGSGSETQFTLAISDLECGDAATYYCAGGYSGNMYVFGGGTEVVVK

SEQ ID NO: 238 - protein, 112 aa, Oryctolagus cuniculus
AAVLTQTPSPVSAAVGGTVTISCQASQSVHNNKNLAWYQQKPGQPPKLLIYDVSTVASGVPSRFKGSGSGTQFTLTISDLECDDAATYYCAGGYGSYTDTFAFGGGTEVVVK

SEQ ID NO: 239 - protein, 111 aa, Oryctolagus cuniculus
AAVLTQTPSPVSAAVGGTVTIKCQSSQSVYRNNELSWYQQKPGQPPKVLVYDASNLASGVPDRFSGSGSGTQFTLTISGVQCDDAATYYCLGGYDDDADNTFGGGTEVVVK

SEQ ID NO: 240 - protein, 111 aa, Oryctolagus cuniculus
DVVMTQTPASVSEPVGGTVTIKCQASEDIESFLAWYQQKPGQPPKLLIYSASTLASGVPSRFKGSGSGTQFTLTIGDLECADAATYFCQCTIYGVNFVPNAFGGGTEVVVK

SEQ ID NO: 241 - protein, 110 aa, Oryctolagus cuniculus
DVVMTQTPASVSEPVGGTVTIKCQASEDISSRLAWYQQKPGQPPKLLIYRASTLASGVPSRFKGSGSGPEYTLTISDLECADAATYYCQSNYAIISCGAAFGGGTEVVVK

SEQ ID NO: 242 - protein, 110 aa, Oryctolagus cuniculus
ALVMTQTPSSVSAAVGGTVTINCQASQNIYSNLAWYQQKPGQRPKLLIYGASNLESGVPSRFKGSGSGTEFTLTISDLECDDAATYYCQSAYYSSSAVYAFGGGTEVVVK

SEQ ID NO: 243 - protein, 111 aa, Oryctolagus cuniculus
AIDMTQTPSSVSAAVGDTVTINCQASENIYSFLAWYQQKPGQRPKLLIYDSSTLASGVPSRFSGSGSGTEFTLTISGIQCDDAATYYCQQTYIYNNAESNAFGGGTEVVVK

SEQ ID NO: 244 - protein, 110 aa, Oryctolagus cuniculus
AQVLTQTPSPVSAAVGGTVTINCQSSQSVADNNLLAWYQQKPGQPPKLLIYKASTLASGVPSRFKGSGYGTQFTLTISDLECDDAATYYCVGGYSTSGYAFGGGTEVVVK

SEQ ID NO: 245 - protein, 113 aa, Oryctolagus cuniculus
AQVLTQTPSPVSAAVGGTVTINCQASQSVYGTNRLAWYQQKPGQPPKLLIYDASTLASGVPSRFSGSGSGTQFTLTISGVQCDDAATYCCQGEFSCSNGDCIAFGGGTEVVVK

SEQ ID NO: 246 - protein, 110 aa, Oryctolagus cuniculus
AFELTQTPSSVSAAVGGTVTIKCQASQNIYSKFAWYQQKPGQRPKLLIYSASTLASGVPSRFKGNGSGTEFTLTISDLECADAATYYCQGGYYGSSDTVTFGGGTEVVVK

SEQ ID NO: 247 - protein, 110 aa, Oryctolagus cuniculus
AYDMTQTPASVEVALGGTVTIKCQASQSIGVSLAWYQQKPGQRPKLLIYSASTLASGVSSRFKGSGSGTEFTLTISGVECADAATYYCQQGYTSSNVDNVFGGGTEVVVK

SEQ ID NO: 248 - protein, 113 aa, Oryctolagus cuniculus
AQVLTQTASPVSAAVGSTVTINCQASQSVYNNNYLGWFQQKPGQPPKRLIYSASKLESGVPSRFSGSGSGTQFTLTISDVQCEDAATYYCLGSYDCSSADCNVFGGGTEVVVK

SEQ ID NO: 249 - protein, 111 aa, Oryctolagus cuniculus
DVVMTQTPASVSAAVGGTVTINCQASESIDNWLAWYQQKPGQPPKLLIYSASNLASGVSSRFEGSTSGTQFTLTISDLECADAATYYCQSTFYGVNPVPNAFGGGTEVVVK

SEQ ID NO: 250 - protein, 111 aa, Oryctolagus cuniculus
AAVLTQTPSPVSAAVGGTVTIKCQSSQSVYSNNNLAWYQQKPGQPPKLLIYDASNLASGVPDRFSGSGSGTQFTLTISGVQCDDAATYYCLGVYDDDADNAFGGGTEVVVK

SEQ ID NO: 251 - protein, 113 aa, Oryctolagus cuniculus
DVVMTQTPASVEAAVGGTVTIKCQASQSISSYLSWYQQKPGQPPKLLIYRASSLESGVPSRFKGTGSGTEFTLTISDLECADAATYYCQCTYGSSTSSRSGNAFGGGTEVVVK

SEQ ID NO: 252 - protein, 111 aa, Oryctolagus cuniculus
DVVMTQTPASVEADVGGTVTIKCQASQSIRSYLAWYQQKPGQPPKVLIYRASTLESGVPSRFKGSGSGTQFTLTISDLECADAATYYCQCTYGSSGSSFLAFGGGTEVVVK

SEQ ID NO: 253 - protein, 110 aa, Oryctolagus cuniculus
AYDMTQTPASVEVAVGGTVTIKCQASESISVNLAWYQQKSGQPPKLLIYLASTLASGVPSRFKGSGSGTEFTLTISDLECADAATYYCQQTYSGSNVENSFGGGTEVVLK

SEQ ID NO: 254 - protein, 111 aa, Oryctolagus cuniculus
AAVLTQTPSPVSAAVGGTVSISCQSSESIYKNNYLAWYQQKSGQPPKLLIYRASTLTSGVPSRFKGSGSGTQFTLTISDVQCDDAATYYCAGDYSSSSDNTFGGGTEVVVK

SEQ ID NO: 255 - protein, 110 aa, Oryctolagus cuniculus
DVVMTQTPASASEPVGGTVTIKCQASQNIYSDFAWYRQKPGQPPKLLIYSASALASGVPSRFKGSGSGTDFTLTISDLECDDAAIYYCQSTYWESNNIGTFGGGTEVVVK

SEQ ID NO: 256 - protein, 112 aa, Oryctolagus cuniculus
AAVLTQTPSPVSAAVGGTVTISCQASQSVYNHKNLAWYQQKPGQPPKLLIYSASSLASGVPSRFKGSGSGTQFTLTISDLDCDDAATYYCAGGYSGSADTFAFGGGTEVVVK

SEQ ID NO: 257 - protein, 109 aa, Oryctolagus cuniculus
AFELTQTPASVEAAVGGTVTIKCQASQSISAYLSWYQQKPGQPPKLLIYDASDLASGVSSRFKGSGSGTEYTLTISGVQCADAATYYCQSYAGISSGVAFGGGTEVVVK

SEQ ID NO: 258 - protein, 112 aa, Oryctolagus cuniculus
DIVMTQTPASVEAAVGGTVTIKCQASQTITSYLAWYQQKPGQPPKLLIYRASILESGVPSRFKGSGSGTEFTLTISDLECADAATYYCQCTYGTTNTGHYVGFGGGTEVVVK

SEQ ID NO: 259 - protein, 112 aa, Oryctolagus cuniculus
AQVLTQTPSPVSAAVGGTVTINCQASQSVYNNKNLAWYQQKPGQPPKLLIYDASKLASGVPLRFSGSGSGTQFTLTISGVQCDDAATYYCAGGYDSSVDTFAFGGGTEVVVK

SEQ ID NO: 260 - protein, 113 aa, Oryctolagus cuniculus
DTVMTQTPASVEAAVGGTVTIQCQASENIYSLLAWYQQKPGQPPKLLIYRASTLASGVPSRFKGSGSGTEFTLTISDLECADAATYYCQSHYCCSSNYDYIYAFGGGTEVVVK

SEQ ID NO: 261 - protein, 112 aa, Oryctolagus cuniculus
DPVLTQTPPSASEPAGGTVTIKCQASEDIYSLLAWYQQKPGQPPKLLIYAASTLASGVPSRFKGSGSGTQFTLTISDLECADAATYYCQSYYYSISDSVDYPFGGGTEVVVK

SEQ ID NO: 262 - protein, 113 aa, Oryctolagus cuniculus
DVVMTQTPASVEAAVGGTVTIKCQASQSISTYLSWYQQKPGQPPKLLIYRATTLESGVPSRFKGTGSGTEFTLTINDLECADAATYYCQCTYGSSASSSYGNAFGGGTEVVVK

SEQ ID NO: 263 - protein, 109 aa, Oryctolagus cuniculus
AQVLTQTPSSVSEPVGGTVTINCQASENIYSSLAWYQQKPGQPPKLLIYDASDLASGVPSRFSGSGLGTEFTLTISGVQCDDAATYYCQTYYPSSVTYAFGGGTEVVVK

SEQ ID NO: 264 - protein, 111 aa, Oryctolagus cuniculus
AYDMTQTPSSVSAAVGGTVTINCQASESIGSWLAWYQQKPGQPPKLLIYSASSLASGVSSRFGGSTSGTEYTLTISDLECADAATYYCQSTFYGVNPVPTAFGGGTEVVVK

SEQ ID NO: 265 - protein, 111 aa, Oryctolagus cuniculus
AQVLTQTASPVSAAVGGTVTINCQSSQSVYNNNRLSWFQQKPGQPPKQLIYRSSTLASGVPSRFSGSGSGTQFTLTISDVQCDDAATYYCAGGYSSSSDNAFGGGTEVVVK

SEQ ID NO: 266 - protein, 110 aa, Oryctolagus cuniculus
AAVLTQTPSPVSAAVGGTVTISCQASQSVYNNNNLAWYQQKPGQPPKLLIYTASSLASGVPSRFKGSGSGTQFTLTISEVQCEDAATYYCQGYYSGYINAFGGGTEVVVK

SEQ ID NO: 267 - protein, 112 aa, Oryctolagus cuniculus
DIVMTQTPASVEAAVGGTVTIKCQASQSIGSYLSWYQQKPGQPPKLLIYYASDLESGVPSRFKGSGSGTEFTLTISDLECADACTYYCQCTYGSISSSAGNAFGGGTEVVVK

SEQ ID NO: 268 - protein, 110 aa, Oryctolagus cuniculus
AQVLTQTASPVSAAVGGTVTISCQSSESVYNNNLLSWYKQKPGQPPKLLIYKASTLDSGVPSRFKGSGSGTQFTLTISGVQCDDAATYYCQGGYTDATYAFGGGTEVVVK

SEQ ID NO: 269 - protein, 112 aa, Oryctolagus cuniculus
AQVLTQTPSPVSATVGGTVTINCQASQSVYNNRLAWYQQKPGQPPKLLIYEASTLTSGVSSRFKGSGSGAQFTLTISGVQCADAATYYCQGEFSCSNGDCIAFGGGTEVVVK

SEQ ID NO: 270 - protein, 112 aa, Oryctolagus cuniculus
DVVMTQTPASVEAAVGGTVTIKCQASQSISTYSSWYEQKPGQPPKLLIYYASDLESGVPSRFKGSGSGTEFTLTISDLECADAATYYCQCTYGSISSSSGNAFGGGTEVVVK

SEQ ID NO: 271 - protein, 110 aa, Oryctolagus cuniculus
AQVLTQTPSSVSAAVGGTVTISCQSSQSVYASVWLGWYQQKPGQPPKQLIYAASTLASGVPSRFKGSGSGTQFTLTISDLECGDAATYYCAGGYIGDIYAFGGGTEVVVE

SEQ ID NO: 272 - protein, 113 aa, Oryctolagus cuniculus
DVVMTQTPASVEAAVGGTVTIKCQASQSIYNYLSWYQQKPGQPPKLLIYGASDLASGVPSRFSGSGSGTEFTLTISDLECADAATYYCQCTYGSSRVSSYGDAFGGGTEVVVK

SEQ ID NO: 273 - protein, 108 aa, Oryctolagus cuniculus
DVVMTQTPVSVSAAVGGTVTINCQASQNIYSYLAWYQQKSGQPPKLLIYDASDLESGVPSRFKGSGSGTEYTLTISDLECADAATYYCQSYYGISAYAFGGGTEVVVK

SEQ ID NO: 274 - protein, 111 aa, Oryctolagus cuniculus
DIVMTQTPASVSEPVGGTVTIKCQASQSIYSYLAWYQQKPGQRPKLLIYGASTLASGVPSRFKGSGSGTDFALTISDLECADAATYYCQDNYGSSTTYGNSFGGGTEVVVK

SEQ ID NO: 275 - protein, 113 aa, Oryctolagus cuniculus
DIVMTQTPASVEAAVGGTVTIKCQASESIGSVLAWYQQKPGQSPKLLIGSASTLASGVPSRFKGSGSGTQFTLTISDLECADAATYYCQSYYHSTSGSSYGNTFGGGTEVVVK

SEQ ID NO: 276 - protein, 111 aa, Oryctolagus cuniculus
ALVMTQTPSSVSAAVGGTVTINCQASQNIYSNLAWYQQKPGQPPKLLIYGASDLESGVPSRFKGSGSGTEYTLTISDLECDDAATYYCQSTYYNISADFYAFGGGTEVVVK

SEQ ID NO: 277 - protein, 111 aa, Oryctolagus cuniculus
AAVLTQTPSPVSAVVGGTVSISCQSNKNVYDNNALSWYQQKPGQPPKFLIYRASTLASGVPSRFKGSGSGTQFTLTISDVQCDDAATYYCAGDYISDSDNTFGGGTEVVVK

SEQ ID NO: 278 - protein, 113 aa, Oryctolagus cuniculus
DIVMTQTPASVSEPVGGTVTIKCQASQSIINYLSWYQQKPGQPPKLLIYRASTLESGVPSRFKGSGSGTEFTLTISDLECADAATYYCQCTYGSSSGSYGGWAFGGGTEVVVK

SEQ ID NO: 279 - protein, 110 aa, Oryctolagus cuniculus
DIVMTQTPASVSEPVGGTVTIKCQASQSIYSYLSWYQQKPGQPPKLLIYQASILASGVPSQFKGSGSGTDFTLTISDLECADAATYYCQSNYGFSSGSYAFGGGTEVVVK

SEQ ID NO: 280 - protein, 112 aa, Oryctolagus cuniculus
DVVMTQTPASVEAAVGGTVTIKCQASQSISSWLAWYQQKPGQPPKLLIYRASTLESGVPSRFKGSGSGTEFTLTISDLECADAATYYCQCTYGSLSSTYGWAFGGGTEVVVK

SEQ ID NO: 281 - protein, 112 aa, Oryctolagus cuniculus
AAVLTQTPSSVSAAVGGTVTINCQSSQSVNNAKNLAWYQQKPGQPPKLLIYDASTLASGVPSRFKGSGSGTQFTLIMSDLECGDAATYFCAGGYDRFIDTFAFGGGTEVVVK

SEQ ID NO: 282 - protein, 111 aa, Oryctolagus cuniculus
AAVLTQTPSPVSAAVGGTVSISCQSSKSVYDNNWLSWYQQKPGQPPKLLIYQASTLASGVPSRFKGSGSGTQFTLTISDVQCDDAATYYCAGGYITNSDNGFGGGTEVVVK

SEQ ID NO: 283 - protein, 110 aa, Oryctolagus cuniculus
DVVMTQTPASVSESVGGTVTIKCQASQSIGSSLAWYQQKPGQPPKLLIYYTSTLASGVPSRFSGSGSGTEFTLTTSGVQCDDAATYYCQSYGYGSGYVFAFGGGTEVVVK

SEQ ID NO: 284 - protein, 111 aa, Oryctolagus cuniculus
AIEMTQTPFSVSAAVGGTVTINCQASENIYRNLAWYQQKPGQPPKLLIYKASTLASGVSSRFKGSGSGTQFTLTIGGVQCDDAATYYCLYSYYIDSNVDFAFGGGTEVVVK

SEQ ID NO: 285 - protein, 111 aa, Oryctolagus cuniculus
DVVMTQTPASVSEPVGGTVTIKCQASEDIESYLAWYQQKPGQPPKLLIYSASTLASGVPSRFSGSGYGTEFTLTISDLECADAATYYCQCTLYGVNFVPNVFGGGTEVVVK

SEQ ID NO: 286 - protein, 113 aa, Oryctolagus cuniculus
DVVMTQTPASVSEPVGGTVTIKCQASQSISSWLSWYQQKPGQPPKVLIYDASDLASGVSSRFKGTGAGTEFTLTISDLECADAATYYCQCTVGSSGVTGYGNAFGGGTEVVVK

SEQ ID NO: 287 - protein, 109 aa, Oryctolagus cuniculus
DVVMTQTPASVSEPVGGTVTIKCQASQSIGSDLAWYQQKPGQPPKLLIYDASSLESGVPSRFKGSGSGTDFTLTISDLECADAATYYCQCTYYGGSPNVFGGGTEVVVK

SEQ ID NO: 288 - protein, 110 aa, Oryctolagus cuniculus
AIEMTQTPASVEAAVGGTVTIKCQGSQSISSYLSWYQQKPGQPPKLLIYGASTLASGVSSRFKGSGSGTEFTLTISGVECADAATYYCQQGYTTSNVDNTFGGGTEVVVK

SEQ ID NO: 289 - protein, 110 aa, Oryctolagus cuniculus
AAVLTQTPSPVSAPVGGTVSISCQSSPSVYSVYLSWYQQKPGQPPKLLIYRASTLASGVPSRFKGSGSGTQFTLTISDVQCDDAATYYCAGAYVGSSDNTFGGGTEMVVK

SEQ ID NO: 290 - protein, 111 aa, Oryctolagus cuniculus
AAVLTQTPSPVSAAVGGTVSISCQSSKSVYNNKWLSWFQQKPGQPPKLLIYGAFTLASGVPSRFRGSGSGTQFTLTISDVQCDDAATYYCAGDYSSNSDDAFGGGTEVVVK

SEQ ID NO: 291 - protein, 112 aa, Oryctolagus cuniculus
DIVMTQTPASVEAAVGGTVTIKCQASESVGDALAWYQQKPGQPPKLLIYRASTLESGVPSRFKGSGSGTEFTLTISDLECADVATYYCQSYWYTMGNSYGNTFGGGTEVVVK

SEQ ID NO: 292 - protein, 111 aa, Oryctolagus cuniculus
AAVLTQTPSPVSAAVGGTVSISCQSSKTIYNDNWLSWFQQKPGQPPKLLIYGASTLASGVPSRFKGSGSGTQFTLTISDVQCDDAATYYCLGSYINSSDNAFGGGTEVVVK

SEQ ID NO: 293 - protein, 111 aa, Oryctolagus cuniculus
AIKMTQTPSSVSAAVGGTVTINCRASEDIKSYLAWYQQKPGQPPKLLIYDASDLASGVPSRFKGSGSGTEYTLTISGVQCDDAATYYCQSAYYSSSTDGGAFGGGTEVVVK

SEQ ID NO: 294 - protein, 111 aa, Oryctolagus cuniculus
ALVMTQTPSSVSAPVGGTVTINCQASQSIYSNLAWYQQKPGQRPKLLIYGASNLESGVPSRFKGSGSGTQFTLTISDLECADAATYCCQGYYYADSDDNIAFGGGTEVVVE

SEQ ID NO: 295 - protein, 110 aa, Oryctolagus cuniculus
AQVLTQTASPVSAAVGSTVTISCQASQSVYNNNYLAWFQQKPGQPPKLLIYLASTLASGVPSRFKGSGSGTQFTLTISGVQCGDAATYYCQGYYSTGMFAFGGGTEVVVK

SEQ ID NO: 296 - protein, 111 aa, Oryctolagus cuniculus
DVVMTQTPSSVSAAVGGTVTINCRASEDIERFLAWYQQKPGQPPKLLIYKASTLASGVPSRFKGSGSGTDFTLTISDLECADAATYYCQCTLYGVNFVPNAFGGGTEVVVK

SEQ ID NO: 297 - protein, 5 aa, Oryctolagus cuniculus
AYAIN

SEQ ID NO: 298 - protein, 5 aa, Oryctolagus cuniculus
GYDMN

SEQ ID NO: 299 - protein, 5 aa, Oryctolagus cuniculus
TYAIS

SEQ ID NO: 300 - protein, 5 aa, Oryctolagus cuniculus
GLVVS

SEQ ID NO: 301 - protein, 6 aa, Oryctolagus cuniculus
SSYYMC

SEQ ID NO: 302 - protein, 5 aa, Oryctolagus cuniculus
IYAIS

SEQ ID NO: 303 - protein, 6 aa, Oryctolagus cuniculus
SSYYMC

SEQ ID NO: 304 - protein, 5 aa, Oryctolagus cuniculus
MYAIN

SEQ ID NO: 305 - protein, 6 aa, Oryctolagus cuniculus
SYYYMC

SEQ ID NO: 306 - protein, 5 aa, Oryctolagus cuniculus
RNAMS

SEQ ID NO: 307 - protein, 6 aa, Oryctolagus cuniculus
DNYAMC

SEQ ID NO: 308 - protein, 6 aa, Oryctolagus cuniculus
SGYYMC

SEQ ID NO: 309 - protein, 6 aa, Oryctolagus cuniculus
GNYYIC

SEQ ID NO: 310 - protein, 6 aa, Oryctolagus cuniculus
RSYYMC

SEQ ID NO: 311 - protein, 6 aa, Oryctolagus cuniculus
SMYWMC

SEQ ID NO: 312 - protein, 5 aa, Oryctolagus cuniculus
SYDMS

SEQ ID NO: 313 - protein, 6 aa, Oryctolagus cuniculus
SSYWIC

SEQ ID NO: 314 - protein, 6 aa, Oryctolagus cuniculus
SSYYIC

SEQ ID NO: 315 - protein, 6 aa, Oryctolagus cuniculus
DGYWMC

SEQ ID NO: 316 - protein, 5 aa, Oryctolagus cuniculus
SYAMS

SEQ ID NO: 317 - protein, 5 aa, Oryctolagus cuniculus
NYQMT

SEQ ID NO: 318 - protein, 5 aa, Oryctolagus cuniculus
MYAIN

SEQ ID NO: 319 - protein, 5 aa, Oryctolagus cuniculus
NYDMN

SEQ ID NO: 320 - protein, 5 aa, Oryctolagus cuniculus
NYDMN

SEQ ID NO: 321 - protein, 5 aa, Oryctolagus cuniculus
SNAMI

SEQ ID NO: 322 - protein, 5 aa, Oryctolagus cuniculus
MYTIN

SEQ ID NO: 323 - protein, 5 aa, Oryctolagus cuniculus
SNSIS

SEQ ID NO: 324 - protein, 6 aa, Oryctolagus cuniculus
STYWMS

SEQ ID NO: 325 - protein, 5 aa, Oryctolagus cuniculus
NYALS

SEQ ID NO: 326 - protein, 5 aa, Oryctolagus cuniculus
SHATS

SEQ ID NO: 327 - protein, 5 aa, Oryctolagus cuniculus
TYGVS

SEQ ID NO: 328 - protein, 6 aa, Oryctolagus cuniculus
SNYYIC

SEQ ID NO: 329 - protein, 5 aa, Oryctolagus cuniculus
TYAMT

SEQ ID NO: 330 - protein, 6 aa, Oryctolagus cuniculus
SSYWIC

SEQ ID NO: 331 - protein, 5 aa, Oryctolagus cuniculus
NYAMS

SEQ ID NO: 332 - protein, 5 aa, Oryctolagus cuniculus
NYQMT

SEQ ID NO: 333 - protein, 6 aa, Oryctolagus cuniculus
STYWAC

SEQ ID NO: 334 - protein, 5 aa, Oryctolagus cuniculus
SYQMT

SEQ ID NO: 335 - protein, 6 aa, Oryctolagus cuniculus
SSYYMC

SEQ ID NO: 336 - protein, 6 aa, Oryctolagus cuniculus
SNYYMC

SEQ ID NO: 337 - protein, 6 aa, Oryctolagus cuniculus
SSYYMC

SEQ ID NO: 338 - protein, 5 aa, Oryctolagus cuniculus
NWIMS

SEQ ID NO: 339 - protein, 6 aa, Oryctolagus cuniculus
STYSMC

SEQ ID NO: 340 - protein, 6 aa, Oryctolagus cuniculus
SGYDMC

SEQ ID NO: 341 - protein, 6 aa, Oryctolagus cuniculus
STYYTC

SEQ ID NO: 342 - protein, 5 aa, Oryctolagus cuniculus
SAAMG

SEQ ID NO: 343 - protein, 5 aa, Oryctolagus cuniculus
SYDMS

SEQ ID NO: 344 - protein, 6 aa, Oryctolagus cuniculus
STYWIC

SEQ ID NO: 345 - protein, 6 aa, Oryctolagus cuniculus
SSYWIC

SEQ ID NO: 346 - protein, 5 aa, Oryctolagus cuniculus
SDGIS

SEQ ID NO: 347 - protein, 5 aa, Oryctolagus cuniculus
SYAIS

SEQ ID NO: 348 - protein, 5 aa, Oryctolagus cuniculus
SNALG

SEQ ID NO: 349 - protein, 5 aa, Oryctolagus cuniculus
SYDMS

SEQ ID NO: 350 - protein, 5 aa, Oryctolagus cuniculus
NYAMG

SEQ ID NO: 351 - protein, 5 aa, Oryctolagus cuniculus
VYAMS

SEQ ID NO: 352 - protein, 5 aa, Oryctolagus cuniculus
TYGVS

SEQ ID NO: 353 - protein, 5 aa, Oryctolagus cuniculus
MYAIN

SEQ ID NO: 354 - protein, 5 aa, Oryctolagus cuniculus
RYAMS

SEQ ID NO: 355 - protein, 5 aa, Oryctolagus cuniculus
SYAMG

SEQ ID NO: 356 - protein, 6 aa, Oryctolagus cuniculus
SSYWIC

SEQ ID NO: 357 - protein, 5 aa, Oryctolagus cuniculus
NYYMT

SEQ ID NO: 358 - protein, 5 aa, Oryctolagus cuniculus
SYHMS

SEQ ID NO: 359 - protein, 5 aa, Oryctolagus cuniculus
TIPMC

SEQ ID NO: 360 - protein, 6 aa, Oryctolagus cuniculus
DNYAMC

SEQ ID NO: 361 - protein, 5 aa, Oryctolagus cuniculus
SYHMG

SEQ ID NO: 362 - protein, 6 aa, Oryctolagus cuniculus
SRYWIY

SEQ ID NO: 363 - protein, 5 aa, Oryctolagus cuniculus
SYFLT

SEQ ID NO: 364 - protein, 5 aa, Oryctolagus cuniculus
SYAMS

SEQ ID NO: 365 - protein, 5 aa, Oryctolagus cuniculus
SNAMC

SEQ ID NO: 366 - protein, 5 aa, Oryctolagus cuniculus
VYAMS

SEQ ID NO: 367 - protein, 5 aa, Oryctolagus cuniculus
SYAMG

SEQ ID NO: 368 - protein, 6 aa, Oryctolagus cuniculus
GSYWNC

SEQ ID NO: 369 - protein, 6 aa, Oryctolagus cuniculus
SGYDMC

SEQ ID NO: 370 - protein, 5 aa, Oryctolagus cuniculus
AYGVN

SEQ ID NO: 371 - protein, 6 aa, Oryctolagus cuniculus
NSYYMC

SEQ ID NO: 372 - protein, 5 aa, Oryctolagus cuniculus
SNAMC

SEQ ID NO: 373 - protein, 5 aa, Oryctolagus cuniculus
SYAMG

SEQ ID NO: 374 - protein, 5 aa, Oryctolagus cuniculus
TNGVS

SEQ ID NO: 375 - protein, 6 aa, Oryctolagus cuniculus
SGYYMC

SEQ ID NO: 376 - protein, 6 aa, Oryctolagus cuniculus
SGYCLC

SEQ ID NO: 377 - protein, 5 aa, Oryctolagus cuniculus
SYWMC

SEQ ID NO: 378 - protein, 6 aa, Oryctolagus cuniculus
SYYYMS

SEQ ID NO: 379 - protein, 5 aa, Oryctolagus cuniculus
YNTIC

SEQ ID NO: 380 - protein, 6 aa, Oryctolagus cuniculus
SSYYMC

SEQ ID NO: 381 - protein, 5 aa, Oryctolagus cuniculus
NYAMS

SEQ ID NO: 382 - protein, 5 aa, Oryctolagus cuniculus
NYAVG

SEQ ID NO: 383 - protein, 6 aa, Oryctolagus cuniculus
SSYYMC

SEQ ID NO: 384 - protein, 6 aa, Oryctolagus cuniculus
SRYYVC

SEQ ID NO: 385 - protein, 5 aa, Oryctolagus cuniculus
ANAMS

SEQ ID NO: 386 - protein, 5 aa, Oryctolagus cuniculus
NYHMS

SEQ ID NO: 387 - protein, 5 aa, Oryctolagus cuniculus
NYGLT

SEQ ID NO: 388 - protein, 6 aa, Oryctolagus cuniculus
SSYYMC

SEQ ID NO: 389 - protein, 5 aa, Oryctolagus cuniculus
TYAMS

SEQ ID NO: 390 - protein, 5 aa, Oryctolagus cuniculus
NYGVS

SEQ ID NO: 391 - protein, 6 aa, Oryctolagus cuniculus
VSYWIC

SEQ ID NO: 392 - protein, 6 aa, Oryctolagus cuniculus
SGYDMC

SEQ ID NO: 393 - protein, 5 aa, Oryctolagus cuniculus
SNAMC

SEQ ID NO: 394 - protein, 6 aa, Oryctolagus cuniculus
SSYYMC

SEQ ID NO: 395 - protein, 6 aa, Oryctolagus cuniculus
SSYWIY

SEQ ID NO: 396 - protein, 5 aa, Oryctolagus cuniculus
RYGVS

SEQ ID NO: 397 - protein, 6 aa, Oryctolagus cuniculus
NNYYMC

SEQ ID NO: 398 - protein, 6 aa, Oryctolagus cuniculus
SNYYMC

SEQ ID NO: 399 - protein, 5 aa, Oryctolagus cuniculus
SYAMS

SEQ ID NO: 400 - protein, 6 aa, Oryctolagus cuniculus
SSYCMC

SEQ ID NO: 401 - protein, 5 aa, Oryctolagus cuniculus
SYAMG

SEQ ID NO: 402 - protein, 6 aa, Oryctolagus cuniculus
SGYDMC

SEQ ID NO: 403 - protein, 5 aa, Oryctolagus cuniculus
DYYMS

SEQ ID NO: 404 - protein, 5 aa, Oryctolagus cuniculus
SHATS

SEQ ID NO: 405 - protein, 6 aa, Oryctolagus cuniculus
SGYWIC

SEQ ID NO: 406 - protein, 5 aa, Oryctolagus cuniculus
SYTMA

SEQ ID NO: 407 - protein, 5 aa, Oryctolagus cuniculus
SYHMC

SEQ ID NO: 408 - protein, 6 aa, Oryctolagus cuniculus
GDYDMC

SEQ ID NO: 409 - protein, 6 aa, Oryctolagus cuniculus
SSYYMC

SEQ ID NO: 410 - protein, 5 aa, Oryctolagus cuniculus
SYAMS

SEQ ID NO: 411 - protein, 5 aa, Oryctolagus cuniculus
SYTMT

SEQ ID NO: 412 - protein, 6 aa, Oryctolagus cuniculus
SKYYMC

SEQ ID NO: 413 - protein, 5 aa, Oryctolagus cuniculus
SYYIY

SEQ ID NO: 414 - protein, 6 aa, Oryctolagus cuniculus
SVYDMC

SEQ ID NO: 415 - protein, 5 aa, Oryctolagus cuniculus
SYHMS

SEQ ID NO: 416 - protein, 5 aa, Oryctolagus cuniculus
GLVVS

SEQ ID NO: 417 - protein, 5 aa, Oryctolagus cuniculus
RDAMS

SEQ ID NO: 418 - protein, 5 aa, Oryctolagus cuniculus
SYWIC

SEQ ID NO: 419 - protein, 5 aa, Oryctolagus cuniculus
RYAMI

SEQ ID NO: 420 - protein, 6 aa, Oryctolagus cuniculus
NNYWIC

SEQ ID NO: 421 - protein, 6 aa, Oryctolagus cuniculus
TYYYMC

SEQ ID NO: 422 - protein, 5 aa, Oryctolagus cuniculus
SYWMS

SEQ ID NO: 423 - protein, 5 aa, Oryctolagus cuniculus
RNAAS

SEQ ID NO: 424 - protein, 5 aa, Oryctolagus cuniculus
NYAMT

SEQ ID NO: 425 - protein, 5 aa, Oryctolagus cuniculus
SNAIS

SEQ ID NO: 426 - protein, 6 aa, Oryctolagus cuniculus
VGYYMC

SEQ ID NO: 427 - protein, 6 aa, Oryctolagus cuniculus
SSYWIC

SEQ ID NO: 428 - protein, 6 aa, Oryctolagus cuniculus
SSYYMC

SEQ ID NO: 429 - protein, 5 aa, Oryctolagus cuniculus
NYHMT

SEQ ID NO: 430 - protein, 5 aa, Oryctolagus cuniculus
SYDMT

SEQ ID NO: 431 - protein, 6 aa, Oryctolagus cuniculus
SSYCVC

SEQ ID NO: 432 - protein, 5 aa, Oryctolagus cuniculus
SNAMC

SEQ ID NO: 433 - protein, 6 aa, Oryctolagus cuniculus
GNYYMC

SEQ ID NO: 434 - protein, 5 aa, Oryctolagus cuniculus
SYHMN

SEQ ID NO: 435 - protein, 6 aa, Oryctolagus cuniculus
SSYYMC

SEQ ID NO: 436 - protein, 5 aa, Oryctolagus cuniculus
SYPVN

SEQ ID NO: 437 - protein, 5 aa, Oryctolagus cuniculus
SYDMS

SEQ ID NO: 438 - protein, 5 aa, Oryctolagus cuniculus
NYGMT

SEQ ID NO: 439 - protein, 5 aa, Oryctolagus cuniculus
TYWMS

SEQ ID NO: 440 - protein, 5 aa, Oryctolagus cuniculus
SYAMG

SEQ ID NO: 441 - protein, 6 aa, Oryctolagus cuniculus
SSYYMC

SEQ ID NO: 442 - protein, 6 aa, Oryctolagus cuniculus
SGQDMC

SEQ ID NO: 443 - protein, 5 aa, Oryctolagus cuniculus
SYNMG

SEQ ID NO: 444 - protein, 6 aa, Oryctolagus cuniculus
SSYYMC

SEQ ID NO: 445 - protein, 16 aa, Oryctolagus cuniculus
GIANNGPTYYANWAKG

SEQ ID NO: 446 - protein, 16 aa, Oryctolagus cuniculus
MIYPNSGTNYATWAKG

SEQ ID NO: 447 - protein, 16 aa, Oryctolagus cuniculus
GISNSGTTYYASWAKG

SEQ ID NO: 448 - protein, 16 aa, Oryctolagus cuniculus
VIGKSGNTYYASWAKG

SEQ ID NO: 449 - protein, 18 aa, Oryctolagus cuniculus
CIYAGSSGSTYYASWAKG

SEQ ID NO: 450 - protein, 16 aa, Oryctolagus cuniculus
GIGNNGIIHYANWAKG

SEQ ID NO: 451 - protein, 18 aa, Oryctolagus cuniculus
CIYGGSSGKTWYASWAKG

SEQ ID NO: 452 - protein, 16 aa, Oryctolagus cuniculus
GIANNGPTYYASWAKG

SEQ ID NO: 453 - protein, 17 aa, Oryctolagus cuniculus
CIYADDATTYYATWAKG

SEQ ID NO: 454 - protein, 16 aa, Oryctolagus cuniculus
IIRNTGTTWYASWAKG

SEQ ID NO: 455 - protein, 17 aa, Oryctolagus cuniculus
CIYVGSGSTYYASWAQG

SEQ ID NO: 456 - protein, 17 aa, Oryctolagus cuniculus
CIYTSSGSTYYASWAKG

SEQ ID NO: 457 - protein, 18 aa, Oryctolagus cuniculus
CIYAGSSGSTYYASWAKG

SEQ ID NO: 458 - protein, 18 aa, Oryctolagus cuniculus
CIYAGSSDSTYYASWAKG

SEQ ID NO: 459 - protein, 18 aa, Oryctolagus cuniculus
CIYTGSSGKTHYASWAKG

SEQ ID NO: 460 - protein, 16 aa, Oryctolagus cuniculus
IIYDSGSTYYANWAKG

SEQ ID NO: 461 - protein, 17 aa, Oryctolagus cuniculus
CIAAGSGSTYYASWAKG

SEQ ID NO: 462 - protein, 18 aa, Oryctolagus cuniculus
CIYAGSSGSTYYASWAKG

SEQ ID NO: 463 - protein, 17 aa, Oryctolagus cuniculus
CIYTGPGGTFYASWAKG

SEQ ID NO: 464 - protein, 16 aa, Oryctolagus cuniculus
IIHYSGYTAYASWAKG

SEQ ID NO: 465 - protein, 16 aa, Oryctolagus cuniculus
FIKADGSAYYANWAKG

SEQ ID NO: 466 - protein, 16 aa, Oryctolagus cuniculus
GIATNGIIHYASWVKG

SEQ ID NO: 467 - protein, 16 aa, Oryctolagus cuniculus
MIYPNSGTNYASWAKG

SEQ ID NO: 468 - protein, 16 aa, Oryctolagus cuniculus
MIYPNGGTNYATWAKG

SEQ ID NO: 469 - protein, 16 aa, Oryctolagus cuniculus
IIYASDSTYYATWAKG

SEQ ID NO: 470 - protein, 16 aa, Oryctolagus cuniculus
GIATHGIIHYASWVKG

SEQ ID NO: 471 - protein, 16 aa, Oryctolagus cuniculus
IISSSGSTYYASWAKG

SEQ ID NO: 472 - protein, 17 aa, Oryctolagus cuniculus
CIVTGRGNTYYANWAKG

SEQ ID NO: 473 - protein, 16 aa, Oryctolagus cuniculus
FINIIHGAYYASWAKG

SEQ ID NO: 474 - protein, 16 aa, Oryctolagus cuniculus
FIKTGGSAYYASWAKG

SEQ ID NO: 475 - protein, 16 aa, Oryctolagus cuniculus
YINTGGSASYATWAKG

SEQ ID NO: 476 - protein, 18 aa, Oryctolagus cuniculus
CIYTGSTGSTYYASWAKG

SEQ ID NO: 477 - protein, 16 aa, Oryctolagus cuniculus
IISNSGATAYASWAKG

SEQ ID NO: 478 - protein, 17 aa, Oryctolagus cuniculus
CIGTSSTISYYASWAKG

SEQ ID NO: 479 - protein, 16 aa, Oryctolagus cuniculus
IIHYSGYIAYANWAKG

SEQ ID NO: 480 - protein, 16 aa, Oryctolagus cuniculus
FIKPGGSAYYASWAKG

SEQ ID NO: 481 - protein, 18 aa, Oryctolagus cuniculus
CIDGGSSGITGYANWAKG

SEQ ID NO: 482 - protein, 16 aa, Oryctolagus cuniculus
FINTGGSAYYASWAKG

SEQ ID NO: 483 - protein, 18 aa, Oryctolagus cuniculus
CIYAGSSGSTYYASWAKG

SEQ ID NO: 484 - protein, 18 aa, Oryctolagus cuniculus
CIYTGSSGSTYYASWAKG

SEQ ID NO: 485 - protein, 18 aa, Oryctolagus cuniculus
CIHAGSSGAAYYATWAKG

SEQ ID NO: 486 - protein, 16 aa, Oryctolagus cuniculus
IITTSGNTYYASWAKG

SEQ ID NO: 487 - protein, 18 aa, Oryctolagus cuniculus
CIYTGSSGGTYYASWAKG

SEQ ID NO: 488 - protein, 17 aa, Oryctolagus cuniculus
CIYTVNDNTWYASWAKG

SEQ ID NO: 489 - protein, 18 aa, Oryctolagus cuniculus
CIVDGSSGNTYYASWAKG

SEQ ID NO: 490 - protein, 16 aa, Oryctolagus cuniculus
YISTSGTPYYASWVNG

SEQ ID NO: 491 - protein, 16 aa, Oryctolagus cuniculus
IIYNSGTTYYANWAKG

SEQ ID NO: 492 - protein, 18 aa, Oryctolagus cuniculus
CIYTDSSTSTYYASWAKG

SEQ ID NO: 493 - protein, 18 aa, Oryctolagus cuniculus
CIVGGGGVNTYYANWAKG

SEQ ID NO: 494 - protein, 17 aa, Oryctolagus cuniculus
FIYPGVGITHYAHSVKG

SEQ ID NO: 495 - protein, 16 aa, Oryctolagus cuniculus
GVANNGITNYASWARG

SEQ ID NO: 496 - protein, 16 aa, Oryctolagus cuniculus
YISTGGSAYYATWVNG

SEQ ID NO: 497 - protein, 16 aa, Oryctolagus cuniculus
IIYDSGSTYYASWAKG

SEQ ID NO: 498 - protein, 16 aa, Oryctolagus cuniculus
VISSNGGTVYANWAKG

SEQ ID NO: 499 - protein, 16 aa, Oryctolagus cuniculus
IITFSGNTYYASWAKG

SEQ ID NO: 500 - protein, 16 aa, Oryctolagus cuniculus
YINIYGRTYYANWAKS

SEQ ID NO: 501 - protein, 16 aa, Oryctolagus cuniculus
GIANNGPTYYASWAKG

SEQ ID NO: 502 - protein, 16 aa, Oryctolagus cuniculus
IISSSGNSYYASWAKG

SEQ ID NO: 503 - protein, 15 aa, Oryctolagus cuniculus
IISSGLTYYASWAKG

SEQ ID NO: 504 - protein, 18 aa, Oryctolagus cuniculus
CINFGRSGNIYYARWAKG

SEQ ID NO: 505 - protein, 16 aa, Oryctolagus cuniculus
FIDPYSSPYYASWAKG

SEQ ID NO: 506 - protein, 16 aa, Oryctolagus cuniculus
VIYGSGSAWYASWAKG

SEQ ID NO: 507 - protein, 17 aa, Oryctolagus cuniculus
CIYPDYGDTFYATWAKG

SEQ ID NO: 508 - protein, 17 aa, Oryctolagus cuniculus
CIFGSSGSIAYATWAKG

SEQ ID NO: 509 - protein, 16 aa, Oryctolagus cuniculus
FITTTGGSYYASWARG

SEQ ID NO: 510 - protein, 18 aa, Oryctolagus cuniculus
CIDTGSRGFTYYPSWAKG

SEQ ID NO: 511 - protein, 16 aa, Oryctolagus cuniculus
FMNSGGSTYYASWVNG

SEQ ID NO: 512 - protein, 16 aa, Oryctolagus cuniculus
MIRSSGITWYASWAKG

SEQ ID NO: 513 - protein, 18 aa, Oryctolagus cuniculus
CIYAGSRGSAYYASWVNG

SEQ ID NO: 514 - protein, 16 aa, Oryctolagus cuniculus
IITWSADTYYTSWAKG

SEQ ID NO: 515 - protein, 16 aa, Oryctolagus cuniculus
INGVSGTTYYATWANG

SEQ ID NO: 516 - protein, 18 aa, Oryctolagus cuniculus
CIDGEGSGNTYYASWVNG

SEQ ID NO: 517 - protein, 17 aa, Oryctolagus cuniculus
CIDTGDGSTYYASWVNG

SEQ ID NO: 518 - protein, 16 aa, Oryctolagus cuniculus
SISNSGGTYYASWAKG

SEQ ID NO: 519 - protein, 18 aa, Oryctolagus cuniculus
CIDAGSVGDTSYATWAKG

SEQ ID NO: 520 - protein, 17 aa, Oryctolagus cuniculus
CIYNGDGSTYYASWVNG

SEQ ID NO: 521 - protein, 16 aa, Oryctolagus cuniculus
IISNSGATAYASWAKG

SEQ ID NO: 522 - protein, 16 aa, Oryctolagus cuniculus
YIFTGGNTYYASWAKG

SEQ ID NO: 523 - protein, 18 aa, Oryctolagus cuniculus
CIYVGITGSTYYASWAKG

SEQ ID NO: 524 - protein, 18 aa, Oryctolagus cuniculus
CKHGGASGTTYYATWAKG

SEQ ID NO: 525 - protein, 18 aa, Oryctolagus cuniculus
CSYAGGSGGTYYASWAKG

SEQ ID NO: 526 - protein, 17 aa, Oryctolagus cuniculus
CTDGTGGITYYASWAKG

SEQ ID NO: 527 - protein, 18 aa, Oryctolagus cuniculus
YINTGSSGTTYYASWAKG

SEQ ID NO: 528 - protein, 18 aa, Oryctolagus cuniculus
CIYAGSSGSTYYASWAKG

SEQ ID NO: 529 - protein, 16 aa, Oryctolagus cuniculus
FINIIDSTYYTNWAKG

SEQ ID NO: 530 - protein, 16 aa, Oryctolagus cuniculus
VINAGGSAYYATWAKG

SEQ ID NO: 531 - protein, 18 aa, Oryctolagus cuniculus
CIYADSSGSTYYASWAKG

SEQ ID NO: 532 - protein, 17 aa, Oryctolagus cuniculus
CIDAGDGSTDYARWAKG

SEQ ID NO: 533 - protein, 16 aa, Oryctolagus cuniculus
TIFDTYLTYNANWAKG

SEQ ID NO: 534 - protein, 16 aa, Oryctolagus cuniculus
FIRTDGSAFYATWAKG

SEQ ID NO: 535 - protein, 16 aa, Oryctolagus cuniculus
YINNNGRTYYASRAKG

SEQ ID NO: 536 - protein, 18 aa, Oryctolagus cuniculus
CVYAGSSGSTYYASWAKG

SEQ ID NO: 537 - protein, 16 aa, Oryctolagus cuniculus
IIDASVTTYYASWAKG

SEQ ID NO: 538 - protein, 17 aa, Oryctolagus cuniculus
YIDPVFRSAYYASWVNG

SEQ ID NO: 539 - protein, 17 aa, Oryctolagus cuniculus
CIGGNSGNIYYARWAKG

SEQ ID NO: 540 - protein, 17 aa, Oryctolagus cuniculus
CIYSSNGLTWYATWAKG

SEQ ID NO: 541 - protein, 17 aa, Oryctolagus cuniculus
CIVTGSGSTYYASWAKG

SEQ ID NO: 542 - protein, 17 aa, Oryctolagus cuniculus
GVDGSGGIKWYANWAKG

SEQ ID NO: 543 - protein, 17 aa, Oryctolagus cuniculus
CFHAGSGSTYYASWVNG

SEQ ID NO: 544 - protein, 16 aa, Oryctolagus cuniculus
WISSSGSAYYATWAKG

SEQ ID NO: 545 - protein, 18 aa, Oryctolagus cuniculus
CIYTGSTGSTYYANWAKG

SEQ ID NO: 546 - protein, 18 aa, Oryctolagus cuniculus
CIYAGSSGSSYYASWAKG

SEQ ID NO: 547 - protein, 16 aa, Oryctolagus cuniculus
IIRRSGATWYANWARG

SEQ ID NO: 548 - protein, 18 aa, Oryctolagus cuniculus
CIYDGSSDSAYYATWAKG

SEQ ID NO: 549 - protein, 16 aa, Oryctolagus cuniculus
IITYGGSTYYASWAKG

SEQ ID NO: 550 - protein, 18 aa, Oryctolagus cuniculus
CIAVYSSGSTYYASWAKG

SEQ ID NO: 551 - protein, 16 aa, Oryctolagus cuniculus
VVSWNGNTYYASWAKG

SEQ ID NO: 552 - protein, 16 aa, Oryctolagus cuniculus
FIKSGGSTYYASWAKG

SEQ ID NO: 553 - protein, 18 aa, Oryctolagus cuniculus
CIDAGSNGSTYYASWARG

SEQ ID NO: 554 - protein, 16 aa, Oryctolagus cuniculus
VINTGGSAYYASWAKG

SEQ ID NO: 555 - protein, 16 aa, Oryctolagus cuniculus
FIKADGNTYYATWAKG

SEQ ID NO: 556 - protein, 18 aa, Oryctolagus cuniculus
CIGAGSSNDTYYASWAKG

SEQ ID NO: 557 - protein, 18 aa, Oryctolagus cuniculus
CISVGSSGSTYYANWAKG

SEQ ID NO: 558 - protein, 16 aa, Oryctolagus cuniculus
IIRRSGFTYYASWARG

SEQ ID NO: 559 - protein, 16 aa, Oryctolagus cuniculus
LISRSGRTYYATWAKG

SEQ ID NO: 560 - protein, 18 aa, Oryctolagus cuniculus
CIYTGTTGSTYYASWAKY

SEQ ID NO: 561 - protein, 17 aa, Oryctolagus cuniculus
CIAIINSITYYANWAKG

SEQ ID NO: 562 - protein, 18 aa, Oryctolagus cuniculus
CIYSDGSGSTYYANWAKG

SEQ ID NO: 563 - protein, 16 aa, Oryctolagus cuniculus
FIVGTGDTYYASWAKG

SEQ ID NO: 564 - protein, 16 aa, Oryctolagus cuniculus
VIGKSGSTYYASWAKG

SEQ ID NO: 565 - protein, 17 aa, Oryctolagus cuniculus
SIVSGSGSTYYASWAKG

SEQ ID NO: 566 - protein, 18 aa, Oryctolagus cuniculus
CIYAGSSGSTYYASWAKG

SEQ ID NO: 567 - protein, 16 aa, Oryctolagus cuniculus
IIDIRGTTYYASWAKG

SEQ ID NO: 568 - protein, 18 aa, Oryctolagus cuniculus
CIVAGSSGRTYYANWAKG

SEQ ID NO: 569 - protein, 18 aa, Oryctolagus cuniculus
CIHAGSSGSTYYASWAKG

SEQ ID NO: 570 - protein, 17 aa, Oryctolagus cuniculus
TINAASGATWYASWAKG

SEQ ID NO: 571 - protein, 16 aa, Oryctolagus cuniculus
IISTGGSTYYATWAKG

SEQ ID NO: 572 - protein, 16 aa, Oryctolagus cuniculus
IIINTGYTYYASWAKG

SEQ ID NO: 573 - protein, 16 aa, Oryctolagus cuniculus
HSDIRGSAYYASWAKG

SEQ ID NO: 574 - protein, 18 aa, Oryctolagus cuniculus
CIYAGSNGSTYYASWAKG

SEQ ID NO: 575 - protein, 18 aa, Oryctolagus cuniculus
CIYADGSGSIYCATWAKG

SEQ ID NO: 576 - protein, 17 aa, Oryctolagus cuniculus
CIYIGDGNTYYASWAKG

SEQ ID NO: 577 - protein, 16 aa, Oryctolagus cuniculus
FIKAGGSAGYASWAKG

SEQ ID NO: 578 - protein, 16 aa, Oryctolagus cuniculus
VISSSDSTYYASWAKG

SEQ ID NO: 579 - protein, 18 aa, Oryctolagus cuniculus
CIYGGSSGGTYYASWAKG

SEQ ID NO: 580 - protein, 18 aa, Oryctolagus cuniculus
CIYTSSSGSTYYASWVNG

SEQ ID NO: 581 - protein, 18 aa, Oryctolagus cuniculus
CIYADNSGSTYYASWAKG

SEQ ID NO: 582 - protein, 16 aa, Oryctolagus cuniculus
VIYGSGSTDYASWAKG

SEQ ID NO: 583 - protein, 18 aa, Oryctolagus cuniculus
CIYSDSSGSTYNANWVKG

SEQ ID NO: 584 - protein, 16 aa, Oryctolagus cuniculus
VIGNRGSTDYASWAKG

SEQ ID NO: 585 - protein, 16 aa, Oryctolagus cuniculus
TIYDGGSTYYASWTKG

SEQ ID NO: 586 - protein, 16 aa, Oryctolagus cuniculus
IINIIDNTYYASWAKG

SEQ ID NO: 587 - protein, 16 aa, Oryctolagus cuniculus
TISTGGSAYYASWAKS

SEQ ID NO: 588 - protein, 15 aa, Oryctolagus cuniculus
YINRGNTYYANWAKG

SEQ ID NO: 589 - protein, 18 aa, Oryctolagus cuniculus
CIHAGSSGSAYYASWAKG

SEQ ID NO: 590 - protein, 17 aa, Oryctolagus cuniculus
CIYGGDGNTYYASWAKG

SEQ ID NO: 591 - protein, 16 aa, Oryctolagus cuniculus
YIWSGGSAYYASWAKG

SEQ ID NO: 592 - protein, 18 aa, Oryctolagus cuniculus
CIYAGSSGSTYYASWAKG

SEQ ID NO: 593 - protein, 14 aa, Oryctolagus cuniculus
FPPGTNGGTDYFNI

SEQ ID NO: 594 - protein, 9 aa, Oryctolagus cuniculus
DSGWGAFDP

SEQ ID NO: 595 - protein, 14 aa, Oryctolagus cuniculus
FPPGSNSGTDYFNI

SEQ ID NO: 596 - protein, 7 aa, Oryctolagus cuniculus
NISGSAV

SEQ ID NO: 597 - protein, 17 aa, Oryctolagus cuniculus
DLGAGYAGYGYASDFNL

SEQ ID NO: 598 - protein, 14 aa, Oryctolagus cuniculus
FPPGSNSGTDYFNI

SEQ ID NO: 599 - protein, 9 aa, Oryctolagus cuniculus
DNYDWYFNL

SEQ ID NO: 600 - protein, 14 aa, Oryctolagus cuniculus
FPPGSNSGTDYFNI

SEQ ID NO: 601 - protein, 16 aa, Oryctolagus cuniculus
RDADYVGFIWAYYFNL

SEQ ID NO: 602 - protein, 8 aa, Oryctolagus cuniculus
GNPGWAST

SEQ ID NO: 603 - protein, 15 aa, Oryctolagus cuniculus
GVVIGNAYSMAHFSL

SEQ ID NO: 604 - protein, 17 aa, Oryctolagus cuniculus
RLNYVTYPAYGYGYFNL

SEQ ID NO: 605 - protein, 11 aa, Oryctolagus cuniculus
DKPAGGSSYTL

SEQ ID NO: 606 - protein, 10 aa, Oryctolagus cuniculus
GGGIIYTQNL

SEQ ID NO: 607 - protein, 15 aa, Oryctolagus cuniculus
AGSVGYGYDTAYFNL

SEQ ID NO: 608 - protein, 9 aa, Oryctolagus cuniculus
TLNTLPFNI

SEQ ID NO: 609 - protein, 11 aa, Oryctolagus cuniculus
DLGDDGYAYGL

SEQ ID NO: 610 - protein, 11 aa, Oryctolagus cuniculus
GTGSSHYTSNL

SEQ ID NO: 611 - protein, 11 aa, Oryctolagus cuniculus
DLNGADSGSAL

SEQ ID NO: 612 - protein, 11 aa, Oryctolagus cuniculus
GGDADNFYYNI

SEQ ID NO: 613 - protein, 14 aa, Oryctolagus cuniculus
DFYAGSSGNVNGDI

SEQ ID NO: 614 - protein, 14 aa, Oryctolagus cuniculus
FPPGSNGGTAYFNI

SEQ ID NO: 615 - protein, 9 aa, Oryctolagus cuniculus
DSGWGAFDP

SEQ ID NO: 616 - protein, 9 aa, Oryctolagus cuniculus
DSGWGAFDP

SEQ ID NO: 617 - protein, 7 aa, Oryctolagus cuniculus
GYSDIDI

SEQ ID NO: 618 - protein, 14 aa, Oryctolagus cuniculus
FPPGSNGGTAYFNI

SEQ ID NO: 619 - protein, 15 aa, Oryctolagus cuniculus
GLGRGEYTSNDAFDP

SEQ ID NO: 620 - protein, 10 aa, Oryctolagus cuniculus
GSSDEIALDL

SEQ ID NO: 621 - protein, 13 aa, Oryctolagus cuniculus
GPYYVGSEYVFDP

SEQ ID NO: 622 - protein, 13 aa, Oryctolagus cuniculus
MFYAGDSGHYLHL

SEQ ID NO: 623 - protein, 3 aa, Oryctolagus cuniculus
NNL

SEQ ID NO: 624 - protein, 11 aa, Oryctolagus cuniculus
GGYSYGGAVSL

SEQ ID NO: 625 - protein, 11 aa, Oryctolagus cuniculus
GRSGGWDALDP

SEQ ID NO: 626 - protein, 13 aa, Oryctolagus cuniculus
EDYAGGTDYYFRL

SEQ ID NO: 627 - protein, 11 aa, Oryctolagus cuniculus
GGDADNFYYNI

SEQ ID NO: 628 - protein, 14 aa, Oryctolagus cuniculus
DFYAGSSGNVNGDI

SEQ ID NO: 629 - protein, 7 aa, Oryctolagus cuniculus
ELDYFNL

SEQ ID NO: 630 - protein, 14 aa, Oryctolagus cuniculus
DFYAGSSGNVNGDI

SEQ ID NO: 631 - protein, 10 aa, Oryctolagus cuniculus
GAGSNGDFNL

SEQ ID NO: 632 - protein, 11 aa, Oryctolagus cuniculus
GAGSYGGAVRL

SEQ ID NO: 633 - protein, 12 aa, Oryctolagus cuniculus
DGYDDYGDPFNL

SEQ ID NO: 634 - protein, 13 aa, Oryctolagus cuniculus
ISAGSDSYIIDNI

SEQ ID NO: 635 - protein, 11 aa, Oryctolagus cuniculus
DAGNSGYYINL

SEQ ID NO: 636 - protein, 4 aa, Oryctolagus cuniculus
LYKL

SEQ ID NO: 637 - protein, 11 aa, Oryctolagus cuniculus
PYVGYGYATDL

SEQ ID NO: 638 - protein, 11 aa, Oryctolagus cuniculus
DSYAGDYAFNL

SEQ ID NO: 639 - protein, 9 aa, Oryctolagus cuniculus
THNTLPFYI

SEQ ID NO: 640 - protein, 10 aa, Oryctolagus cuniculus
GSGGSDYFNL

SEQ ID NO: 641 - protein, 11 aa, Oryctolagus cuniculus
DLGADGYAYHL

SEQ ID NO: 642 - protein, 13 aa, Oryctolagus cuniculus
DPIYDDYGGRLDL

SEQ ID NO: 643 - protein, 14 aa, Oryctolagus cuniculus
FPPGSNGGTDYFNI

SEQ ID NO: 644 - protein, 11 aa, Oryctolagus cuniculus
DSYAGDYAFNL

SEQ ID NO: 645 - protein, 9 aa, Oryctolagus cuniculus
ARNTLPFNI

SEQ ID NO: 646 - protein, 14 aa, Oryctolagus cuniculus
GLYSASGWSYCFDI

SEQ ID NO: 647 - protein, 13 aa, Oryctolagus cuniculus
FDFLVGLTYAGVL

SEQ ID NO: 648 - protein, 13 aa, Oryctolagus cuniculus
NGASGTYYSSLYI

SEQ ID NO: 649 - protein, 14 aa, Oryctolagus cuniculus
FPPGSNSGTDYFNI

SEQ ID NO: 650 - protein, 6 aa, Oryctolagus cuniculus
GSGWDL

SEQ ID NO: 651 - protein, 11 aa, Oryctolagus cuniculus
GLGAASATWDI

SEQ ID NO: 652 - protein, 11 aa, Oryctolagus cuniculus
DKAGDSYYFNL

SEQ ID NO: 653 - protein, 7 aa, Oryctolagus cuniculus
GVAVGDI

SEQ ID NO: 654 - protein, 7 aa, Oryctolagus cuniculus
GILVSDL

SEQ ID NO: 655 - protein, 13 aa, Oryctolagus cuniculus
GPIMVVSPSYFNF

SEQ ID NO: 656 - protein, 15 aa, Oryctolagus cuniculus
SYYSGGYKYVYVFDL

SEQ ID NO: 657 - protein, 7 aa, Oryctolagus cuniculus
GIAVASL

SEQ ID NO: 658 - protein, 9 aa, Oryctolagus cuniculus
LDTYDDYDL

SEQ ID NO: 659 - protein, 13 aa, Oryctolagus cuniculus
MFYAGDSGHYFDL

SEQ ID NO: 660 - protein, 16 aa, Oryctolagus cuniculus
DSDYDDYGNSYYGMDP

SEQ ID NO: 661 - protein, 11 aa, Oryctolagus cuniculus
EYVGSQGYFNL

SEQ ID NO: 662 - protein, 13 aa, Oryctolagus cuniculus
FDYLVGGTWAGVL

SEQ ID NO: 663 - protein, 12 aa, Oryctolagus cuniculus
GVGDTTDTQLDL

SEQ ID NO: 664 - protein, 10 aa, Oryctolagus cuniculus
DPSAWGGLDL

SEQ ID NO: 665 - protein, 10 aa, Oryctolagus cuniculus
YNNGWDYFNL

SEQ ID NO: 666 - protein, 3 aa, Oryctolagus cuniculus
GSL

SEQ ID NO: 667 - protein, 14 aa, Oryctolagus cuniculus
RYGAGSGYFISPNL

SEQ ID NO: 668 - protein, 11 aa, Oryctolagus cuniculus
EYVDSQGYFNL

SEQ ID NO: 669 - protein, 11 aa, Oryctolagus cuniculus
GRSGGWDAFDP

SEQ ID NO: 670 - protein, 3 aa, Oryctolagus cuniculus
FDI

SEQ ID NO: 671 - protein, 11 aa, Oryctolagus cuniculus
DTGNSNYQFNL

SEQ ID NO: 672 - protein, 17 aa, Oryctolagus cuniculus
DDVSVGDANYPYTAFDL

SEQ ID NO: 673 - protein, 12 aa, Oryctolagus cuniculus
EAYSSANSYYDL

SEQ ID NO: 674 - protein, 12 aa, Oryctolagus cuniculus
DPTAAGGVYFDL

SEQ ID NO: 675 - protein, 9 aa, Oryctolagus cuniculus
GSGYSKFRL

SEQ ID NO: 676 - protein, 9 aa, Oryctolagus cuniculus
DRGDTDISL

SEQ ID NO: 677 - protein, 13 aa, Oryctolagus cuniculus
GPYYVNNENVFDP

SEQ ID NO: 678 - protein, 11 aa, Oryctolagus cuniculus
SYAGNRYDFAI

SEQ ID NO: 679 - protein, 7 aa, Oryctolagus cuniculus
GPYSFDF

SEQ ID NO: 680 - protein, 12 aa, Oryctolagus cuniculus
GDAYRDDYASDL

SEQ ID NO: 681 - protein, 12 aa, Oryctolagus cuniculus
YIGSVGYRRMDI

SEQ ID NO: 682 - protein, 13 aa, Oryctolagus cuniculus
MFYAGDSGHYFDL

SEQ ID NO: 683 - protein, 13 aa, Oryctolagus cuniculus
NGAGGYYYSSLYI

SEQ ID NO: 684 - protein, 9 aa, Oryctolagus cuniculus
DRGGTDISL

SEQ ID NO: 685 - protein, 11 aa, Oryctolagus cuniculus
SSSTYAYGFDP

SEQ ID NO: 686 - protein, 9 aa, Oryctolagus cuniculus
KGYFHYFNL

SEQ ID NO: 687 - protein, 11 aa, Oryctolagus cuniculus
DRAGNSYYFNL

SEQ ID NO: 688 - protein, 4 aa, Oryctolagus cuniculus
VWSL

SEQ ID NO: 689 - protein, 11 aa, Oryctolagus cuniculus
GYDGYGYVLVL

SEQ ID NO: 690 - protein, 12 aa, Oryctolagus cuniculus
DPTAAGGVYFDL

SEQ ID NO: 691 - protein, 14 aa, Oryctolagus cuniculus
GSGSIYYTPSYFDL

SEQ ID NO: 692 - protein, 3 aa, Oryctolagus cuniculus
SDI

SEQ ID NO: 693 - protein, 10 aa, Oryctolagus cuniculus
DDKVEHGYGL

SEQ ID NO: 694 - protein, 19 aa, Oryctolagus cuniculus
SMEAYGYAGYAMPGYYFNL

SEQ ID NO: 695 - protein, 16 aa, Oryctolagus cuniculus
DSDYDDYGDSYYGMDP

SEQ ID NO: 696 - protein, 18 aa, Oryctolagus cuniculus
DYDTYDYDGYTYAAGFDL

SEQ ID NO: 697 - protein, 11 aa, Oryctolagus cuniculus
GLGGASTTWDI

SEQ ID NO: 698 - protein, 14 aa, Oryctolagus cuniculus
DIITDSVWITRLDL

SEQ ID NO: 699 - protein, 13 aa, Oryctolagus cuniculus
FDYLVGDTYAGVL

SEQ ID NO: 700 - protein, 14 aa, Oryctolagus cuniculus
MFYAGDSSGNYLHL

SEQ ID NO: 701 - protein, 12 aa, Oryctolagus cuniculus
EGSSAYPSYFNF

SEQ ID NO: 702 - protein, 11 aa, Oryctolagus cuniculus
SYGGNRYDFNI

SEQ ID NO: 703 - protein, 14 aa, Oryctolagus cuniculus
MFYAGHTSGHYFDL

SEQ ID NO: 704 - protein, 21 aa, Oryctolagus cuniculus
GFDYTYGDAGYTYSTSHYFNL

SEQ ID NO: 705 - protein, 11 aa, Oryctolagus cuniculus
EGADYQGHFNL

SEQ ID NO: 706 - protein, 16 aa, Oryctolagus cuniculus
DSDYDDYGNSYYGMDP

SEQ ID NO: 707 - protein, 14 aa, Oryctolagus cuniculus
EIGSGYDAPYYFNL

SEQ ID NO: 708 - protein, 10 aa, Oryctolagus cuniculus
DDRVEHGYGL

SEQ ID NO: 709 - protein, 11 aa, Oryctolagus cuniculus
DLSSSIYDMDL

SEQ ID NO: 710 - protein, 12 aa, Oryctolagus cuniculus
VLNGWGEYYFNL

SEQ ID NO: 711 - protein, 7 aa, Oryctolagus cuniculus
GVAAGDI

SEQ ID NO: 712 - protein, 7 aa, Oryctolagus cuniculus
NISGSAV

SEQ ID NO: 713 - protein, 11 aa, Oryctolagus cuniculus
GGDGYGYVLVL

SEQ ID NO: 714 - protein, 7 aa, Oryctolagus cuniculus
GISYALL

SEQ ID NO: 715 - protein, 10 aa, Oryctolagus cuniculus
GGVGHEVNNL

SEQ ID NO: 716 - protein, 12 aa, Oryctolagus cuniculus
KLSDWDYGYFNL

SEQ ID NO: 717 - protein, 18 aa, Oryctolagus cuniculus
GYAGYYGYGYPTPSWLDL

SEQ ID NO: 718 - protein, 13 aa, Oryctolagus cuniculus
GGTTGSNYYGMDP

SEQ ID NO: 719 - protein, 4 aa, Oryctolagus cuniculus
GIRF

SEQ ID NO: 720 - protein, 17 aa, Oryctolagus cuniculus
VLGAGSSYYTSYDRLDL

SEQ ID NO: 721 - protein, 10 aa, Oryctolagus cuniculus
IADVNTQLDL

SEQ ID NO: 722 - protein, 11 aa, Oryctolagus cuniculus
GAGYAGYGFNL

SEQ ID NO: 723 - protein, 15 aa, Oryctolagus cuniculus
GNAGSYWDIYYGMDL

SEQ ID NO: 724 - protein, 10 aa, Oryctolagus cuniculus
GSGGYFVDNL

SEQ ID NO: 725 - protein, 13 aa, Oryctolagus cuniculus
MFYAGDSGHYFDL

SEQ ID NO: 726 - protein, 12 aa, Oryctolagus cuniculus
DHPAFSTVDLDI

SEQ ID NO: 727 - protein, 11 aa, Oryctolagus cuniculus
DAGSSGYYINL

SEQ ID NO: 728 - protein, 10 aa, Oryctolagus cuniculus
YNNGWDYFNL

SEQ ID NO: 729 - protein, 11 aa, Oryctolagus cuniculus
HKPAGGSSYIL

SEQ ID NO: 730 - protein, 7 aa, Oryctolagus cuniculus
GILVSNL

SEQ ID NO: 731 - protein, 7 aa, Oryctolagus cuniculus
GTYPFTL

SEQ ID NO: 732 - protein, 13 aa, Oryctolagus cuniculus
GSGYGTGWDAFDP

SEQ ID NO: 733 - protein, 9 aa, Oryctolagus cuniculus
GSTNMEFWF

SEQ ID NO: 734 - protein, 14 aa, Oryctolagus cuniculus
ADYYPDTTGWYLNI

SEQ ID NO: 735 - protein, 8 aa, Oryctolagus cuniculus
DGDSYFKL

SEQ ID NO: 736 - protein, 11 aa, Oryctolagus cuniculus
DSYGGDYAFNL

SEQ ID NO: 737 - protein, 12 aa, Oryctolagus cuniculus
DGYDDYGDPFNL

SEQ ID NO: 738 - protein, 18 aa, Oryctolagus cuniculus
LHYSPYGDAGYPYVSFNL

SEQ ID NO: 739 - protein, 9 aa, Oryctolagus cuniculus
NGASGTFDI

SEQ ID NO: 740 - protein, 11 aa, Oryctolagus cuniculus
GGGSGGVDNNL

SEQ ID NO: 741 - protein, 13 aa, Oryctolagus cuniculus
QASQSLYNNKNLA

SEQ ID NO: 742 - protein, 13 aa, Oryctolagus cuniculus
QSSQSVYDKKWLG

SEQ ID NO: 743 - protein, 13 aa, Oryctolagus cuniculus
QASQSLYNNKNLA

SEQ ID NO: 744 - protein, 13 aa, Oryctolagus cuniculus
QSSESVYNNNLLS

SEQ ID NO: 745 - protein, 11 aa, Oryctolagus cuniculus
QASQSVSNLLA

SEQ ID NO: 746 - protein, 13 aa, Oryctolagus cuniculus
QASQSLYNNKNLA

SEQ ID NO: 747 - protein, 11 aa, Oryctolagus cuniculus
QASEDIESYLA

SEQ ID NO: 748 - protein, 13 aa, Oryctolagus cuniculus
QASQSLYNNKNLG

SEQ ID NO: 749 - protein, 11 aa, Oryctolagus cuniculus
QASQTISSYLA

SEQ ID NO: 750 - protein, 13 aa, Oryctolagus cuniculus
QSSQSVYDNNALA

SEQ ID NO: 751 - protein, 13 aa, Oryctolagus cuniculus
QSSQNVDRNNRLA

SEQ ID NO: 752 - protein, 11 aa, Oryctolagus cuniculus
QASQSIGSNLA

SEQ ID NO: 753 - protein, 11 aa, Oryctolagus cuniculus
QASEDIESYLA

SEQ ID NO: 754 - protein, 11 aa, Oryctolagus cuniculus
QASEDIESYLA

SEQ ID NO: 755 - protein, 11 aa, Oryctolagus cuniculus
QASQNIYDNLA

SEQ ID NO: 756 - protein, 13 aa, Oryctolagus cuniculus
QSSPSVYNNNRLS

SEQ ID NO: 757 - protein, 11 aa, Oryctolagus cuniculus
QASQNIGNNLA

SEQ ID NO: 758 - protein, 11 aa, Oryctolagus cuniculus
QASEDIESYLA

SEQ ID NO: 759 - protein, 11 aa, Oryctolagus cuniculus
QASQNINSWLS

SEQ ID NO: 760 - protein, 13 aa, Oryctolagus cuniculus
QSSQSVYSNNHLA

SEQ ID NO: 761 - protein, 13 aa, Oryctolagus cuniculus
QSSQIVHNNNNLA

SEQ ID NO: 762 - protein, 13 aa, Oryctolagus cuniculus
QASQSLYNKKNLA

SEQ ID NO: 763 - protein, 13 aa, Oryctolagus cuniculus
QSSQSVYDNKWLG

SEQ ID NO: 764 - protein, 13 aa, Oryctolagus cuniculus
QSSQSVYDNKWLG

SEQ ID NO: 765 - protein, 13 aa, Oryctolagus cuniculus
QSSKSVFDNNWLS

SEQ ID NO: 766 - protein, 13 aa, Oryctolagus cuniculus
QASQSLYNKKNLA

SEQ ID NO: 767 - protein, 11 aa, Oryctolagus cuniculus
QASETIYSYLN

SEQ ID NO: 768 - protein, 13 aa, Oryctolagus cuniculus
QSSQNIYNKNQLS

SEQ ID NO: 769 - protein, 11 aa, Oryctolagus cuniculus
QASQSIGGSLA

SEQ ID NO: 770 - protein, 13 aa, Oryctolagus cuniculus
QSSQSVNNNKNLA

SEQ ID NO: 771 - protein, 11 aa, Oryctolagus cuniculus
QASQNIGSTLA

SEQ ID NO: 772 - protein, 11 aa, Oryctolagus cuniculus
QASEDIETYLA

SEQ ID NO: 773 - protein, 11 aa, Oryctolagus cuniculus
QASEDIENYLA

SEQ ID NO: 774 - protein, 12 aa, Oryctolagus cuniculus
QSSQSVDNNWLS

SEQ ID NO: 775 - protein, 13 aa, Oryctolagus cuniculus
QSSQSVYSNNHLA

SEQ ID NO: 776 - protein, 13 aa, Oryctolagus cuniculus
QSSQSVHNNNNLA

SEQ ID NO: 777 - protein, 11 aa, Oryctolagus cuniculus
QASEDISSSLA

SEQ ID NO: 778 - protein, 13 aa, Oryctolagus cuniculus
QASQSVHNNNNLA

SEQ ID NO: 779 - protein, 11 aa, Oryctolagus cuniculus
QASEDIESYLA

SEQ ID NO: 780 - protein, 11 aa, Oryctolagus cuniculus
QATEDIESFLA

SEQ ID NO: 781 - protein, 11 aa, Oryctolagus cuniculus
RASEDIKSYLA

SEQ ID NO: 782 - protein, 13 aa, Oryctolagus cuniculus
QASQSVYNHKNLA

SEQ ID NO: 783 - protein, 11 aa, Oryctolagus cuniculus
QASQSIGSSLA

SEQ ID NO: 784 - protein, 13 aa, Oryctolagus cuniculus
QSSQSVYGVNELS

SEQ ID NO: 785 - protein, 11 aa, Oryctolagus cuniculus
QASQSISNLLA

SEQ ID NO: 786 - protein, 13 aa, Oryctolagus cuniculus
QSSKSVYNNNWLS

SEQ ID NO: 787 - protein, 13 aa, Oryctolagus cuniculus
QSSPSVYNNNRLS

SEQ ID NO: 788 - protein, 11 aa, Oryctolagus cuniculus
QASQSIGSYLS

SEQ ID NO: 789 - protein, 11 aa, Oryctolagus cuniculus
QASQNIGNNLA

SEQ ID NO: 790 - protein, 11 aa, Oryctolagus cuniculus
QASEDIYSNLA

SEQ ID NO: 791 - protein, 13 aa, Oryctolagus cuniculus
QASQSLYNNKNLA

SEQ ID NO: 792 - protein, 13 aa, Oryctolagus cuniculus
QSSKTVYNNNWLA

SEQ ID NO: 793 - protein, 13 aa, Oryctolagus cuniculus
QSSPSVYNNVRLS

SEQ ID NO: 794 - protein, 12 aa, Oryctolagus cuniculus
QSSQSVYSTNLA

SEQ ID NO: 795 - protein, 11 aa, Oryctolagus cuniculus
QASENIANHLA

SEQ ID NO: 796 - protein, 13 aa, Oryctolagus cuniculus
QSSQSVYGNNELS

SEQ ID NO: 797 - protein, 13 aa, Oryctolagus cuniculus
QASQSLYNKKNLA

SEQ ID NO: 798 - protein, 13 aa, Oryctolagus cuniculus
QSSQSVYGSDALA

SEQ ID NO: 799 - protein, 11 aa, Oryctolagus cuniculus
QASQSISSNLA

SEQ ID NO: 800 - protein, 11 aa, Oryctolagus cuniculus
QASENIYSFLA

SEQ ID NO: 801 - protein, 11 aa, Oryctolagus cuniculus
QASQSISDYLS

SEQ ID NO: 802 - protein, 11 aa, Oryctolagus cuniculus
QASQSISSYLS

SEQ ID NO: 803 - protein, 11 aa, Oryctolagus cuniculus
QASQNINNLLA

SEQ ID NO: 804 - protein, 13 aa, Oryctolagus cuniculus
QASQSVYANNYLA

SEQ ID NO: 805 - protein, 11 aa, Oryctolagus cuniculus
QASESISNYLS

SEQ ID NO: 806 - protein, 13 aa, Oryctolagus cuniculus
QSSQSVYNNNWLS

SEQ ID NO: 807 - protein, 13 aa, Oryctolagus cuniculus
QASQSVHKHKNLA

SEQ ID NO: 808 - protein, 11 aa, Oryctolagus cuniculus
QASQSISSYLS

SEQ ID NO: 809 - protein, 11 aa, Oryctolagus cuniculus
QASQNINNELS

SEQ ID NO: 810 - protein, 11 aa, Oryctolagus cuniculus
RASEDIESYLA

SEQ ID NO: 811 - protein, 13 aa, Oryctolagus cuniculus
QSSQSVYNDNDLA

SEQ ID NO: 812 - protein, 11 aa, Oryctolagus cuniculus
QASESIYSGLA

SEQ ID NO: 813 - protein, 11 aa, Oryctolagus cuniculus
QASQSISYYLN

SEQ ID NO: 814 - protein, 13 aa, Oryctolagus cuniculus
QASQSVYKNNYLA

SEQ ID NO: 815 - protein, 13 aa, Oryctolagus cuniculus
QSSQSVYNNNWLG

SEQ ID NO: 816 - protein, 11 aa, Oryctolagus cuniculus
QASEDIYNLLA

SEQ ID NO: 817 - protein, 11 aa, Oryctolagus cuniculus
QASEDIESYLA

SEQ ID NO: 818 - protein, 13 aa, Oryctolagus cuniculus
QASQSVYSNNYLS

SEQ ID NO: 819 - protein, 11 aa, Oryctolagus cuniculus
QASESIDSYLN

SEQ ID NO: 820 - protein, 11 aa, Oryctolagus cuniculus
QASQNIYSSLA

SEQ ID NO: 821 - protein, 11 aa, Oryctolagus cuniculus
QASQSISYYLA

SEQ ID NO: 822 - protein, 11 aa, Oryctolagus cuniculus
QASQNIYSRLA

SEQ ID NO: 823 - protein, 12 aa, Oryctolagus cuniculus
QSSQSVTDNFLS

SEQ ID NO: 824 - protein, 11 aa, Oryctolagus cuniculus
QASEDIESYLA

SEQ ID NO: 825 - protein, 11 aa, Oryctolagus cuniculus
QASQSIGSSLA

SEQ ID NO: 826 - protein, 11 aa, Oryctolagus cuniculus
QASQSISSYLA

SEQ ID NO: 827 - protein, 11 aa, Oryctolagus cuniculus
QASQNIGSDLA

SEQ ID NO: 828 - protein, 11 aa, Oryctolagus cuniculus
QASQSISSYLA

SEQ ID NO: 829 - protein, 13 aa, Oryctolagus cuniculus
QASESVVGKNELS

SEQ ID NO: 830 - protein, 13 aa, Oryctolagus cuniculus
QASQSVHNNKNLA

SEQ ID NO: 831 - protein, 13 aa, Oryctolagus cuniculus
QSSQSVYRNNELS

SEQ ID NO: 832 - protein, 11 aa, Oryctolagus cuniculus
QASEDIESFLA

SEQ ID NO: 833 - protein, 11 aa, Oryctolagus cuniculus
QASEDISSRLA

SEQ ID NO: 834 - protein, 11 aa, Oryctolagus cuniculus
QASQNIYSNLA

SEQ ID NO: 835 - protein, 11 aa, Oryctolagus cuniculus
QASENIYSFLA

SEQ ID NO: 836 - protein, 13 aa, Oryctolagus cuniculus
QSSQSVADNNLLA

SEQ ID NO: 837 - protein, 13 aa, Oryctolagus cuniculus
QASQSVYGTNRLA

SEQ ID NO: 838 - protein, 11 aa, Oryctolagus cuniculus
QASQNIYSKFA

SEQ ID NO: 839 - protein, 11 aa, Oryctolagus cuniculus
QASQSIGVSLA

SEQ ID NO: 840 - protein, 13 aa, Oryctolagus cuniculus
QASQSVYNNNYLG

SEQ ID NO: 841 - protein, 11 aa, Oryctolagus cuniculus
QASESIDNWLA

SEQ ID NO: 842 - protein, 13 aa, Oryctolagus cuniculus
QSSQSVYSNNNLA

SEQ ID NO: 843 - protein, 11 aa, Oryctolagus cuniculus
QASQSISSYLS

SEQ ID NO: 844 - protein, 11 aa, Oryctolagus cuniculus
QASQSIRSYLA

SEQ ID NO: 845 - protein, 11 aa, Oryctolagus cuniculus
QASESISVNLA

SEQ ID NO: 846 - protein, 13 aa, Oryctolagus cuniculus
QSSESIYKNNYLA

SEQ ID NO: 847 - protein, 11 aa, Oryctolagus cuniculus
QASQNIYSDFA

SEQ ID NO: 848 - protein, 13 aa, Oryctolagus cuniculus
QASQSVYNHKNLA

SEQ ID NO: 849 - protein, 11 aa, Oryctolagus cuniculus
QASQSISAYLS

SEQ ID NO: 850 - protein, 11 aa, Oryctolagus cuniculus
QASQTITSYLA

SEQ ID NO: 851 - protein, 13 aa, Oryctolagus cuniculus
QASQSVYNNKNLA

SEQ ID NO: 852 - protein, 11 aa, Oryctolagus cuniculus
QASENIYSLLA

SEQ ID NO: 853 - protein, 11 aa, Oryctolagus cuniculus
QASEDIYSLLA

SEQ ID NO: 854 - protein, 11 aa, Oryctolagus cuniculus
QASQSISTYLS

SEQ ID NO: 855 - protein, 11 aa, Oryctolagus cuniculus
QASENIYSSLA

SEQ ID NO: 856 - protein, 11 aa, Oryctolagus cuniculus
QASESIGSWLA

SEQ ID NO: 857 - protein, 13 aa, Oryctolagus cuniculus
QSSQSVYNNNRLS

SEQ ID NO: 858 - protein, 13 aa, Oryctolagus cuniculus
QASQSVYNNNNLA

SEQ ID NO: 859 - protein, 11 aa, Oryctolagus cuniculus
QASQSIGSYLS

SEQ ID NO: 860 - protein, 13 aa, Oryctolagus cuniculus
QSSESVYNNNLLS

SEQ ID NO: 861 - protein, 12 aa, Oryctolagus cuniculus
QASQSVYNNRLA

SEQ ID NO: 862 - protein, 11 aa, Oryctolagus cuniculus
QASQSISTYSS

SEQ ID NO: 863 - protein, 13 aa, Oryctolagus cuniculus
QSSQSVYASVWLG

SEQ ID NO: 864 - protein, 11 aa, Oryctolagus cuniculus
QASQSIYNYLS

SEQ ID NO: 865 - protein, 11 aa, Oryctolagus cuniculus
QASQNIYSYLA

SEQ ID NO: 866 - protein, 11 aa, Oryctolagus cuniculus
QASQSIYSYLA

SEQ ID NO: 867 - protein, 11 aa, Oryctolagus cuniculus
QASESIGSVLA

SEQ ID NO: 868 - protein, 11 aa, Oryctolagus cuniculus
QASQNIYSNLA

SEQ ID NO: 869 - protein, 13 aa, Oryctolagus cuniculus
QSNKNVYDNNALS

SEQ ID NO: 870 - protein, 11 aa, Oryctolagus cuniculus
QASQSIINYLS

SEQ ID NO: 871 - protein, 11 aa, Oryctolagus cuniculus
QASQSIYSYLS

SEQ ID NO: 872 - protein, 11 aa, Oryctolagus cuniculus
QASQSISSWLA

SEQ ID NO: 873 - protein, 13 aa, Oryctolagus cuniculus
QSSQSVNNAKNLA

SEQ ID NO: 874 - protein, 13 aa, Oryctolagus cuniculus
QSSKSVYDNNWLS

SEQ ID NO: 875 - protein, 11 aa, Oryctolagus cuniculus
QASQSIGSSLA

SEQ ID NO: 876 - protein, 11 aa, Oryctolagus cuniculus
QASENIYRNLA

SEQ ID NO: 877 - protein, 11 aa, Oryctolagus cuniculus
QASEDIESYLA

SEQ ID NO: 878 - protein, 11 aa, Oryctolagus cuniculus
QASQSISSWLS

SEQ ID NO: 879 - protein, 11 aa, Oryctolagus cuniculus
QASQSIGSDLA

SEQ ID NO: 880 - protein, 11 aa, Oryctolagus cuniculus
QGSQSISSYLS

SEQ ID NO: 881 - protein, 12 aa, Oryctolagus cuniculus
QSSPSVYSVYLS

SEQ ID NO: 882 - protein, 13 aa, Oryctolagus cuniculus
QSSKSVYNNKWLS

SEQ ID NO: 883 - protein, 11 aa, Oryctolagus cuniculus
QASESVGDALA

SEQ ID NO: 884 - protein, 13 aa, Oryctolagus cuniculus
QSSKTIYNDNWLS

SEQ ID NO: 885 - protein, 11 aa, Oryctolagus cuniculus
RASEDIKSYLA

SEQ ID NO: 886 - protein, 11 aa, Oryctolagus cuniculus
QASQSIYSNLA

SEQ ID NO: 887 - protein, 13 aa, Oryctolagus cuniculus
QASQSVYNNNYLA

SEQ ID NO: 888 - protein, 11 aa, Oryctolagus cuniculus
RASEDIERFLA

SEQ ID NO: 889 - protein, 7 aa, Oryctolagus cuniculus
DVSTLAS

SEQ ID NO: 890 - protein, 7 aa, Oryctolagus cuniculus
KASTLAS

SEQ ID NO: 891 - protein, 7 aa, Oryctolagus cuniculus
DVSTLAS

SEQ ID NO: 892 - protein, 7 aa, Oryctolagus cuniculus
TTSSLAS

SEQ ID NO: 893 - protein, 7 aa, Oryctolagus cuniculus
GASNLES

SEQ ID NO: 894 - protein, 7 aa, Oryctolagus cuniculus
DASTLAS

SEQ ID NO: 895 - protein, 7 aa, Oryctolagus cuniculus
DASDLAS

SEQ ID NO: 896 - protein, 7 aa, Oryctolagus cuniculus
DVSTLAS

SEQ ID NO: 897 - protein, 7 aa, Oryctolagus cuniculus
GASTLAS

SEQ ID NO: 898 - protein, 7 aa, Oryctolagus cuniculus
ETSTLAS

SEQ ID NO: 899 - protein, 7 aa, Oryctolagus cuniculus
YASILAS

SEQ ID NO: 900 - protein, 7 aa, Oryctolagus cuniculus
KASTLAS

SEQ ID NO: 901 - protein, 7 aa, Oryctolagus cuniculus
QASKLAS

SEQ ID NO: 902 - protein, 7 aa, Oryctolagus cuniculus
SASTLAS

SEQ ID NO: 903 - protein, 7 aa, Oryctolagus cuniculus
GASNLES

SEQ ID NO: 904 - protein, 7 aa, Oryctolagus cuniculus
YASTLAS

SEQ ID NO: 905 - protein, 7 aa, Oryctolagus cuniculus
YASTLAS

SEQ ID NO: 906 - protein, 7 aa, Oryctolagus cuniculus
GASNLAS

SEQ ID NO: 907 - protein, 7 aa, Oryctolagus cuniculus
KASTLAS

SEQ ID NO: 908 - protein, 7 aa, Oryctolagus cuniculus
RASKLAS

SEQ ID NO: 909 - protein, 7 aa, Oryctolagus cuniculus
QASTLAS

SEQ ID NO: 910 - protein, 7 aa, Oryctolagus cuniculus
DASTLTS

SEQ ID NO: 911 - protein, 7 aa, Oryctolagus cuniculus
SASTLAS

SEQ ID NO: 912 - protein, 7 aa, Oryctolagus cuniculus
KASTLAS

SEQ ID NO: 913 - protein, 7 aa, Oryctolagus cuniculus
KASTLAS

SEQ ID NO: 914 - protein, 7 aa, Oryctolagus cuniculus
DASTLAS

SEQ ID NO: 915 - protein, 7 aa, Oryctolagus cuniculus
SASTLAS

SEQ ID NO: 916 - protein, 7 aa, Oryctolagus cuniculus
EASKLAS

SEQ ID NO: 917 - protein, 7 aa, Oryctolagus cuniculus
SASNLAS

SEQ ID NO: 918 - protein, 7 aa, Oryctolagus cuniculus
DTSTLAS

SEQ ID NO: 919 - protein, 7 aa, Oryctolagus cuniculus
GASTLSS

SEQ ID NO: 920 - protein, 7 aa, Oryctolagus cuniculus
RASTLAS

SEQ ID NO: 921 - protein, 7 aa, Oryctolagus cuniculus
SASTLAS

SEQ ID NO: 922 - protein, 7 aa, Oryctolagus cuniculus
TTSKLAS

SEQ ID NO: 923 - protein, 7 aa, Oryctolagus cuniculus
RASKLAS

SEQ ID NO: 924 - protein, 7 aa, Oryctolagus cuniculus
QASTLAS

SEQ ID NO: 925 - protein, 7 aa, Oryctolagus cuniculus
RASNLAS

SEQ ID NO: 926 - protein, 7 aa, Oryctolagus cuniculus
QASTLAS

SEQ ID NO: 927 - protein, 7 aa, Oryctolagus cuniculus
RASTLAS

SEQ ID NO: 928 - protein, 7 aa, Oryctolagus cuniculus
RASTLES

SEQ ID NO: 929 - protein, 7 aa, Oryctolagus cuniculus
DASDLAS

SEQ ID NO: 930 - protein, 7 aa, Oryctolagus cuniculus
DTSTLAS

SEQ ID NO: 931 - protein, 7 aa, Oryctolagus cuniculus
YVSNLES

SEQ ID NO: 932 - protein, 7 aa, Oryctolagus cuniculus
KAATLAS

SEQ ID NO: 933 - protein, 7 aa, Oryctolagus cuniculus
DASDLAS

SEQ ID NO: 934 - protein, 7 aa, Oryctolagus cuniculus
GASTLAS

SEQ ID NO: 935 - protein, 7 aa, Oryctolagus cuniculus
YASTLAS

SEQ ID NO: 936 - protein, 7 aa, Oryctolagus cuniculus
DASTLAS

SEQ ID NO: 937 - protein, 7 aa, Oryctolagus cuniculus
DASDLAS

SEQ ID NO: 938 - protein, 7 aa, Oryctolagus cuniculus
SASTLAS

SEQ ID NO: 939 - protein, 7 aa, Oryctolagus cuniculus
DVSTLAS

SEQ ID NO: 940 - protein, 7 aa, Oryctolagus cuniculus
GASTLAS

SEQ ID NO: 941 - protein, 7 aa, Oryctolagus cuniculus
SASTLAS

SEQ ID NO: 942 - protein, 7 aa, Oryctolagus cuniculus
YASTLAS

SEQ ID NO: 943 - protein, 7 aa, Oryctolagus cuniculus
SASALAS

SEQ ID NO: 944 - protein, 7 aa, Oryctolagus cuniculus
DASKLAS

SEQ ID NO: 945 - protein, 7 aa, Oryctolagus cuniculus
DVSTLAS

SEQ ID NO: 946 - protein, 7 aa, Oryctolagus cuniculus
GASTLAS

SEQ ID NO: 947 - protein, 7 aa, Oryctolagus cuniculus
LASTLAS

SEQ ID NO: 948 - protein, 7 aa, Oryctolagus cuniculus
SASTLES

SEQ ID NO: 949 - protein, 7 aa, Oryctolagus cuniculus
RASNLAS

SEQ ID NO: 950 - protein, 7 aa, Oryctolagus cuniculus
DASDLAS

SEQ ID NO: 951 - protein, 7 aa, Oryctolagus cuniculus
KASTLAS

SEQ ID NO: 952 - protein, 7 aa, Oryctolagus cuniculus
KASTLAS

SEQ ID NO: 953 - protein, 7 aa, Oryctolagus cuniculus
YDSTLES

SEQ ID NO: 954 - protein, 7 aa, Oryctolagus cuniculus
GASTLAS

SEQ ID NO: 955 - protein, 7 aa, Oryctolagus cuniculus
EASKLAS

SEQ ID NO: 956 - protein, 7 aa, Oryctolagus cuniculus
RASSLKS

SEQ ID NO: 957 - protein, 7 aa, Oryctolagus cuniculus
KASTLAS

SEQ ID NO: 958 - protein, 7 aa, Oryctolagus cuniculus
SASSLAS

SEQ ID NO: 959 - protein, 7 aa, Oryctolagus cuniculus
GASTLAS

SEQ ID NO: 960 - protein, 7 aa, Oryctolagus cuniculus
RASTLES

SEQ ID NO: 961 - protein, 7 aa, Oryctolagus cuniculus
RASTLAS

SEQ ID NO: 962 - protein, 7 aa, Oryctolagus cuniculus
SASTLDS

SEQ ID NO: 963 - protein, 7 aa, Oryctolagus cuniculus
SASTLAS

SEQ ID NO: 964 - protein, 7 aa, Oryctolagus cuniculus
GASTLAS

SEQ ID NO: 965 - protein, 7 aa, Oryctolagus cuniculus
GASTLAS

SEQ ID NO: 966 - protein, 7 aa, Oryctolagus cuniculus
DASDLAS

SEQ ID NO: 967 - protein, 7 aa, Oryctolagus cuniculus
GASTLAS

SEQ ID NO: 968 - protein, 7 aa, Oryctolagus cuniculus
GASNLES

SEQ ID NO: 969 - protein, 7 aa, Oryctolagus cuniculus
RASTLAS

SEQ ID NO: 970 - protein, 7 aa, Oryctolagus cuniculus
AASTLAS

SEQ ID NO: 971 - protein, 7 aa, Oryctolagus cuniculus
GASTLAS

SEQ ID NO: 972 - protein, 7 aa, Oryctolagus cuniculus
SASTLAS

SEQ ID NO: 973 - protein, 7 aa, Oryctolagus cuniculus
SASNLAS

SEQ ID NO: 974 - protein, 7 aa, Oryctolagus cuniculus
RTSILES

SEQ ID NO: 975 - protein, 7 aa, Oryctolagus cuniculus
DASALAS

SEQ ID NO: 976 - protein, 7 aa, Oryctolagus cuniculus
RASTLAS

SEQ ID NO: 977 - protein, 7 aa, Oryctolagus cuniculus
GTSTLAS

SEQ ID NO: 978 - protein, 7 aa, Oryctolagus cuniculus
DVSTVAS

SEQ ID NO: 979 - protein, 7 aa, Oryctolagus cuniculus
DASNLAS

SEQ ID NO: 980 - protein, 7 aa, Oryctolagus cuniculus
SASTLAS

SEQ ID NO: 981 - protein, 7 aa, Oryctolagus cuniculus
RASTLAS

SEQ ID NO: 982 - protein, 7 aa, Oryctolagus cuniculus
GASNLES

SEQ ID NO: 983 - protein, 7 aa, Oryctolagus cuniculus
DSSTLAS

SEQ ID NO: 984 - protein, 7 aa, Oryctolagus cuniculus
KASTLAS

SEQ ID NO: 985 - protein, 7 aa, Oryctolagus cuniculus
DASTLAS

SEQ ID NO: 986 - protein, 7 aa, Oryctolagus cuniculus
SASTLAS

SEQ ID NO: 987 - protein, 7 aa, Oryctolagus cuniculus
SASTLAS

SEQ ID NO: 988 - protein, 7 aa, Oryctolagus cuniculus
SASKLES

SEQ ID NO: 989 - protein, 7 aa, Oryctolagus cuniculus
SASNLAS

SEQ ID NO: 990 - protein, 7 aa, Oryctolagus cuniculus
DASNLAS

SEQ ID NO: 991 - protein, 7 aa, Oryctolagus cuniculus
RASSLES

SEQ ID NO: 992 - protein, 7 aa, Oryctolagus cuniculus
RASTLES

SEQ ID NO: 993 - protein, 7 aa, Oryctolagus cuniculus
LASTLAS

SEQ ID NO: 994 - protein, 7 aa, Oryctolagus cuniculus
RASTLTS

SEQ ID NO: 995 - protein, 7 aa, Oryctolagus cuniculus
SASALAS

SEQ ID NO: 996 - protein, 7 aa, Oryctolagus cuniculus
SASSLAS

SEQ ID NO: 997 - protein, 7 aa, Oryctolagus cuniculus
DASDLAS

SEQ ID NO: 998 - protein, 7 aa, Oryctolagus cuniculus
RASILES

SEQ ID NO: 999 - protein, 7 aa, Oryctolagus cuniculus
DASKLAS

SEQ ID NO: 1000 - protein, 7 aa, Oryctolagus cuniculus
RASTLAS

SEQ ID NO: 1001 - protein, 7 aa, Oryctolagus cuniculus
AASTLAS

SEQ ID NO: 1002 - protein, 7 aa, Oryctolagus cuniculus
RATTLES

SEQ ID NO: 1003 - protein, 7 aa, Oryctolagus cuniculus
DASDLAS

SEQ ID NO: 1004 - protein, 7 aa, Oryctolagus cuniculus
SASSLAS

SEQ ID NO: 1005 - protein, 7 aa, Oryctolagus cuniculus
RSSTLAS

SEQ ID NO: 1006 - protein, 7 aa, Oryctolagus cuniculus
TASSLAS

SEQ ID NO: 1007 - protein, 7 aa, Oryctolagus cuniculus
YASDLES

SEQ ID NO: 1008 - protein, 7 aa, Oryctolagus cuniculus
KASTLDS

SEQ ID NO: 1009 - protein, 7 aa, Oryctolagus cuniculus
EASTLTS

SEQ ID NO: 1010 - protein, 7 aa, Oryctolagus cuniculus
YASDLES

SEQ ID NO: 1011 - protein, 7 aa, Oryctolagus cuniculus
AASTLAS

SEQ ID NO: 1012 - protein, 7 aa, Oryctolagus cuniculus
GASDLAS

SEQ ID NO: 1013 - protein, 7 aa, Oryctolagus cuniculus
DASDLES

SEQ ID NO: 1014 - protein, 7 aa, Oryctolagus cuniculus
GASTLAS

SEQ ID NO: 1015 - protein, 7 aa, Oryctolagus cuniculus
SASTLAS

SEQ ID NO: 1016 - protein, 7 aa, Oryctolagus cuniculus
GASDLES

SEQ ID NO: 1017 - protein, 7 aa, Oryctolagus cuniculus
RASTLAS

SEQ ID NO: 1018 - protein, 7 aa, Oryctolagus cuniculus
RASTLES

SEQ ID NO: 1019 - protein, 7 aa, Oryctolagus cuniculus
QASILAS

SEQ ID NO: 1020 - protein, 7 aa, Oryctolagus cuniculus
RASTLES

SEQ ID NO: 1021 - protein, 7 aa, Oryctolagus cuniculus
DASTLAS

SEQ ID NO: 1022 - protein, 7 aa, Oryctolagus cuniculus
QASTLAS

SEQ ID NO: 1023 - protein, 7 aa, Oryctolagus cuniculus
YTSTLAS

SEQ ID NO: 1024 - protein, 7 aa, Oryctolagus cuniculus
KASTLAS

SEQ ID NO: 1025 - protein, 7 aa, Oryctolagus cuniculus
SASTLAS

SEQ ID NO: 1026 - protein, 7 aa, Oryctolagus cuniculus
DASDLAS

SEQ ID NO: 1027 - protein, 7 aa, Oryctolagus cuniculus
DASSLES

SEQ ID NO: 1028 - protein, 7 aa, Oryctolagus cuniculus
GASTLAS

SEQ ID NO: 1029 - protein, 7 aa, Oryctolagus cuniculus
RASTLAS

SEQ ID NO: 1030 - protein, 7 aa, Oryctolagus cuniculus
GAFTLAS

SEQ ID NO: 1031 - protein, 7 aa, Oryctolagus cuniculus
RASTLES

SEQ ID NO: 1032 - protein, 7 aa, Oryctolagus cuniculus
GASTLAS

SEQ ID NO: 1033 - protein, 7 aa, Oryctolagus cuniculus
DASDLAS

SEQ ID NO: 1034 - protein, 7 aa, Oryctolagus cuniculus
GASNLES

SEQ ID NO: 1035 - protein, 7 aa, Oryctolagus cuniculus
LASTLAS

SEQ ID NO: 1036 - protein, 7 aa, Oryctolagus cuniculus
KASTLAS

SEQ ID NO: 1037 - protein, 13 aa, Oryctolagus cuniculus
QGEFSCSSGDCYA

SEQ ID NO: 1038 - protein, 10 aa, Oryctolagus cuniculus
AGGYSGNIWS

SEQ ID NO: 1039 - protein, 13 aa, Oryctolagus cuniculus
QGEFSCSSGDCYA

SEQ ID NO: 1040 - protein, 10 aa, Oryctolagus cuniculus
QGGYTDATYA

SEQ ID NO: 1041 - protein, 6 aa, Oryctolagus cuniculus
QSGYYT

SEQ ID NO: 1042 - protein, 13 aa, Oryctolagus cuniculus
QGEFSCGSGDCYA

SEQ ID NO: 1043 - protein, 12 aa, Oryctolagus cuniculus
QSYYYGSSYVVA

SEQ ID NO: 1044 - protein, 13 aa, Oryctolagus cuniculus
QGEFSCSSGDCYA

SEQ ID NO: 1045 - protein, 13 aa, Oryctolagus cuniculus
LYSYYTSNSADNT

SEQ ID NO: 1046 - protein, 11 aa, Oryctolagus cuniculus
AGGYNSGSDAA

SEQ ID NO: 1047 - protein, 10 aa, Oryctolagus cuniculus
QGYYSGDINV

SEQ ID NO: 1048 - protein, 13 aa, Oryctolagus cuniculus
QSYYGTSNSYGDA

SEQ ID NO: 1049 - protein, 13 aa, Oryctolagus cuniculus
QCTLYGVNFVPNV

SEQ ID NO: 1050 - protein, 13 aa, Oryctolagus cuniculus
QCILYGVNFVPNT

SEQ ID NO: 1051 - protein, 13 aa, Oryctolagus cuniculus
QCSYDGGSYVPNA

SEQ ID NO: 1052 - protein, 11 aa, Oryctolagus cuniculus
AGGYSTISDNA

SEQ ID NO: 1053 - protein, 12 aa, Oryctolagus cuniculus
QCTFYGSGYVAA

SEQ ID NO: 1054 - protein, 13 aa, Oryctolagus cuniculus
QCGIYGVNFVPNV

SEQ ID NO: 1055 - protein, 12 aa, Oryctolagus cuniculus
QQGAGWNNLDNA

SEQ ID NO: 1056 - protein, 11 aa, Oryctolagus cuniculus
LGVYDDDADNA

SEQ ID NO: 1057 - protein, 12 aa, Oryctolagus cuniculus
AGGYSTNTDTYI

SEQ ID NO: 1058 - protein, 13 aa, Oryctolagus cuniculus
QGEFSCSAGDCYA

SEQ ID NO: 1059 - protein, 10 aa, Oryctolagus cuniculus
AGGYSGNIWS

SEQ ID NO: 1060 - protein, 10 aa, Oryctolagus cuniculus
AGGYSGNIWS

SEQ ID NO: 1061 - protein, 11 aa, Oryctolagus cuniculus
AGIYSSDSDNA

SEQ ID NO: 1062 - protein, 13 aa, Oryctolagus cuniculus
QGEFSCSSGDCYA

SEQ ID NO: 1063 - protein, 12 aa, Oryctolagus cuniculus
QQGYSGRNVENT

SEQ ID NO: 1064 - protein, 11 aa, Oryctolagus cuniculus
LGGYISSSDTT

SEQ ID NO: 1065 - protein, 12 aa, Oryctolagus cuniculus
QCTYYDDSYDVP

SEQ ID NO: 1066 - protein, 12 aa, Oryctolagus cuniculus
AGGYSSSADTFA

SEQ ID NO: 1067 - protein, 14 aa, Oryctolagus cuniculus
QSNYGSNSGGYVFP

SEQ ID NO: 1068 - protein, 13 aa, Oryctolagus cuniculus
QCTLYGVNFVANA

SEQ ID NO: 1069 - protein, 11 aa, Oryctolagus cuniculus
QSYYDGAVTFT

SEQ ID NO: 1070 - protein, 13 aa, Oryctolagus cuniculus
LGGYDSMSADCFA

SEQ ID NO: 1071 - protein, 11 aa, Oryctolagus cuniculus
LGVYDDDADNA

SEQ ID NO: 1072 - protein, 12 aa, Oryctolagus cuniculus
AGGYSTNTDTFT

SEQ ID NO: 1073 - protein, 14 aa, Oryctolagus cuniculus
QAYYYSISDDLYNA

SEQ ID NO: 1074 - protein, 12 aa, Oryctolagus cuniculus
AGGYSTNTDTFT

SEQ ID NO: 1075 - protein, 13 aa, Oryctolagus cuniculus
QCTIYGVNFVPNA

SEQ ID NO: 1076 - protein, 13 aa, Oryctolagus cuniculus
QCTVYGVNFVANA

SEQ ID NO: 1077 - protein, 10 aa, Oryctolagus cuniculus
QSVWYAGGAA

SEQ ID NO: 1078 - protein, 13 aa, Oryctolagus cuniculus
AGEFSCASADCFA

SEQ ID NO: 1079 - protein, 12 aa, Oryctolagus cuniculus
QSYGYGSGYVFA

SEQ ID NO: 1080 - protein, 13 aa, Oryctolagus cuniculus
LGNYDCESDDCYA

SEQ ID NO: 1081 - protein, 15 aa, Oryctolagus cuniculus
QCTYGSSSSSAYGWA

SEQ ID NO: 1082 - protein, 11 aa, Oryctolagus cuniculus
LGSYISSSDNA

SEQ ID NO: 1083 - protein, 11 aa, Oryctolagus cuniculus
AGGYSSISDNG

SEQ ID NO: 1084 - protein, 14 aa, Oryctolagus cuniculus
QGYYYYISNTYGYP

SEQ ID NO: 1085 - protein, 12 aa, Oryctolagus cuniculus
QCTYGYSGYVSA

SEQ ID NO: 1086 - protein, 12 aa, Oryctolagus cuniculus
LGVYTYISADNA

SEQ ID NO: 1087 - protein, 13 aa, Oryctolagus cuniculus
QGEFSCSSGDCYA

SEQ ID NO: 1088 - protein, 11 aa, Oryctolagus cuniculus
LGSYISSSDNG

SEQ ID NO: 1089 - protein, 11 aa, Oryctolagus cuniculus
AGGYSDISDNA

SEQ ID NO: 1090 - protein, 13 aa, Oryctolagus cuniculus
QGEFNCGSGDCST

SEQ ID NO: 1091 - protein, 12 aa, Oryctolagus cuniculus
QCTFWDINNFGG

SEQ ID NO: 1092 - protein, 11 aa, Oryctolagus cuniculus
LGGYDADADNA

SEQ ID NO: 1093 - protein, 13 aa, Oryctolagus cuniculus
QGEFSCSSGDCYA

SEQ ID NO: 1094 - protein, 10 aa, Oryctolagus cuniculus
AGAYSGNVGT

SEQ ID NO: 1095 - protein, 12 aa, Oryctolagus cuniculus
QQTYSGSNVENS

SEQ ID NO: 1096 - protein, 13 aa, Oryctolagus cuniculus
QQTYIYNNAEDNT

SEQ ID NO: 1097 - protein, 14 aa, Oryctolagus cuniculus
QCTFGATNDDYGNA

SEQ ID NO: 1098 - protein, 15 aa, Oryctolagus cuniculus
QCTVGSSGVTGYGNA

SEQ ID NO: 1099 - protein, 14 aa, Oryctolagus cuniculus
QNYYGYGLSTNYVV

SEQ ID NO: 1100 - protein, 13 aa, Oryctolagus cuniculus
QGEFSCSSGDCTA

SEQ ID NO: 1101 - protein, 14 aa, Oryctolagus cuniculus
QCTAGSINVSYGNA

SEQ ID NO: 1102 - protein, 13 aa, Oryctolagus cuniculus
LGSYDCSSVDCNA

SEQ ID NO: 1103 - protein, 12 aa, Oryctolagus cuniculus
AGGYDSTIDTFT

SEQ ID NO: 1104 - protein, 15 aa, Oryctolagus cuniculus
QCTYGSSTSSRSGNA

SEQ ID NO: 1105 - protein, 15 aa, Oryctolagus cuniculus
QSYYYGISSTYAFYT

SEQ ID NO: 1106 - protein, 12 aa, Oryctolagus cuniculus
QCTYWDSSTVGA

SEQ ID NO: 1107 - protein, 11 aa, Oryctolagus cuniculus
SGGYISSSDNA

SEQ ID NO: 1108 - protein, 11 aa, Oryctolagus cuniculus
QSTYYGSSGNA

SEQ ID NO: 1109 - protein, 13 aa, Oryctolagus cuniculus
LYGYVTSSNADFA

SEQ ID NO: 1110 - protein, 13 aa, Oryctolagus cuniculus
LGTYDCVSADCGA

SEQ ID NO: 1111 - protein, 12 aa, Oryctolagus cuniculus
QGTYSNNGWYFA

SEQ ID NO: 1112 - protein, 15 aa, Oryctolagus cuniculus
QSYYYGISSTYAFYT

SEQ ID NO: 1113 - protein, 11 aa, Oryctolagus cuniculus
QTYYGGINIFT

SEQ ID NO: 1114 - protein, 13 aa, Oryctolagus cuniculus
LGTYDCSSTDCYA

SEQ ID NO: 1115 - protein, 13 aa, Oryctolagus cuniculus
QCTVYGVNFVPNA

SEQ ID NO: 1116 - protein, 12 aa, Oryctolagus cuniculus
QGGYYISSTDNA

SEQ ID NO: 1117 - protein, 12 aa, Oryctolagus cuniculus
QQGYSSSNVDNA

SEQ ID NO: 1118 - protein, 12 aa, Oryctolagus cuniculus
QGGYYGSSDTVT

SEQ ID NO: 1119 - protein, 12 aa, Oryctolagus cuniculus
AGGYSGSSDVFA

SEQ ID NO: 1120 - protein, 13 aa, Oryctolagus cuniculus
QCTVYGVNYVPNA

SEQ ID NO: 1121 - protein, 12 aa, Oryctolagus cuniculus
QCTYYGGSGDVP

SEQ ID NO: 1122 - protein, 14 aa, Oryctolagus cuniculus
QCTYGTTNTGHYVG

SEQ ID NO: 1123 - protein, 11 aa, Oryctolagus cuniculus
QCTYYSGSPHT

SEQ ID NO: 1124 - protein, 16 aa, Oryctolagus cuniculus
QSNYGSSSISNYGGGA

SEQ ID NO: 1125 - protein, 10 aa, Oryctolagus cuniculus
AGGYSGNMYV

SEQ ID NO: 1126 - protein, 12 aa, Oryctolagus cuniculus
AGGYGSYTDTFA

SEQ ID NO: 1127 - protein, 11 aa, Oryctolagus cuniculus
LGGYDDDADNT

SEQ ID NO: 1128 - protein, 13 aa, Oryctolagus cuniculus
QCTIYGVNFVPNA

SEQ ID NO: 1129 - protein, 12 aa, Oryctolagus cuniculus
QSNYAIISCGAA

SEQ ID NO: 1130 - protein, 12 aa, Oryctolagus cuniculus
QSAYYSSSAVYA

SEQ ID NO: 1131 - protein, 13 aa, Oryctolagus cuniculus
QQTYIYNNAESNA

SEQ ID NO: 1132 - protein, 10 aa, Oryctolagus cuniculus
VGGYSTSGYA

SEQ ID NO: 1133 - protein, 13 aa, Oryctolagus cuniculus
QGEFSCSNGDCIA

SEQ ID NO: 1134 - protein, 12 aa, Oryctolagus cuniculus
QGGYYGSSDTVT

SEQ ID NO: 1135 - protein, 12 aa, Oryctolagus cuniculus
QQGYTSSNVDNV

SEQ ID NO: 1136 - protein, 13 aa, Oryctolagus cuniculus
LGSYDCSSADCNV

SEQ ID NO: 1137 - protein, 13 aa, Oryctolagus cuniculus
QSTFYGVNPVPNA

SEQ ID NO: 1138 - protein, 11 aa, Oryctolagus cuniculus
LGVYDDDADNA

SEQ ID NO: 1139 - protein, 15 aa, Oryctolagus cuniculus
QCTYGSSTSSRSGNA

SEQ ID NO: 1140 - protein, 13 aa, Oryctolagus cuniculus
QCTYGSSGSSFLA

SEQ ID NO: 1141 - protein, 12 aa, Oryctolagus cuniculus
QQTYSGSNVENS

SEQ ID NO: 1142 - protein, 11 aa, Oryctolagus cuniculus
AGDYSSSSDNT

SEQ ID NO: 1143 - protein, 12 aa, Oryctolagus cuniculus
QSTYWESNNIGT

SEQ ID NO: 1144 - protein, 12 aa, Oryctolagus cuniculus
AGGYSGSADTFA

SEQ ID NO: 1145 - protein, 11 aa, Oryctolagus cuniculus
QSYAGISSGVA

SEQ ID NO: 1146 - protein, 14 aa, Oryctolagus cuniculus
QCTYGTTNTGHYVG

SEQ ID NO: 1147 - protein, 12 aa, Oryctolagus cuniculus
AGGYDSSVDTFA

SEQ ID NO: 1148 - protein, 15 aa, Oryctolagus cuniculus
QSHYCCSSNYDYIYA

SEQ ID NO: 1149 - protein, 14 aa, Oryctolagus cuniculus
QSYYYSISDSVDYP

SEQ ID NO: 1150 - protein, 15 aa, Oryctolagus cuniculus
QCTYGSSASSSYGNA

SEQ ID NO: 1151 - protein, 11 aa, Oryctolagus cuniculus
QTYYPSSVTYA

SEQ ID NO: 1152 - protein, 13 aa, Oryctolagus cuniculus
QSTFYGVNPVPTA

SEQ ID NO: 1153 - protein, 11 aa, Oryctolagus cuniculus
AGGYSSSSDNA

SEQ ID NO: 1154 - protein, 10 aa, Oryctolagus cuniculus
QGYYSGYINA

SEQ ID NO: 1155 - protein, 14 aa, Oryctolagus cuniculus
QCTYGSISSSAGNA

SEQ ID NO: 1156 - protein, 10 aa, Oryctolagus cuniculus
QGGYTDATYA

SEQ ID NO: 1157 - protein, 13 aa, Oryctolagus cuniculus
QGEFSCSNGDCIA

SEQ ID NO: 1158 - protein, 14 aa, Oryctolagus cuniculus
QCTYGSISSSSGNA

SEQ ID NO: 1159 - protein, 10 aa, Oryctolagus cuniculus
AGGYIGDIYA

SEQ ID NO: 1160 - protein, 15 aa, Oryctolagus cuniculus
QCTYGSSRVSSYGDA

SEQ ID NO: 1161 - protein, 10 aa, Oryctolagus cuniculus
QSYYGISAYA

SEQ ID NO: 1162 - protein, 13 aa, Oryctolagus cuniculus
QDNYGSSTTYGNS

SEQ ID NO: 1163 - protein, 15 aa, Oryctolagus cuniculus
QSYYHSTSGSSYGNT

SEQ ID NO: 1164 - protein, 13 aa, Oryctolagus cuniculus
QSTYYNISADFYA

SEQ ID NO: 1165 - protein, 11 aa, Oryctolagus cuniculus
AGDYISDSDNT

SEQ ID NO: 1166 - protein, 15 aa, Oryctolagus cuniculus
QCTYGSSSGSYGGWA

SEQ ID NO: 1167 - protein, 12 aa, Oryctolagus cuniculus
QSNYGFSSGSYA

SEQ ID NO: 1168 - protein, 14 aa, Oryctolagus cuniculus
QCTYGSLSSTYGWA

SEQ ID NO: 1169 - protein, 12 aa, Oryctolagus cuniculus
AGGYDRFIDTFA

SEQ ID NO: 1170 - protein, 11 aa, Oryctolagus cuniculus
AGGYITNSDNG

SEQ ID NO: 1171 - protein, 12 aa, Oryctolagus cuniculus
QSYGYGSGYVFA

SEQ ID NO: 1172 - protein, 13 aa, Oryctolagus cuniculus
LYSYYIDSNVDFA

SEQ ID NO: 1173 - protein, 13 aa, Oryctolagus cuniculus
QCTLYGVNFVPNV

SEQ ID NO: 1174 - protein, 15 aa, Oryctolagus cuniculus
QCTVGSSGVTGYGNA

SEQ ID NO: 1175 - protein, 11 aa, Oryctolagus cuniculus
QCTYYGGSPNV

SEQ ID NO: 1176 - protein, 12 aa, Oryctolagus cuniculus
QQGYTTSNVDNT

SEQ ID NO: 1177 - protein, 11 aa, Oryctolagus cuniculus
AGAYVGSSDNT

SEQ ID NO: 1178 - protein, 11 aa, Oryctolagus cuniculus
AGDYSSNSDDA

SEQ ID NO: 1179 - protein, 14 aa, Oryctolagus cuniculus
QSYWYTMGNSYGNT

SEQ ID NO: 1180 - protein, 11 aa, Oryctolagus cuniculus
LGSYINSSDNA

SEQ ID NO: 1181 - protein, 13 aa, Oryctolagus cuniculus
QSAYYSSSTDGGA

SEQ ID NO: 1182 - protein, 13 aa, Oryctolagus cuniculus
QGYYYADSDDNIA

SEQ ID NO: 1183 - protein, 10 aa, Oryctolagus cuniculus
QGYYSTGMFA

SEQ ID NO: 1184 - protein, 13 aa, Oryctolagus cuniculus
QCTLYGVNFVPNA

SEQ ID NO: 1185 - protein, 117 aa, Artificial Sequence
  MAB-17-0119 HC VR
EVQLEESGGRLVQPGTSLRLSCAVSGFSLNSYDMSWVRQAPGKGLEYVGIIYNSGTTYYANWAKGRFTISKDTSKTTLYLQMNSLRAEDTATYFCARTHNTLPFYIWGQGTLVTVSS

SEQ ID NO: 1186 - protein, 122 aa, Artificial Sequence
  MAB-17-0127 HC VR
EVQLVESGGGLVQPGGSLRLSCAASGFSFSSSYYMCWVRQAPGKGLEWVACIYAGSSGSTYYASWAKGRFTISKDISKTTLYLQMNSLRAEDTAVYFCARGGGSGGVDNNLWGQGTLVTVSS

SEQ ID NO: 1187 - protein, 121 aa, Artificial Sequence
  MAB-17-0193 HC VR
EVQLEESGGGLVQPGGSLRLSCAASGFSFNNNYYMCWVRQAPGKGLEWVACIYTGSTGSTYYANWAKGRFTISKDLSKTTLYLQMNSLRAEDTATYFCARDDKVEHGYGLWGQGTLVTVSS

SEQ ID NO: 1188 - protein, 123 aa, Artificial Sequence
  MAB-17-0200 HC VR
EVQLEESGGRLVQPGTSLRLSCAASGFSLSSNSISWVRQAPGKGLEWVGIISSSGSTYYASWAKGRFTISKDASKTTLYLQMNSLRAEDTATYFCAKGLGRGEYTSNDAFDPWGQGTLVTVSS

SEQ ID NO: 1189 - protein, 122 aa, Artificial Sequence
  MAB-17-0201 HC VR
EVQLEESGGDLVQPGGSLRLSCAASGFSFNGNYYICWVRQAPGKGLEWVACIYAGSSGSTYYASWAKGRFTISRDTSKNTLYLQMNSLRAEDTAVYFCVRDKPAGGSSYTLWGQGTLVTVSS

SEQ ID NO: 1190 - protein, 122 aa, Artificial Sequence
  MAB-17-0212 HC VR
EVQLEESGGDLVQPGGSLRLSCAASGFDFSSNYYMCWVRQAPGKGLEWVACIYTGSSGSTYYASWAKGRFTISKDTSKNTLYLQMNSLRAEDTAVYFCARGAGSYGGAVRLWGQGTLVTVSS

SEQ ID NO: 1191 - protein, 121 aa, Artificial Sequence
  MAB-17-0218 HC VR
EVQLEESGGDLVQPGGSLRLSCAASGFSFSRSYYMCWVRQAPGKGLEWVACIYAGSSDSTYYASWAKGRFTISRDTSKNTLYLQMNSLRAEDTAVYFCARGGGIIYTQNLWGQGTLVTVSS

SEQ ID NO: 1192 - protein, 121 aa, Artificial Sequence
  MAB-17-0223 HC VR
EVQLEESGGDLVQPGGSLRLSCAASGFSFSSSYYMCWVRQAPGKGLEWVACIYAGSSGSTYYASWAKGRFTISRDNSKNTLYLQMNSLRAEDTAVYFCARGAGSNGDFNLWGQGTLVTVSS

SEQ ID NO: 1193 - protein, 120 aa, Artificial Sequence
  MAB-17-0225 HC VR
EVQLEESGGDLVQPGGSLRLSCAASGFSFSSSYYMCWVRQAPGKGLEWVACVYAGSSGSTYYASWAKGRFTISRDNSKNTLYLQMNSLRAEDTAVYFCARDRGGTDISLWGQGTLVTVSS

SEQ ID NO: 1194 - protein, 111 aa, Artificial Sequence
  MAB-17-0119 LC VR
DIVMTQSPSSLSASVGDRVTITCQSSPSVYNNNRLSWFQQKPGQAPKLLIYYASTLASGVPSRFSGSGSGTDFTLTISSLQPEDFATYYCAGGYSSISDNGFGQGTKVVIK

SEQ ID NO: 1195 - protein, 111 aa, Artificial Sequence
  MAB-17-0127 LC VR
DIQMTQSPSSLSASVGDRVTITCRASEDIERFLAWYQQKPGQAPKLLIYKASTLASGVPSRFSGSGSGTDFTLTISSLQPEDFATYYCQCTLYGVNFVPNAFGGGTKVVIK

SEQ ID NO: 1196 - protein, 111 aa, Artificial Sequence
  MAB-17-0193 LC VR
DIQMTQSPSSLSASVGDRVTITCQASESIDNWLAWYQQKPGQAPKLLIYSASNLASGVPSRFSGSGSGTDFTLTISSLQPEDFATYYCQSTFYGVNPVPNAFGQGTKVVIK

SEQ ID NO: 1197 - protein, 110 aa, Artificial Sequence
  MAB-17-0200 LC VR
DIQMTQSPSSLSASVGDRVTITCQASETIYSYLNWYQQKPGQAPKLLIYSASTLASGVPSRFSGSGSGTDFTLTISSLQPEDFATYYCQQGYSGRNVENTFGQGTKVVIK

SEQ ID NO: 1198 - protein, 111 aa, Artificial Sequence
  MAB-17-0201 LC VR
DIQMTQSPSSLSASVGDRVTITCQASEDIESYLAWYQQKPGQAPKLLIYQASKLASGVPSRFSGSGSGTDFTLTISSLQPEDFATYYCQCTLYGVNFVPNVFGGGTKVVIK

SEQ ID NO: 1199 - protein, 111 aa, Artificial Sequence
  MAB-17-0212 LC VR
DIQMTQSPSSLSASVGDRVTITCQATEDIESFLAWYQQKPGQAPKLLIYRASTLESGVPSRFSGSGSGTDFTLTISSLQPEDFATYYCQCTVYGVNFVANAFGGGTKVVIK

SEQ ID NO: 1200 - protein, 111 aa, Artificial Sequence
  MAB-17-0218 LC VR
DIQMTQSPSSLSASVGDRVTITCQASEDIESYLAWYQQKPGQAPKLLIYSASTLASGVPSRFSGSGSGTDFTLTISSLQPEDFATYYCQCILYGVNFVPNTFGGGTKVVIK

SEQ ID NO: 1201 - protein, 111 aa, Artificial Sequence
  MAB-17-0223 LC VR
DIQMTQSPSSLSASVGDRVTITCQASEDIESYLAWYQQKPGQAPKLLIYRASTLASGVPSRFSGSGSGTDFTLTISSLQPEDFATYYCQCTIYGVNFVPNAFGGGTKVVIK

SEQ ID NO: 1202 - protein, 111 aa, Artificial Sequence
  MAB-17-0225 LC VR
DIQMTQSPSSLSASVGDRVTITCQASEDIESFLAWYQQKPGQAPKLLIYSASTLASGVPSRFSGSGSGTDFTLTISSLQPEDFATYFCQCTIYGVNFVPNAFGGGTKVVIK

SEQ ID NO: 1203 - protein, 111 aa, Artificial Sequence
  MAB-17-0545 LC VR
DIQMTQSPSSLSASVGDRVTITCQASEDIESYLAWYQQKPGQAPKLLIYQASKLASGVPSRFSGSGSGTDFTLTISSLQPEDFATYYCQSTLYGVNFVPNVFGGGTKVVIK

SEQ ID NO: 1204 - protein, 111 aa, Artificial Sequence
  MAB-17-0547 LC VR
DIQMTQSPSSLSASVGDRVTITCQASEDIESYLAWYQQKPGQAPKLLIYRASTLASGVPSRFSGSGSGTDFTLTISSLQPEDFATYYCQSTIYGVNFVPNAFGGGTKVVIK

SEQ ID NO: 1205 - protein, 13 aa, Artificial Sequence
  MAB-17-0545 CDR H3
QSTLYGVNFVPNV

SEQ ID NO: 1206 - protein, 13 aa, Artificial Sequence
  MAB-17-0547 CDR H3
QSTIYGVNFVPNA